European Patent Specification EP 3 625 371 B1, published May 3, 2023. Title: Set of random primers and method for preparing DNA library using the same. Applicant: TOYOTA JIDOSHA KABUSHIKI KAISHA. The sequence listing filed with the application follows.

SEQUENCE LISTING (2162 sequences)

SEQ ID NO: 1 - DNA, 10 bp, Artificial
  synthetic DNA
agacgtcgtt

SEQ ID NO: 2 - DNA, 10 bp, Artificial
  synthetic DNA
gaggcgatat

SEQ ID NO: 3 - DNA, 10 bp, Artificial
  synthetic DNA
gtgcgaacgt

SEQ ID NO: 4 - DNA, 10 bp, Artificial
  synthetic DNA
ttatactgcc

SEQ ID NO: 5 - DNA, 10 bp, Artificial
  synthetic DNA
caagttcgca

SEQ ID NO: 6 - DNA, 10 bp, Artificial
  synthetic DNA
acaaggtagt

SEQ ID NO: 7 - DNA, 10 bp, Artificial
  synthetic DNA
acacagcgac

SEQ ID NO: 8 - DNA, 10 bp, Artificial
  synthetic DNA
ttaccgatgt

SEQ ID NO: 9 - DNA, 10 bp, Artificial
  synthetic DNA
cacagagtcg

SEQ ID NO: 10 - DNA, 10 bp, Artificial
  synthetic DNA
ttcagcgcgt

SEQ ID NO: 11 - DNA, 10 bp, Artificial
  synthetic DNA
aggaccgtga

SEQ ID NO: 12 - DNA, 10 bp, Artificial
  synthetic DNA
gtctgttcgc

SEQ ID NO: 13 - DNA, 10 bp, Artificial
  synthetic DNA
acctgtccac

SEQ ID NO: 14 - DNA, 10 bp, Artificial
  synthetic DNA
ccgcaatgac

SEQ ID NO: 15 - DNA, 10 bp, Artificial
  synthetic DNA
ctgccgatca

SEQ ID NO: 16 - DNA, 10 bp, Artificial
  synthetic DNA
tacacggagc

SEQ ID NO: 17 - DNA, 10 bp, Artificial
  synthetic DNA
ccgcattcat

SEQ ID NO: 18 - DNA, 10 bp, Artificial
  synthetic DNA
gactctagac

SEQ ID NO: 19 - DNA, 10 bp, Artificial
  synthetic DNA
ggagaactta

SEQ ID NO: 20 - DNA, 10 bp, Artificial
  synthetic DNA
tccggtatgc

SEQ ID NO: 21 - DNA, 10 bp, Artificial
  synthetic DNA
ggtcaggagt

SEQ ID NO: 22 - DNA, 10 bp, Artificial
  synthetic DNA
acattggcag

SEQ ID NO: 23 - DNA, 10 bp, Artificial
  synthetic DNA
cgtagactgc

SEQ ID NO: 24 - DNA, 10 bp, Artificial
  synthetic DNA
agactgtact

SEQ ID NO: 25 - DNA, 10 bp, Artificial
  synthetic DNA
tagacgcagt

SEQ ID NO: 26 - DNA, 10 bp, Artificial
  synthetic DNA
ccgataatct

SEQ ID NO: 27 - DNA, 10 bp, Artificial
  synthetic DNA
gagagctagt

SEQ ID NO: 28 - DNA, 10 bp, Artificial
  synthetic DNA
gtaccgcgtt

SEQ ID NO: 29 - DNA, 10 bp, Artificial
  synthetic DNA
gacttgcgca

SEQ ID NO: 30 - DNA, 10 bp, Artificial
  synthetic DNA
cgtgattgcg

SEQ ID NO: 31 - DNA, 10 bp, Artificial
  synthetic DNA
atcgtctctg

SEQ ID NO: 32 - DNA, 10 bp, Artificial
  synthetic DNA
cgtagctacg

SEQ ID NO: 33 - DNA, 10 bp, Artificial
  synthetic DNA
gccgaatagt

SEQ ID NO: 34 - DNA, 10 bp, Artificial
  synthetic DNA
gtacctaggc

SEQ ID NO: 35 - DNA, 10 bp, Artificial
  synthetic DNA
gcttacatga

SEQ ID NO: 36 - DNA, 10 bp, Artificial
  synthetic DNA
tccacgtagt

SEQ ID NO: 37 - DNA, 10 bp, Artificial
  synthetic DNA
agaggccatc

SEQ ID NO: 38 - DNA, 10 bp, Artificial
  synthetic DNA
cggtgatgct

SEQ ID NO: 39 - DNA, 10 bp, Artificial
  synthetic DNA
cactgtgctt

SEQ ID NO: 40 - DNA, 10 bp, Artificial
  synthetic DNA
catgatggct

SEQ ID NO: 41 - DNA, 10 bp, Artificial
  synthetic DNA
gccacacatg

SEQ ID NO: 42 - DNA, 10 bp, Artificial
  synthetic DNA
cacacactgt

SEQ ID NO: 43 - DNA, 10 bp, Artificial
  synthetic DNA
cagaatcata

SEQ ID NO: 44 - DNA, 10 bp, Artificial
  synthetic DNA
atcgtctacg

SEQ ID NO: 45 - DNA, 10 bp, Artificial
  synthetic DNA
cgagcaatac

SEQ ID NO: 46 - DNA, 10 bp, Artificial
  synthetic DNA
acaagcgcac

SEQ ID NO: 47 - DNA, 10 bp, Artificial
  synthetic DNA
gcttagatgt

SEQ ID NO: 48 - DNA, 10 bp, Artificial
  synthetic DNA
tgcattctgg

SEQ ID NO: 49 - DNA, 10 bp, Artificial
  synthetic DNA
tgtcggacca

SEQ ID NO: 50 - DNA, 10 bp, Artificial
  synthetic DNA
aggcactcgt

SEQ ID NO: 51 - DNA, 10 bp, Artificial
  synthetic DNA
ctgcatgtga

SEQ ID NO: 52 - DNA, 10 bp, Artificial
  synthetic DNA
accacgccta

SEQ ID NO: 53 - DNA, 10 bp, Artificial
  synthetic DNA
gaggtcgtac

SEQ ID NO: 54 - DNA, 10 bp, Artificial
  synthetic DNA
aatactctgt

SEQ ID NO: 55 - DNA, 10 bp, Artificial
  synthetic DNA
tgccaactga

SEQ ID NO: 56 - DNA, 10 bp, Artificial
  synthetic DNA
cctgttcggt

SEQ ID NO: 57 - DNA, 10 bp, Artificial
  synthetic DNA
gtagagagtt

SEQ ID NO: 58 - DNA, 10 bp, Artificial
  synthetic DNA
tacagcgtaa

SEQ ID NO: 59 - DNA, 10 bp, Artificial
  synthetic DNA
tgacgtgatg

SEQ ID NO: 60 - DNA, 10 bp, Artificial
  synthetic DNA
agacgtcggt

SEQ ID NO: 61 - DNA, 10 bp, Artificial
  synthetic DNA
cgctaggttc

SEQ ID NO: 62 - DNA, 10 bp, Artificial
  synthetic DNA
gccttatagc

SEQ ID NO: 63 - DNA, 10 bp, Artificial
  synthetic DNA
ccttcgatct

SEQ ID NO: 64 - DNA, 10 bp, Artificial
  synthetic DNA
aggcaacgtg

SEQ ID NO: 65 - DNA, 10 bp, Artificial
  synthetic DNA
tgagcggtgt

SEQ ID NO: 66 - DNA, 10 bp, Artificial
  synthetic DNA
gtgtcgaacg

SEQ ID NO: 67 - DNA, 10 bp, Artificial
  synthetic DNA
cgatgttgcg

SEQ ID NO: 68 - DNA, 10 bp, Artificial
  synthetic DNA
aacaagacac

SEQ ID NO: 69 - DNA, 10 bp, Artificial
  synthetic DNA
gatgctggtt

SEQ ID NO: 70 - DNA, 10 bp, Artificial
  synthetic DNA
accggtagtc

SEQ ID NO: 71 - DNA, 10 bp, Artificial
  synthetic DNA
gtgactagca

SEQ ID NO: 72 - DNA, 10 bp, Artificial
  synthetic DNA
agcctatatt

SEQ ID NO: 73 - DNA, 10 bp, Artificial
  synthetic DNA
tcgtgagctt

SEQ ID NO: 74 - DNA, 10 bp, Artificial
  synthetic DNA
acactatggc

SEQ ID NO: 75 - DNA, 10 bp, Artificial
  synthetic DNA
gactctgtcg

SEQ ID NO: 76 - DNA, 10 bp, Artificial
  synthetic DNA
tcgatgatgc

SEQ ID NO: 77 - DNA, 10 bp, Artificial
  synthetic DNA
cttggacact

SEQ ID NO: 78 - DNA, 10 bp, Artificial
  synthetic DNA
ggctgatcgt

SEQ ID NO: 79 - DNA, 10 bp, Artificial
  synthetic DNA
actcacaggc

SEQ ID NO: 80 - DNA, 10 bp, Artificial
  synthetic DNA
atgtgcgtac

SEQ ID NO: 81 - DNA, 10 bp, Artificial
  synthetic DNA
caccatcgat

SEQ ID NO: 82 - DNA, 10 bp, Artificial
  synthetic DNA
agccattaac

SEQ ID NO: 83 - DNA, 10 bp, Artificial
  synthetic DNA
aatcgactgt

SEQ ID NO: 84 - DNA, 10 bp, Artificial
  synthetic DNA
aatactagcg

SEQ ID NO: 85 - DNA, 10 bp, Artificial
  synthetic DNA
tcgtcactga

SEQ ID NO: 86 - DNA, 10 bp, Artificial
  synthetic DNA
caggctctta

SEQ ID NO: 87 - DNA, 10 bp, Artificial
  synthetic DNA
ggtcggtgat

SEQ ID NO: 88 - DNA, 10 bp, Artificial
  synthetic DNA
cattaggcgt

SEQ ID NO: 89 - DNA, 10 bp, Artificial
  synthetic DNA
actcgcgagt

SEQ ID NO: 90 - DNA, 10 bp, Artificial
  synthetic DNA
ttccgaataa

SEQ ID NO: 91 - DNA, 10 bp, Artificial
  synthetic DNA
tgagcatcgt

SEQ ID NO: 92 - DNA, 10 bp, Artificial
  synthetic DNA
gccacgtaac

SEQ ID NO: 93 - DNA, 10 bp, Artificial
  synthetic DNA
gaactacatg

SEQ ID NO: 94 - DNA, 10 bp, Artificial
  synthetic DNA
tcgtgaggac

SEQ ID NO: 95 - DNA, 10 bp, Artificial
  synthetic DNA
gcggccttaa

SEQ ID NO: 96 - DNA, 10 bp, Artificial
  synthetic DNA
gctaaggacc

SEQ ID NO: 97 - DNA, 10 bp, Artificial
  synthetic DNA
atagccatta

SEQ ID NO: 98 - DNA, 10 bp, Artificial
  synthetic DNA
cagtaatcat

SEQ ID NO: 99 - DNA, 10 bp, Artificial
  synthetic DNA
actccttaat

SEQ ID NO: 100 - DNA, 10 bp, Artificial
  synthetic DNA
tcgaacatta

SEQ ID NO: 101 - DNA, 10 bp, Artificial
  synthetic DNA
attatgaggt

SEQ ID NO: 102 - DNA, 10 bp, Artificial
  synthetic DNA
aatcttagag

SEQ ID NO: 103 - DNA, 10 bp, Artificial
  synthetic DNA
ttagatgatg

SEQ ID NO: 104 - DNA, 10 bp, Artificial
  synthetic DNA
tacatatctg

SEQ ID NO: 105 - DNA, 10 bp, Artificial
  synthetic DNA
tccttaatca

SEQ ID NO: 106 - DNA, 10 bp, Artificial
  synthetic DNA
gttgagatta

SEQ ID NO: 107 - DNA, 10 bp, Artificial
  synthetic DNA
tgttaacgta

SEQ ID NO: 108 - DNA, 10 bp, Artificial
  synthetic DNA
catacagtaa

SEQ ID NO: 109 - DNA, 10 bp, Artificial
  synthetic DNA
cttatacgaa

SEQ ID NO: 110 - DNA, 10 bp, Artificial
  synthetic DNA
agatctatgt

SEQ ID NO: 111 - DNA, 10 bp, Artificial
  synthetic DNA
aagacttagt

SEQ ID NO: 112 - DNA, 10 bp, Artificial
  synthetic DNA
tgcgcaataa

SEQ ID NO: 113 - DNA, 10 bp, Artificial
  synthetic DNA
ttggccatat

SEQ ID NO: 114 - DNA, 10 bp, Artificial
  synthetic DNA
tattacgagg

SEQ ID NO: 115 - DNA, 10 bp, Artificial
  synthetic DNA
ttatgatcgc

SEQ ID NO: 116 - DNA, 10 bp, Artificial
  synthetic DNA
aacttaggag

SEQ ID NO: 117 - DNA, 10 bp, Artificial
  synthetic DNA
tcacaatcgt

SEQ ID NO: 118 - DNA, 10 bp, Artificial
  synthetic DNA
gagtatatgg

SEQ ID NO: 119 - DNA, 10 bp, Artificial
  synthetic DNA
atcaggacaa

SEQ ID NO: 120 - DNA, 10 bp, Artificial
  synthetic DNA
gtactgatag

SEQ ID NO: 121 - DNA, 10 bp, Artificial
  synthetic DNA
cttatactcg

SEQ ID NO: 122 - DNA, 10 bp, Artificial
  synthetic DNA
taacggacta

SEQ ID NO: 123 - DNA, 10 bp, Artificial
  synthetic DNA
gcgttgtata

SEQ ID NO: 124 - DNA, 10 bp, Artificial
  synthetic DNA
cttaagtgct

SEQ ID NO: 125 - DNA, 10 bp, Artificial
  synthetic DNA
atacgactgt

SEQ ID NO: 126 - DNA, 10 bp, Artificial
  synthetic DNA
actgttatcg

SEQ ID NO: 127 - DNA, 10 bp, Artificial
  synthetic DNA
aatcttgacg

SEQ ID NO: 128 - DNA, 10 bp, Artificial
  synthetic DNA
acatcacctt

SEQ ID NO: 129 - DNA, 10 bp, Artificial
  synthetic DNA
ggtatagtac

SEQ ID NO: 130 - DNA, 10 bp, Artificial
  synthetic DNA
ctaatccaca

SEQ ID NO: 131 - DNA, 10 bp, Artificial
  synthetic DNA
gcaccttatt

SEQ ID NO: 132 - DNA, 10 bp, Artificial
  synthetic DNA
attgacggta

SEQ ID NO: 133 - DNA, 10 bp, Artificial
  synthetic DNA
gacatatggt

SEQ ID NO: 134 - DNA, 10 bp, Artificial
  synthetic DNA
gatagtcgta

SEQ ID NO: 135 - DNA, 10 bp, Artificial
  synthetic DNA
caattatcgc

SEQ ID NO: 136 - DNA, 10 bp, Artificial
  synthetic DNA
cttaggtgat

SEQ ID NO: 137 - DNA, 10 bp, Artificial
  synthetic DNA
catactactg

SEQ ID NO: 138 - DNA, 10 bp, Artificial
  synthetic DNA
taacgcgaat

SEQ ID NO: 139 - DNA, 10 bp, Artificial
  synthetic DNA
caagttacga

SEQ ID NO: 140 - DNA, 10 bp, Artificial
  synthetic DNA
aatctcaagg

SEQ ID NO: 141 - DNA, 10 bp, Artificial
  synthetic DNA
gcaatcatca

SEQ ID NO: 142 - DNA, 10 bp, Artificial
  synthetic DNA
tgtaacgttc

SEQ ID NO: 143 - DNA, 10 bp, Artificial
  synthetic DNA
tatcgttggt

SEQ ID NO: 144 - DNA, 10 bp, Artificial
  synthetic DNA
cgcttaagat

SEQ ID NO: 145 - DNA, 10 bp, Artificial
  synthetic DNA
ttagaactgg

SEQ ID NO: 146 - DNA, 10 bp, Artificial
  synthetic DNA
gtcataacgt

SEQ ID NO: 147 - DNA, 10 bp, Artificial
  synthetic DNA
agagcagtat

SEQ ID NO: 148 - DNA, 10 bp, Artificial
  synthetic DNA
caacatcact

SEQ ID NO: 149 - DNA, 10 bp, Artificial
  synthetic DNA
cagaagctta

SEQ ID NO: 150 - DNA, 10 bp, Artificial
  synthetic DNA
aactaacgtg

SEQ ID NO: 151 - DNA, 10 bp, Artificial
  synthetic DNA
ttataccgct

SEQ ID NO: 152 - DNA, 10 bp, Artificial
  synthetic DNA
gaattcgaga

SEQ ID NO: 153 - DNA, 10 bp, Artificial
  synthetic DNA
ttacgtaacc

SEQ ID NO: 154 - DNA, 10 bp, Artificial
  synthetic DNA
gcatggttaa

SEQ ID NO: 155 - DNA, 10 bp, Artificial
  synthetic DNA
gcacctaatt

SEQ ID NO: 156 - DNA, 10 bp, Artificial
  synthetic DNA
tgtaggttgt

SEQ ID NO: 157 - DNA, 10 bp, Artificial
  synthetic DNA
ccatctggaa

SEQ ID NO: 158 - DNA, 10 bp, Artificial
  synthetic DNA
ttcgcgttga

SEQ ID NO: 159 - DNA, 10 bp, Artificial
  synthetic DNA
aaccgaggtt

SEQ ID NO: 160 - DNA, 10 bp, Artificial
  synthetic DNA
gtacgctgtt

SEQ ID NO: 161 - DNA, 10 bp, Artificial
  synthetic DNA
agtatcctgg

SEQ ID NO: 162 - DNA, 10 bp, Artificial
  synthetic DNA
ggttgtacag

SEQ ID NO: 163 - DNA, 10 bp, Artificial
  synthetic DNA
acgtacacca

SEQ ID NO: 164 - DNA, 10 bp, Artificial
  synthetic DNA
tgtcgagcaa

SEQ ID NO: 165 - DNA, 10 bp, Artificial
  synthetic DNA
gtcgtgttac

SEQ ID NO: 166 - DNA, 10 bp, Artificial
  synthetic DNA
gtgcaatagg

SEQ ID NO: 167 - DNA, 10 bp, Artificial
  synthetic DNA
actcgatgct

SEQ ID NO: 168 - DNA, 10 bp, Artificial
  synthetic DNA
gaatcgcgta

SEQ ID NO: 169 - DNA, 10 bp, Artificial
  synthetic DNA
cggtcattgt

SEQ ID NO: 170 - DNA, 10 bp, Artificial
  synthetic DNA
atcaggcgat

SEQ ID NO: 171 - DNA, 10 bp, Artificial
  synthetic DNA
gtaagatgcg

SEQ ID NO: 172 - DNA, 10 bp, Artificial
  synthetic DNA
ggtctcttga

SEQ ID NO: 173 - DNA, 10 bp, Artificial
  synthetic DNA
tcctcgctaa

SEQ ID NO: 174 - DNA, 10 bp, Artificial
  synthetic DNA
ctgcgtgata

SEQ ID NO: 175 - DNA, 10 bp, Artificial
  synthetic DNA
catactcgtc

SEQ ID NO: 176 - DNA, 10 bp, Artificial
  synthetic DNA
atctgagctc

SEQ ID NO: 177 - DNA, 10 bp, Artificial
  synthetic DNA
acggatagtg

SEQ ID NO: 178 - DNA, 10 bp, Artificial
  synthetic DNA
actgcaatgc

SEQ ID NO: 179 - DNA, 10 bp, Artificial
  synthetic DNA
taacgacgtg

SEQ ID NO: 180 - DNA, 10 bp, Artificial
  synthetic DNA
tagactgtcg

SEQ ID NO: 181 - DNA, 10 bp, Artificial
  synthetic DNA
cagcacttca

SEQ ID NO: 182 - DNA, 10 bp, Artificial
  synthetic DNA
aacattcgcc

SEQ ID NO: 183 - DNA, 10 bp, Artificial
  synthetic DNA
actagtgcgt

SEQ ID NO: 184 - DNA, 10 bp, Artificial
  synthetic DNA
acgctgttct

SEQ ID NO: 185 - DNA, 10 bp, Artificial
  synthetic DNA
cgtcgaatgc

SEQ ID NO: 186 - DNA, 10 bp, Artificial
  synthetic DNA
ctctgacggt

SEQ ID NO: 187 - DNA, 10 bp, Artificial
  synthetic DNA
gtcgccatgt

SEQ ID NO: 188 - DNA, 10 bp, Artificial
  synthetic DNA
ggtccacgtt

SEQ ID NO: 189 - DNA, 10 bp, Artificial
  synthetic DNA
cgagcgactt

SEQ ID NO: 190 - DNA, 10 bp, Artificial
  synthetic DNA
ttgacgcgtg

SEQ ID NO: 191 - DNA, 10 bp, Artificial
  synthetic DNA
ctgagagcct

SEQ ID NO: 192 - DNA, 10 bp, Artificial
  synthetic DNA
cgcgctaact

SEQ ID NO: 193 - DNA, 10 bp, Artificial
  synthetic DNA
ggtcgtcaag

SEQ ID NO: 194 - DNA, 10 bp, Artificial
  synthetic DNA
aggttgacca

SEQ ID NO: 195 - DNA, 10 bp, Artificial
  synthetic DNA
taacggcaac

SEQ ID NO: 196 - DNA, 10 bp, Artificial
  synthetic DNA
gaggctggat

SEQ ID NO: 197 - DNA, 10 bp, Artificial
  synthetic DNA
gtgcacacct

SEQ ID NO: 198 - DNA, 10 bp, Artificial
  synthetic DNA
tgaggaccag

SEQ ID NO: 199 - DNA, 10 bp, Artificial
  synthetic DNA
tacttgcgag

SEQ ID NO: 200 - DNA, 10 bp, Artificial
  synthetic DNA
aactgtgaga

SEQ ID NO: 201 - DNA, 10 bp, Artificial
  synthetic DNA
ctccatcaac

SEQ ID NO: 202 - DNA, 10 bp, Artificial
  synthetic DNA
cggactgtta

SEQ ID NO: 203 - DNA, 10 bp, Artificial
  synthetic DNA
taggacagtc

SEQ ID NO: 204 - DNA, 10 bp, Artificial
  synthetic DNA
agaggacaca

SEQ ID NO: 205 - DNA, 10 bp, Artificial
  synthetic DNA
acattcgcgg

SEQ ID NO: 206 - DNA, 10 bp, Artificial
  synthetic DNA
gcttactgca

SEQ ID NO: 207 - DNA, 10 bp, Artificial
  synthetic DNA
caatacgtaa

SEQ ID NO: 208 - DNA, 10 bp, Artificial
  synthetic DNA
agacttgcgc

SEQ ID NO: 209 - DNA, 10 bp, Artificial
  synthetic DNA
gagcggtgtt

SEQ ID NO: 210 - DNA, 10 bp, Artificial
  synthetic DNA
cgtgagaggt

SEQ ID NO: 211 - DNA, 10 bp, Artificial
  synthetic DNA
aatccgtcag

SEQ ID NO: 212 - DNA, 10 bp, Artificial
  synthetic DNA
atacgtaccg

SEQ ID NO: 213 - DNA, 10 bp, Artificial
  synthetic DNA
aactgattcc

SEQ ID NO: 214 - DNA, 10 bp, Artificial
  synthetic DNA
ctgagcgtac

SEQ ID NO: 215 - DNA, 10 bp, Artificial
  synthetic DNA
gtcggattcg

SEQ ID NO: 216 - DNA, 10 bp, Artificial
  synthetic DNA
gccgaccata

SEQ ID NO: 217 - DNA, 10 bp, Artificial
  synthetic DNA
gcagaactaa

SEQ ID NO: 218 - DNA, 10 bp, Artificial
  synthetic DNA
ctaacgaccg

SEQ ID NO: 219 - DNA, 10 bp, Artificial
  synthetic DNA
gctggaccat

SEQ ID NO: 220 - DNA, 10 bp, Artificial
  synthetic DNA
gacgcggtta

SEQ ID NO: 221 - DNA, 10 bp, Artificial
  synthetic DNA
agtggtgagc

SEQ ID NO: 222 - DNA, 10 bp, Artificial
  synthetic DNA
caggcagtca

SEQ ID NO: 223 - DNA, 10 bp, Artificial
  synthetic DNA
tctgacgtca

SEQ ID NO: 224 - DNA, 10 bp, Artificial
  synthetic DNA
tacatgacgt

SEQ ID NO: 225 - DNA, 10 bp, Artificial
  synthetic DNA
tgaggcaacc

SEQ ID NO: 226 - DNA, 10 bp, Artificial
  synthetic DNA
caactgcagt

SEQ ID NO: 227 - DNA, 10 bp, Artificial
  synthetic DNA
cggagatacg

SEQ ID NO: 228 - DNA, 10 bp, Artificial
  synthetic DNA
cttcgcaagt

SEQ ID NO: 229 - DNA, 10 bp, Artificial
  synthetic DNA
ctggcatacg

SEQ ID NO: 230 - DNA, 10 bp, Artificial
  synthetic DNA
taacgttcgc

SEQ ID NO: 231 - DNA, 10 bp, Artificial
  synthetic DNA
ccggcgttaa

SEQ ID NO: 232 - DNA, 10 bp, Artificial
  synthetic DNA
acaagacgcc

SEQ ID NO: 233 - DNA, 10 bp, Artificial
  synthetic DNA
ccattagact

SEQ ID NO: 234 - DNA, 10 bp, Artificial
  synthetic DNA
gtctgtgaca

SEQ ID NO: 235 - DNA, 10 bp, Artificial
  synthetic DNA
ggcattggac

SEQ ID NO: 236 - DNA, 10 bp, Artificial
  synthetic DNA
tcttcgcacg

SEQ ID NO: 237 - DNA, 10 bp, Artificial
  synthetic DNA
tagcctgtgc

SEQ ID NO: 238 - DNA, 10 bp, Artificial
  synthetic DNA
cactgaccta

SEQ ID NO: 239 - DNA, 10 bp, Artificial
  synthetic DNA
ccgcacgatt

SEQ ID NO: 240 - DNA, 10 bp, Artificial
  synthetic DNA
atagcacacg

SEQ ID NO: 241 - DNA, 10 bp, Artificial
  synthetic DNA
gcacgtcata

SEQ ID NO: 242 - DNA, 10 bp, Artificial
  synthetic DNA
aagccgttgg

SEQ ID NO: 243 - DNA, 10 bp, Artificial
  synthetic DNA
cggaccgtta

SEQ ID NO: 244 - DNA, 10 bp, Artificial
  synthetic DNA
tacacagcgt

SEQ ID NO: 245 - DNA, 10 bp, Artificial
  synthetic DNA
cggacttcag

SEQ ID NO: 246 - DNA, 10 bp, Artificial
  synthetic DNA
tagaacgtca

SEQ ID NO: 247 - DNA, 10 bp, Artificial
  synthetic DNA
ggcattggag

SEQ ID NO: 248 - DNA, 10 bp, Artificial
  synthetic DNA
ggcactcgtt

SEQ ID NO: 249 - DNA, 10 bp, Artificial
  synthetic DNA
gtaccgttaa

SEQ ID NO: 250 - DNA, 10 bp, Artificial
  synthetic DNA
aatacgtgtc

SEQ ID NO: 251 - DNA, 10 bp, Artificial
  synthetic DNA
ccattgacgt

SEQ ID NO: 252 - DNA, 10 bp, Artificial
  synthetic DNA
cgtgaatcgc

SEQ ID NO: 253 - DNA, 10 bp, Artificial
  synthetic DNA
atcaacgcgg

SEQ ID NO: 254 - DNA, 10 bp, Artificial
  synthetic DNA
cgccaaggta

SEQ ID NO: 255 - DNA, 10 bp, Artificial
  synthetic DNA
agaagacgcc

SEQ ID NO: 256 - DNA, 10 bp, Artificial
  synthetic DNA
ccgcatagtc

SEQ ID NO: 257 - DNA, 10 bp, Artificial
  synthetic DNA
cttatatgtg

SEQ ID NO: 258 - DNA, 10 bp, Artificial
  synthetic DNA
ggtctcatcg

SEQ ID NO: 259 - DNA, 10 bp, Artificial
  synthetic DNA
ccaccatgtc

SEQ ID NO: 260 - DNA, 10 bp, Artificial
  synthetic DNA
acgaatgtgt

SEQ ID NO: 261 - DNA, 10 bp, Artificial
  synthetic DNA
ggtagtaaca

SEQ ID NO: 262 - DNA, 10 bp, Artificial
  synthetic DNA
gccacttaat

SEQ ID NO: 263 - DNA, 10 bp, Artificial
  synthetic DNA
atattgcgcc

SEQ ID NO: 264 - DNA, 10 bp, Artificial
  synthetic DNA
gaccaatagt

SEQ ID NO: 265 - DNA, 10 bp, Artificial
  synthetic DNA
aacaacacgg

SEQ ID NO: 266 - DNA, 10 bp, Artificial
  synthetic DNA
atagccgatg

SEQ ID NO: 267 - DNA, 10 bp, Artificial
  synthetic DNA
cgagagcata

SEQ ID NO: 268 - DNA, 10 bp, Artificial
  synthetic DNA
cgagacatga

SEQ ID NO: 269 - DNA, 10 bp, Artificial
  synthetic DNA
cgccaagtta

SEQ ID NO: 270 - DNA, 10 bp, Artificial
  synthetic DNA
ttataatcgc

SEQ ID NO: 271 - DNA, 10 bp, Artificial
  synthetic DNA
tagaagtgca

SEQ ID NO: 272 - DNA, 10 bp, Artificial
  synthetic DNA
ggaggcatgt

SEQ ID NO: 273 - DNA, 10 bp, Artificial
  synthetic DNA
gccacttcga

SEQ ID NO: 274 - DNA, 10 bp, Artificial
  synthetic DNA
tccacggtac

SEQ ID NO: 275 - DNA, 10 bp, Artificial
  synthetic DNA
caactatgca

SEQ ID NO: 276 - DNA, 10 bp, Artificial
  synthetic DNA
caaggaggac

SEQ ID NO: 277 - DNA, 10 bp, Artificial
  synthetic DNA
gaggtaccta

SEQ ID NO: 278 - DNA, 10 bp, Artificial
  synthetic DNA
gagcgcataa

SEQ ID NO: 279 - DNA, 10 bp, Artificial
  synthetic DNA
tcgtcacgtg

SEQ ID NO: 280 - DNA, 10 bp, Artificial
  synthetic DNA
aactgtgaca

SEQ ID NO: 281 - DNA, 10 bp, Artificial
  synthetic DNA
tccacgtgag

SEQ ID NO: 282 - DNA, 10 bp, Artificial
  synthetic DNA
acactgctct

SEQ ID NO: 283 - DNA, 10 bp, Artificial
  synthetic DNA
tacggtgagc

SEQ ID NO: 284 - DNA, 10 bp, Artificial
  synthetic DNA
cggactaagt

SEQ ID NO: 285 - DNA, 10 bp, Artificial
  synthetic DNA
aagccacgtt

SEQ ID NO: 286 - DNA, 10 bp, Artificial
  synthetic DNA
caattactcg

SEQ ID NO: 287 - DNA, 10 bp, Artificial
  synthetic DNA
tctggccata

SEQ ID NO: 288 - DNA, 10 bp, Artificial
  synthetic DNA
tcaggctagt

SEQ ID NO: 289 - DNA, 10 bp, Artificial
  synthetic DNA
ttgacccgga

SEQ ID NO: 290 - DNA, 10 bp, Artificial
  synthetic DNA
tttttatggt

SEQ ID NO: 291 - DNA, 10 bp, Artificial
  synthetic DNA
atgtggtgcg

SEQ ID NO: 292 - DNA, 10 bp, Artificial
  synthetic DNA
aaggcgctag

SEQ ID NO: 293 - DNA, 10 bp, Artificial
  synthetic DNA
tccaactttg

SEQ ID NO: 294 - DNA, 10 bp, Artificial
  synthetic DNA
ccatcccatc

SEQ ID NO: 295 - DNA, 10 bp, Artificial
  synthetic DNA
caatacgagg

SEQ ID NO: 296 - DNA, 10 bp, Artificial
  synthetic DNA
gagtgttacc

SEQ ID NO: 297 - DNA, 10 bp, Artificial
  synthetic DNA
gcctcctgta

SEQ ID NO: 298 - DNA, 10 bp, Artificial
  synthetic DNA
cgaaggttgc

SEQ ID NO: 299 - DNA, 10 bp, Artificial
  synthetic DNA
gaggtgctat

SEQ ID NO: 300 - DNA, 10 bp, Artificial
  synthetic DNA
taggataatt

SEQ ID NO: 301 - DNA, 10 bp, Artificial
  synthetic DNA
cgttgtcctc

SEQ ID NO: 302 - DNA, 10 bp, Artificial
  synthetic DNA
tgagaccagc

SEQ ID NO: 303 - DNA, 10 bp, Artificial
  synthetic DNA
tgcccaagct

SEQ ID NO: 304 - DNA, 10 bp, Artificial
  synthetic DNA
tactgaatcg

SEQ ID NO: 305 - DNA, 10 bp, Artificial
  synthetic DNA
ttacatagtc

SEQ ID NO: 306 - DNA, 10 bp, Artificial
  synthetic DNA
acaaaggaaa

SEQ ID NO: 307 - DNA, 10 bp, Artificial
  synthetic DNA
ctcgcttggg

SEQ ID NO: 308 - DNA, 10 bp, Artificial
  synthetic DNA
ccttgcgtca

SEQ ID NO: 309 - DNA, 10 bp, Artificial
  synthetic DNA
taattccgaa

SEQ ID NO: 310 - DNA, 10 bp, Artificial
  synthetic DNA
gtgagcttga

SEQ ID NO: 311 - DNA, 10 bp, Artificial
  synthetic DNA
atgccgattc

SEQ ID NO: 312 - DNA, 10 bp, Artificial
  synthetic DNA
gcttgggctt

SEQ ID NO: 313 - DNA, 10 bp, Artificial
  synthetic DNA
acaaagcgcc

SEQ ID NO: 314 - DNA, 10 bp, Artificial
  synthetic DNA
gaaagctcta

SEQ ID NO: 315 - DNA, 10 bp, Artificial
  synthetic DNA
taccgaccgt

SEQ ID NO: 316 - DNA, 10 bp, Artificial
  synthetic DNA
tcgaagagac

SEQ ID NO: 317 - DNA, 10 bp, Artificial
  synthetic DNA
gtcgcttacg

SEQ ID NO: 318 - DNA, 10 bp, Artificial
  synthetic DNA
gggctctcca

SEQ ID NO: 319 - DNA, 10 bp, Artificial
  synthetic DNA
gcgcccttgt

SEQ ID NO: 320 - DNA, 10 bp, Artificial
  synthetic DNA
ggcaataggc

SEQ ID NO: 321 - DNA, 10 bp, Artificial
  synthetic DNA
caagtcagga

SEQ ID NO: 322 - DNA, 10 bp, Artificial
  synthetic DNA
gggtcgcaat

SEQ ID NO: 323 - DNA, 10 bp, Artificial
  synthetic DNA
cagcaaccta

SEQ ID NO: 324 - DNA, 10 bp, Artificial
  synthetic DNA
ttcccgccac

SEQ ID NO: 325 - DNA, 10 bp, Artificial
  synthetic DNA
tgtgcatttt

SEQ ID NO: 326 - DNA, 10 bp, Artificial
  synthetic DNA
atcaacgacg

SEQ ID NO: 327 - DNA, 10 bp, Artificial
  synthetic DNA
gtgacgtcca

SEQ ID NO: 328 - DNA, 10 bp, Artificial
  synthetic DNA
cgatctagtc

SEQ ID NO: 329 - DNA, 10 bp, Artificial
  synthetic DNA
ttacatcctg

SEQ ID NO: 330 - DNA, 10 bp, Artificial
  synthetic DNA
agccttcaat

SEQ ID NO: 331 - DNA, 10 bp, Artificial
  synthetic DNA
tccatccgat

SEQ ID NO: 332 - DNA, 10 bp, Artificial
  synthetic DNA
gactgggtct

SEQ ID NO: 333 - DNA, 10 bp, Artificial
  synthetic DNA
ttcggtggag

SEQ ID NO: 334 - DNA, 10 bp, Artificial
  synthetic DNA
gaccagcaca

SEQ ID NO: 335 - DNA, 10 bp, Artificial
  synthetic DNA
cattaacgga

SEQ ID NO: 336 - DNA, 10 bp, Artificial
  synthetic DNA
tttttcttga

SEQ ID NO: 337 - DNA, 10 bp, Artificial
  synthetic DNA
cattgcactg

SEQ ID NO: 338 - DNA, 10 bp, Artificial
  synthetic DNA
tgcggcgatc

SEQ ID NO: 339 - DNA, 10 bp, Artificial
  synthetic DNA
atattgcggt

SEQ ID NO: 340 - DNA, 10 bp, Artificial
  synthetic DNA
gacgtcgctc

SEQ ID NO: 341 - DNA, 10 bp, Artificial
  synthetic DNA
tcgcttatcg

SEQ ID NO: 342 - DNA, 10 bp, Artificial
  synthetic DNA
gcgcagacac

SEQ ID NO: 343 - DNA, 10 bp, Artificial
  synthetic DNA
catgtattgt

SEQ ID NO: 344 - DNA, 10 bp, Artificial
  synthetic DNA
tctataacct

SEQ ID NO: 345 - DNA, 10 bp, Artificial
  synthetic DNA
gtggagacaa

SEQ ID NO: 346 - DNA, 10 bp, Artificial
  synthetic DNA
cgaagattat

SEQ ID NO: 347 - DNA, 10 bp, Artificial
  synthetic DNA
tagcaactgc

SEQ ID NO: 348 - DNA, 10 bp, Artificial
  synthetic DNA
ataatcggta

SEQ ID NO: 349 - DNA, 10 bp, Artificial
  synthetic DNA
caggatgggt

SEQ ID NO: 350 - DNA, 10 bp, Artificial
  synthetic DNA
gacgattccc

SEQ ID NO: 351 - DNA, 10 bp, Artificial
  synthetic DNA
cacgccttac

SEQ ID NO: 352 - DNA, 10 bp, Artificial
  synthetic DNA
agttggttcc

SEQ ID NO: 353 - DNA, 10 bp, Artificial
  synthetic DNA
tcttatcagg

SEQ ID NO: 354 - DNA, 10 bp, Artificial
  synthetic DNA
cgagaagttc

SEQ ID NO: 355 - DNA, 10 bp, Artificial
  synthetic DNA
gtggtagaat

SEQ ID NO: 356 - DNA, 10 bp, Artificial
  synthetic DNA
taggcttgtg

SEQ ID NO: 357 - DNA, 10 bp, Artificial
  synthetic DNA
atgcgttacg

SEQ ID NO: 358 - DNA, 10 bp, Artificial
  synthetic DNA
actaccgagg

SEQ ID NO: 359 - DNA, 10 bp, Artificial
  synthetic DNA
cgagttggtg

SEQ ID NO: 360 - DNA, 10 bp, Artificial
  synthetic DNA
ggacgatcaa

SEQ ID NO: 361 - DNA, 10 bp, Artificial
  synthetic DNA
aacagtatgc

SEQ ID NO: 362 - DNA, 10 bp, Artificial
  synthetic DNA
ttggctgatc

SEQ ID NO: 363 - DNA, 10 bp, Artificial
  synthetic DNA
aggattggaa

SEQ ID NO: 364 - DNA, 10 bp, Artificial
  synthetic DNA
catatggaga

SEQ ID NO: 365 - DNA, 10 bp, Artificial
  synthetic DNA
ctgcaggttt

SEQ ID NO: 366 - DNA, 10 bp, Artificial
  synthetic DNA
ctctcttttt

SEQ ID NO: 367 - DNA, 10 bp, Artificial
  synthetic DNA
agtaggggtc

SEQ ID NO: 368 - DNA, 10 bp, Artificial
  synthetic DNA
acaccgcaag

SEQ ID NO: 369 - DNA, 10 bp, Artificial
  synthetic DNA
gaagcgggag

SEQ ID NO: 370 - DNA, 10 bp, Artificial
  synthetic DNA
gatacggact

SEQ ID NO: 371 - DNA, 10 bp, Artificial
  synthetic DNA
tacgacgtgt

SEQ ID NO: 372 - DNA, 10 bp, Artificial
  synthetic DNA
gtgcctcctt

SEQ ID NO: 373 - DNA, 10 bp, Artificial
  synthetic DNA
ggtgactgat

SEQ ID NO: 374 - DNA, 10 bp, Artificial
  synthetic DNA
atatcttacg

SEQ ID NO: 375 - DNA, 10 bp, Artificial
  synthetic DNA
aatcatacgg

SEQ ID NO: 376 - DNA, 10 bp, Artificial
  synthetic DNA
ctcttgggac

SEQ ID NO: 377 - DNA, 10 bp, Artificial
  synthetic DNA
gacgacaaat

SEQ ID NO: 378 - DNA, 10 bp, Artificial
  synthetic DNA
gttgcgaggt

SEQ ID NO: 379 - DNA, 10 bp, Artificial
  synthetic DNA
aaaccgcacc

SEQ ID NO: 380 - DNA, 10 bp, Artificial
  synthetic DNA
gctaacacgt

SEQ ID NO: 381 - DNA, 10 bp, Artificial
  synthetic DNA
atcatgaggg

SEQ ID NO: 382 - DNA, 10 bp, Artificial
  synthetic DNA
gattcacgta

SEQ ID NO: 383 - DNA, 10 bp, Artificial
  synthetic DNA
tctcgaaaag

SEQ ID NO: 384 - DNA, 10 bp, Artificial
  synthetic DNA
ctcgtaacca

SEQ ID NO: 385 - DNA, 10 bp, Artificial
  synthetic DNA
gttacacacg

SEQ ID NO: 386 - DNA, 10 bp, Artificial
  synthetic DNA
cgtgaagggt

SEQ ID NO: 387 - DNA, 10 bp, Artificial
  synthetic DNA
acgagcatct

SEQ ID NO: 388 - DNA, 10 bp, Artificial
  synthetic DNA
acgagggatt

SEQ ID NO: 389 - DNA, 10 bp, Artificial
  synthetic DNA
gcaacgtcgg

SEQ ID NO: 390 - DNA, 10 bp, Artificial
  synthetic DNA
cacggctagg

SEQ ID NO: 391 - DNA, 10 bp, Artificial
  synthetic DNA
cgtgactctc

SEQ ID NO: 392 - DNA, 10 bp, Artificial
  synthetic DNA
tctagacgca

SEQ ID NO: 393 - DNA, 10 bp, Artificial
  synthetic DNA
ctgcgcacat

SEQ ID NO: 394 - DNA, 10 bp, Artificial
  synthetic DNA
atgcttgaca

SEQ ID NO: 395 - DNA, 10 bp, Artificial
  synthetic DNA
tttgtcgaca

SEQ ID NO: 396 - DNA, 10 bp, Artificial
  synthetic DNA
acgtgtcagc

SEQ ID NO: 397 - DNA, 10 bp, Artificial
  synthetic DNA
gaaaacatta

SEQ ID NO: 398 - DNA, 10 bp, Artificial
  synthetic DNA
acattaacgg

SEQ ID NO: 399 - DNA, 10 bp, Artificial
  synthetic DNA
gtacaggtcc

SEQ ID NO: 400 - DNA, 10 bp, Artificial
  synthetic DNA
ctatgtgtac

SEQ ID NO: 401 - DNA, 10 bp, Artificial
  synthetic DNA
gcgtacatta

SEQ ID NO: 402 - DNA, 10 bp, Artificial
  synthetic DNA
gatttgtggc

SEQ ID NO: 403 - DNA, 10 bp, Artificial
  synthetic DNA
tcgcgcgcta

SEQ ID NO: 404 - DNA, 10 bp, Artificial
  synthetic DNA
acaagggcga

SEQ ID NO: 405 - DNA, 10 bp, Artificial
  synthetic DNA
aacgcgcgat

SEQ ID NO: 406 - DNA, 10 bp, Artificial
  synthetic DNA
cgtaaatgcg

SEQ ID NO: 407 - DNA, 10 bp, Artificial
  synthetic DNA
taggcactac

SEQ ID NO: 408 - DNA, 10 bp, Artificial
  synthetic DNA
gcgaggatcg

SEQ ID NO: 409 - DNA, 10 bp, Artificial
  synthetic DNA
cacgtttact

SEQ ID NO: 410 - DNA, 10 bp, Artificial
  synthetic DNA
taccaccacg

SEQ ID NO: 411 - DNA, 10 bp, Artificial
  synthetic DNA
ttaacaggac

SEQ ID NO: 412 - DNA, 10 bp, Artificial
  synthetic DNA
gctgtataac

SEQ ID NO: 413 - DNA, 10 bp, Artificial
  synthetic DNA
gttgctggca

SEQ ID NO: 414 - DNA, 10 bp, Artificial
  synthetic DNA
agtgtggcca

SEQ ID NO: 415 - DNA, 10 bp, Artificial
  synthetic DNA
ctgcggttgt

SEQ ID NO: 416 - DNA, 10 bp, Artificial
  synthetic DNA
tagatcagcg

SEQ ID NO: 417 - DNA, 10 bp, Artificial
  synthetic DNA
ttccggttat

SEQ ID NO: 418 - DNA, 10 bp, Artificial
  synthetic DNA
gataaactgt

SEQ ID NO: 419 - DNA, 10 bp, Artificial
  synthetic DNA
tacagttgcc

SEQ ID NO: 420 - DNA, 10 bp, Artificial
  synthetic DNA
cgatggcgaa

SEQ ID NO: 421 - DNA, 10 bp, Artificial
  synthetic DNA
ccgacgtcag

SEQ ID NO: 422 - DNA, 10 bp, Artificial
  synthetic DNA
tatggtgcaa

SEQ ID NO: 423 - DNA, 10 bp, Artificial
  synthetic DNA
gacgacagtc

SEQ ID NO: 424 - DNA, 10 bp, Artificial
  synthetic DNA
gtcaccgtcc

SEQ ID NO: 425 - DNA, 10 bp, Artificial
  synthetic DNA
ggttttaaca

SEQ ID NO: 426 - DNA, 10 bp, Artificial
  synthetic DNA
gaggacagta

SEQ ID NO: 427 - DNA, 10 bp, Artificial
  synthetic DNA
gttacctaag

SEQ ID NO: 428 - DNA, 10 bp, Artificial
  synthetic DNA
atcacgtgtt

SEQ ID NO: 429 - DNA, 10 bp, Artificial
  synthetic DNA
taaggcctgg

SEQ ID NO: 430 - DNA, 10 bp, Artificial
  synthetic DNA
tgttcgtagc

SEQ ID NO: 431 - DNA, 10 bp, Artificial
  synthetic DNA
tgaggacgtg

SEQ ID NO: 432 - DNA, 10 bp, Artificial
  synthetic DNA
gtgctgtgta

SEQ ID NO: 433 - DNA, 10 bp, Artificial
  synthetic DNA
gagggtacgc

SEQ ID NO: 434 - DNA, 10 bp, Artificial
  synthetic DNA
ccgtgattgt

SEQ ID NO: 435 - DNA, 10 bp, Artificial
  synthetic DNA
aaaatcgcct

SEQ ID NO: 436 - DNA, 10 bp, Artificial
  synthetic DNA
cgatcgcagt

SEQ ID NO: 437 - DNA, 10 bp, Artificial
  synthetic DNA
acgcaataag

SEQ ID NO: 438 - DNA, 10 bp, Artificial
  synthetic DNA
aaggtgcatc

SEQ ID NO: 439 - DNA, 10 bp, Artificial
  synthetic DNA
cgcgtagata

SEQ ID NO: 440 - DNA, 10 bp, Artificial
  synthetic DNA
cgagcagtgc

SEQ ID NO: 441 - DNA, 10 bp, Artificial
  synthetic DNA
atacgtgacg

SEQ ID NO: 442 - DNA, 10 bp, Artificial
  synthetic DNA
agattgcgcg

SEQ ID NO: 443 - DNA, 10 bp, Artificial
  synthetic DNA
acgtgatgcc

SEQ ID NO: 444 - DNA, 10 bp, Artificial
  synthetic DNA
gtacgcatcg

SEQ ID NO: 445 - DNA, 10 bp, Artificial
  synthetic DNA
tcccgactta

SEQ ID NO: 446 - DNA, 10 bp, Artificial
  synthetic DNA
gtttttacac

SEQ ID NO: 447 - DNA, 10 bp, Artificial
  synthetic DNA
cctgagcgtg

SEQ ID NO: 448 - DNA, 10 bp, Artificial
  synthetic DNA
cggcattgta

SEQ ID NO: 449 - DNA, 10 bp, Artificial
  synthetic DNA
tagagtgcgt

SEQ ID NO: 450 - DNA, 10 bp, Artificial
  synthetic DNA
atggccagac

SEQ ID NO: 451 - DNA, 10 bp, Artificial
  synthetic DNA
cttagcatgc

SEQ ID NO: 452 - DNA, 10 bp, Artificial
  synthetic DNA
acaacacctg

SEQ ID NO: 453 - DNA, 10 bp, Artificial
  synthetic DNA
agtgactatc

SEQ ID NO: 454 - DNA, 10 bp, Artificial
  synthetic DNA
catgctacac

SEQ ID NO: 455 - DNA, 10 bp, Artificial
  synthetic DNA
aaagcgggcg

SEQ ID NO: 456 - DNA, 10 bp, Artificial
  synthetic DNA
agatcgccgt

SEQ ID NO: 457 - DNA, 10 bp, Artificial
  synthetic DNA
cgtagatatt

SEQ ID NO: 458 - DNA, 10 bp, Artificial
  synthetic DNA
aatggcagac

SEQ ID NO: 459 - DNA, 10 bp, Artificial
  synthetic DNA
gtataacgtg

SEQ ID NO: 460 - DNA, 10 bp, Artificial
  synthetic DNA
atgtgcgtca

SEQ ID NO: 461 - DNA, 10 bp, Artificial
  synthetic DNA
cctgccaact

SEQ ID NO: 462 - DNA, 10 bp, Artificial
  synthetic DNA
tttataactc

SEQ ID NO: 463 - DNA, 10 bp, Artificial
  synthetic DNA
acggttacgc

SEQ ID NO: 464 - DNA, 10 bp, Artificial
  synthetic DNA
tagcctcttg

SEQ ID NO: 465 - DNA, 10 bp, Artificial
  synthetic DNA
tcgcgaagtt

SEQ ID NO: 466 - DNA, 10 bp, Artificial
  synthetic DNA
gtctacaacc

SEQ ID NO: 467 - DNA, 10 bp, Artificial
  synthetic DNA
gtctactgcg

SEQ ID NO: 468 - DNA, 10 bp, Artificial
  synthetic DNA
gttgcgtctc

SEQ ID NO: 469 - DNA, 10 bp, Artificial
  synthetic DNA
gggccgctaa

SEQ ID NO: 470 - DNA, 10 bp, Artificial
  synthetic DNA
gtacgtcgga

SEQ ID NO: 471 - DNA, 10 bp, Artificial
  synthetic DNA
agcgagagac

SEQ ID NO: 472 - DNA, 10 bp, Artificial
  synthetic DNA
tggctacggt

SEQ ID NO: 473 - DNA, 10 bp, Artificial
  synthetic DNA
aggcatcacg

SEQ ID NO: 474 - DNA, 10 bp, Artificial
  synthetic DNA
tagctcctcg

SEQ ID NO: 475 - DNA, 10 bp, Artificial
  synthetic DNA
ggctagtcag

SEQ ID NO: 476 - DNA, 10 bp, Artificial
  synthetic DNA
ctcactttat

SEQ ID NO: 477 - DNA, 10 bp, Artificial
  synthetic DNA
acggccacgt

SEQ ID NO: 478 - DNA, 10 bp, Artificial
  synthetic DNA
agcgtatatc

SEQ ID NO: 479 - DNA, 10 bp, Artificial
  synthetic DNA
gacacgtcta

SEQ ID NO: 480 - DNA, 10 bp, Artificial
  synthetic DNA
gccagcgtac

SEQ ID NO: 481 - DNA, 10 bp, Artificial
  synthetic DNA
aacattagcg

SEQ ID NO: 482 - DNA, 10 bp, Artificial
  synthetic DNA
agtgtgctat

SEQ ID NO: 483 - DNA, 10 bp, Artificial
  synthetic DNA
cacgagcgtt

SEQ ID NO: 484 - DNA, 10 bp, Artificial
  synthetic DNA
gtaacgccta

SEQ ID NO: 485 - DNA, 10 bp, Artificial
  synthetic DNA
cacatagtac

SEQ ID NO: 486 - DNA, 10 bp, Artificial
  synthetic DNA
cgcgatatcg

SEQ ID NO: 487 - DNA, 10 bp, Artificial
  synthetic DNA
cgttctgtgc

SEQ ID NO: 488 - DNA, 10 bp, Artificial
  synthetic DNA
ctgatcgcat

SEQ ID NO: 489 - DNA, 10 bp, Artificial
  synthetic DNA
tggcgtgaga

SEQ ID NO: 490 - DNA, 10 bp, Artificial
  synthetic DNA
ttgccaggct

SEQ ID NO: 491 - DNA, 10 bp, Artificial
  synthetic DNA
gttatacaca

SEQ ID NO: 492 - DNA, 10 bp, Artificial
  synthetic DNA
agtgccaact

SEQ ID NO: 493 - DNA, 10 bp, Artificial
  synthetic DNA
tcacgtagca

SEQ ID NO: 494 - DNA, 10 bp, Artificial
  synthetic DNA
taattcagcg

SEQ ID NO: 495 - DNA, 10 bp, Artificial
  synthetic DNA
aagtatcgtc

SEQ ID NO: 496 - DNA, 10 bp, Artificial
  synthetic DNA
cacagttact

SEQ ID NO: 497 - DNA, 10 bp, Artificial
  synthetic DNA
ccttaccgtg

SEQ ID NO: 498 - DNA, 10 bp, Artificial
  synthetic DNA
acggtgtcgt

SEQ ID NO: 499 - DNA, 10 bp, Artificial
  synthetic DNA
cgcgtaagac

SEQ ID NO: 500 - DNA, 10 bp, Artificial
  synthetic DNA
ttcgcaccag

SEQ ID NO: 501 - DNA, 10 bp, Artificial
  synthetic DNA
cacgaacaga

SEQ ID NO: 502 - DNA, 10 bp, Artificial
  synthetic DNA
gttggacatt

SEQ ID NO: 503 - DNA, 10 bp, Artificial
  synthetic DNA
ggtgcttaag

SEQ ID NO: 504 - DNA, 10 bp, Artificial
  synthetic DNA
tcggtctcgt

SEQ ID NO: 505 - DNA, 10 bp, Artificial
  synthetic DNA
tctagtacgc

SEQ ID NO: 506 - DNA, 10 bp, Artificial
  synthetic DNA
ttaggccgag

SEQ ID NO: 507 - DNA, 10 bp, Artificial
  synthetic DNA
cgtcaagagc

SEQ ID NO: 508 - DNA, 10 bp, Artificial
  synthetic DNA
acatgtctac

SEQ ID NO: 509 - DNA, 10 bp, Artificial
  synthetic DNA
atcgttacgt

SEQ ID NO: 510 - DNA, 10 bp, Artificial
  synthetic DNA
acggatcgtt

SEQ ID NO: 511 - DNA, 10 bp, Artificial
  synthetic DNA
aatcttggcg

SEQ ID NO: 512 - DNA, 10 bp, Artificial
  synthetic DNA
agtatctggt

SEQ ID NO: 513 - DNA, 10 bp, Artificial
  synthetic DNA
caaccgacgt

SEQ ID NO: 514 - DNA, 10 bp, Artificial
  synthetic DNA
tggtaacgcg

SEQ ID NO: 515 - DNA, 10 bp, Artificial
  synthetic DNA
gtgcagacat

SEQ ID NO: 516 - DNA, 10 bp, Artificial
  synthetic DNA
gtctagttgc

SEQ ID NO: 517 - DNA, 10 bp, Artificial
  synthetic DNA
caattcgacg

SEQ ID NO: 518 - DNA, 10 bp, Artificial
  synthetic DNA
cttagcacct

SEQ ID NO: 519 - DNA, 10 bp, Artificial
  synthetic DNA
taatgtcgca

SEQ ID NO: 520 - DNA, 10 bp, Artificial
  synthetic DNA
caatcggtac

SEQ ID NO: 521 - DNA, 10 bp, Artificial
  synthetic DNA
agcacgcatt

SEQ ID NO: 522 - DNA, 10 bp, Artificial
  synthetic DNA
aggtcctcgt

SEQ ID NO: 523 - DNA, 10 bp, Artificial
  synthetic DNA
ttgtgcctgc

SEQ ID NO: 524 - DNA, 10 bp, Artificial
  synthetic DNA
accgcctgta

SEQ ID NO: 525 - DNA, 10 bp, Artificial
  synthetic DNA
gtacgtcagg

SEQ ID NO: 526 - DNA, 10 bp, Artificial
  synthetic DNA
gcacacaact

SEQ ID NO: 527 - DNA, 10 bp, Artificial
  synthetic DNA
tgagcactta

SEQ ID NO: 528 - DNA, 10 bp, Artificial
  synthetic DNA
gtgccgcata

SEQ ID NO: 529 - DNA, 10 bp, Artificial
  synthetic DNA
atgttttcgc

SEQ ID NO: 530 - DNA, 10 bp, Artificial
  synthetic DNA
acacttaggt

SEQ ID NO: 531 - DNA, 10 bp, Artificial
  synthetic DNA
cgtgccgtga

SEQ ID NO: 532 - DNA, 10 bp, Artificial
  synthetic DNA
ttactaatca

SEQ ID NO: 533 - DNA, 10 bp, Artificial
  synthetic DNA
gtggcaggta

SEQ ID NO: 534 - DNA, 10 bp, Artificial
  synthetic DNA
gcgcgatatg

SEQ ID NO: 535 - DNA, 10 bp, Artificial
  synthetic DNA
gaacgacgtt

SEQ ID NO: 536 - DNA, 10 bp, Artificial
  synthetic DNA
atcaggagtg

SEQ ID NO: 537 - DNA, 10 bp, Artificial
  synthetic DNA
gccagtaagt

SEQ ID NO: 538 - DNA, 10 bp, Artificial
  synthetic DNA
gcaagaagca

SEQ ID NO: 539 - DNA, 10 bp, Artificial
  synthetic DNA
aactccgcca

SEQ ID NO: 540 - DNA, 10 bp, Artificial
  synthetic DNA
acttgagcct

SEQ ID NO: 541 - DNA, 10 bp, Artificial
  synthetic DNA
cgtgatcgtg

SEQ ID NO: 542 - DNA, 10 bp, Artificial
  synthetic DNA
aattagcgaa

SEQ ID NO: 543 - DNA, 10 bp, Artificial
  synthetic DNA
acttccttag

SEQ ID NO: 544 - DNA, 10 bp, Artificial
  synthetic DNA
tgtgctgata

SEQ ID NO: 545 - DNA, 10 bp, Artificial
  synthetic DNA
aggcggctga

SEQ ID NO: 546 - DNA, 10 bp, Artificial
  synthetic DNA
cgtttagagc

SEQ ID NO: 547 - DNA, 10 bp, Artificial
  synthetic DNA
acgcgtctaa

SEQ ID NO: 548 - DNA, 10 bp, Artificial
  synthetic DNA
gcgaatgtac

SEQ ID NO: 549 - DNA, 10 bp, Artificial
  synthetic DNA
cgtgatccaa

SEQ ID NO: 550 - DNA, 10 bp, Artificial
  synthetic DNA
caaccagatg

SEQ ID NO: 551 - DNA, 10 bp, Artificial
  synthetic DNA
accattaacc

SEQ ID NO: 552 - DNA, 10 bp, Artificial
  synthetic DNA
cgattcacgt

SEQ ID NO: 553 - DNA, 10 bp, Artificial
  synthetic DNA
ctagaacctg

SEQ ID NO: 554 - DNA, 10 bp, Artificial
  synthetic DNA
cctaacgaca

SEQ ID NO: 555 - DNA, 10 bp, Artificial
  synthetic DNA
gacgtgcatg

SEQ ID NO: 556 - DNA, 10 bp, Artificial
  synthetic DNA
atgtaacctt

SEQ ID NO: 557 - DNA, 10 bp, Artificial
  synthetic DNA
gatacagtcg

SEQ ID NO: 558 - DNA, 10 bp, Artificial
  synthetic DNA
cgtatgtctc

SEQ ID NO: 559 - DNA, 10 bp, Artificial
  synthetic DNA
agattatcga

SEQ ID NO: 560 - DNA, 10 bp, Artificial
  synthetic DNA
atactggtaa

SEQ ID NO: 561 - DNA, 10 bp, Artificial
  synthetic DNA
gttgagtagc

SEQ ID NO: 562 - DNA, 10 bp, Artificial
  synthetic DNA
accattatca

SEQ ID NO: 563 - DNA, 10 bp, Artificial
  synthetic DNA
cacacttcag

SEQ ID NO: 564 - DNA, 10 bp, Artificial
  synthetic DNA
gactagcggt

SEQ ID NO: 565 - DNA, 10 bp, Artificial
  synthetic DNA
aattgtcgag

SEQ ID NO: 566 - DNA, 10 bp, Artificial
  synthetic DNA
ctaaggacgt

SEQ ID NO: 567 - DNA, 10 bp, Artificial
  synthetic DNA
attacgatga

SEQ ID NO: 568 - DNA, 10 bp, Artificial
  synthetic DNA
attgaagact

SEQ ID NO: 569 - DNA, 10 bp, Artificial
  synthetic DNA
gcttgtacgt

SEQ ID NO: 570 - DNA, 10 bp, Artificial
  synthetic DNA
cctacgtcac

SEQ ID NO: 571 - DNA, 10 bp, Artificial
  synthetic DNA
cacaacttag

SEQ ID NO: 572 - DNA, 10 bp, Artificial
  synthetic DNA
gcggttcatc

SEQ ID NO: 573 - DNA, 10 bp, Artificial
  synthetic DNA
gtactcatct

SEQ ID NO: 574 - DNA, 10 bp, Artificial
  synthetic DNA
gtgcatcagt

SEQ ID NO: 575 - DNA, 10 bp, Artificial
  synthetic DNA
tcacatccta

SEQ ID NO: 576 - DNA, 10 bp, Artificial
  synthetic DNA
cacgcgctat

SEQ ID NO: 577 - DNA, 8 bp, Artificial
  synthetic DNA
ctatcttg

SEQ ID NO: 578 - DNA, 8 bp, Artificial
  synthetic DNA
aagtgcgt

SEQ ID NO: 579 - DNA, 8 bp, Artificial
  synthetic DNA
acatgcga

SEQ ID NO: 580 - DNA, 8 bp, Artificial
  synthetic DNA
accaatgg

SEQ ID NO: 581 - DNA, 8 bp, Artificial
  synthetic DNA
tgcgttga

SEQ ID NO: 582 - DNA, 8 bp, Artificial
  synthetic DNA
gacatgtc

SEQ ID NO: 583 - DNA, 8 bp, Artificial
  synthetic DNA
ttgtgcgt

SEQ ID NO: 584 - DNA, 8 bp, Artificial
  synthetic DNA
acatcgca

SEQ ID NO: 585 - DNA, 8 bp, Artificial
  synthetic DNA
gaagacga

SEQ ID NO: 586 - DNA, 8 bp, Artificial
  synthetic DNA
tcgataga

SEQ ID NO: 587 - DNA, 8 bp, Artificial
  synthetic DNA
tcttgcaa

SEQ ID NO: 588 - DNA, 8 bp, Artificial
  synthetic DNA
agcaagtt

SEQ ID NO: 589 - DNA, 8 bp, Artificial
  synthetic DNA
ttcatgga

SEQ ID NO: 590 - DNA, 8 bp, Artificial
  synthetic DNA
tcaattcg

SEQ ID NO: 591 - DNA, 8 bp, Artificial
  synthetic DNA
cggtatgt

SEQ ID NO: 592 - DNA, 8 bp, Artificial
  synthetic DNA
accactac

SEQ ID NO: 593 - DNA, 8 bp, Artificial
  synthetic DNA
tcgcttat

SEQ ID NO: 594 - DNA, 8 bp, Artificial
  synthetic DNA
tctcgact

SEQ ID NO: 595 - DNA, 8 bp, Artificial
  synthetic DNA
gaatcggt

SEQ ID NO: 596 - DNA, 8 bp, Artificial
  synthetic DNA
gttacaag

SEQ ID NO: 597 - DNA, 8 bp, Artificial
  synthetic DNA
ctgtgtag

SEQ ID NO: 598 - DNA, 8 bp, Artificial
  synthetic DNA
tggtagaa

SEQ ID NO: 599 - DNA, 8 bp, Artificial
  synthetic DNA
atactgcg

SEQ ID NO: 600 - DNA, 8 bp, Artificial
  synthetic DNA
aactcgtc

SEQ ID NO: 601 - DNA, 8 bp, Artificial
  synthetic DNA
atatgtgc

SEQ ID NO: 602 - DNA, 8 bp, Artificial
  synthetic DNA
aagttgcg

SEQ ID NO: 603 - DNA, 8 bp, Artificial
  synthetic DNA
gatcatgt

SEQ ID NO: 604 - DNA, 8 bp, Artificial
  synthetic DNA
ttgttgct

SEQ ID NO: 605 - DNA, 8 bp, Artificial
  synthetic DNA
cctcttag

SEQ ID NO: 606 - DNA, 8 bp, Artificial
  synthetic DNA
tcacagct

SEQ ID NO: 607 - DNA, 8 bp, Artificial
  synthetic DNA
agattgac

SEQ ID NO: 608 - DNA, 8 bp, Artificial
  synthetic DNA
agcctgat

SEQ ID NO: 609 - DNA, 8 bp, Artificial
  synthetic DNA
cgtcaagt

SEQ ID NO: 610 - DNA, 8 bp, Artificial
  synthetic DNA
aagtagac

SEQ ID NO: 611 - DNA, 8 bp, Artificial
  synthetic DNA
tcagacaa

SEQ ID NO: 612 - DNA, 8 bp, Artificial
  synthetic DNA
tccttgac

SEQ ID NO: 613 - DNA, 8 bp, Artificial
  synthetic DNA
gtagctgt

SEQ ID NO: 614 - DNA, 8 bp, Artificial
  synthetic DNA
cgtcgtaa

SEQ ID NO: 615 - DNA, 8 bp, Artificial
  synthetic DNA
ccaatgga

SEQ ID NO: 616 - DNA, 8 bp, Artificial
  synthetic DNA
ttgagaga

SEQ ID NO: 617 - DNA, 8 bp, Artificial
  synthetic DNA
acaacacc

SEQ ID NO: 618 - DNA, 8 bp, Artificial
  synthetic DNA
tctagtac

SEQ ID NO: 619 - DNA, 8 bp, Artificial
  synthetic DNA
gaggaagt

SEQ ID NO: 620 - DNA, 8 bp, Artificial
  synthetic DNA
gcgtattg

SEQ ID NO: 621 - DNA, 8 bp, Artificial
  synthetic DNA
aagtagct

SEQ ID NO: 622 - DNA, 8 bp, Artificial
  synthetic DNA
tgaacctt

SEQ ID NO: 623 - DNA, 8 bp, Artificial
  synthetic DNA
tgtgttac

SEQ ID NO: 624 - DNA, 8 bp, Artificial
  synthetic DNA
taacctga

SEQ ID NO: 625 - DNA, 8 bp, Artificial
  synthetic DNA
gctattcc

SEQ ID NO: 626 - DNA, 8 bp, Artificial
  synthetic DNA
gttagatg

SEQ ID NO: 627 - DNA, 8 bp, Artificial
  synthetic DNA
caggataa

SEQ ID NO: 628 - DNA, 8 bp, Artificial
  synthetic DNA
accgtagt

SEQ ID NO: 629 - DNA, 8 bp, Artificial
  synthetic DNA
ccgtgtat

SEQ ID NO: 630 - DNA, 8 bp, Artificial
  synthetic DNA
tccactct

SEQ ID NO: 631 - DNA, 8 bp, Artificial
  synthetic DNA
tagctcat

SEQ ID NO: 632 - DNA, 8 bp, Artificial
  synthetic DNA
cgctaata

SEQ ID NO: 633 - DNA, 8 bp, Artificial
  synthetic DNA
tacctctg

SEQ ID NO: 634 - DNA, 8 bp, Artificial
  synthetic DNA
tgcactac

SEQ ID NO: 635 - DNA, 8 bp, Artificial
  synthetic DNA
cttggaag

SEQ ID NO: 636 - DNA, 8 bp, Artificial
  synthetic DNA
aatgcacg

SEQ ID NO: 637 - DNA, 8 bp, Artificial
  synthetic DNA
cactgtta

SEQ ID NO: 638 - DNA, 8 bp, Artificial
  synthetic DNA
tcgactag

SEQ ID NO: 639 - DNA, 8 bp, Artificial
  synthetic DNA
ctaggtta

SEQ ID NO: 640 - DNA, 8 bp, Artificial
  synthetic DNA
gcagatgt

SEQ ID NO: 641 - DNA, 8 bp, Artificial
  synthetic DNA
agttcaga

SEQ ID NO: 642 - DNA, 8 bp, Artificial
  synthetic DNA
ctccatca

SEQ ID NO: 643 - DNA, 8 bp, Artificial
  synthetic DNA
tggttacg

SEQ ID NO: 644 - DNA, 8 bp, Artificial
  synthetic DNA
acgtagca

SEQ ID NO: 645 - DNA, 8 bp, Artificial
  synthetic DNA
ctcttcca

SEQ ID NO: 646 - DNA, 8 bp, Artificial
  synthetic DNA
cgtcagat

SEQ ID NO: 647 - DNA, 8 bp, Artificial
  synthetic DNA
tggatcat

SEQ ID NO: 648 - DNA, 8 bp, Artificial
  synthetic DNA
atatcgac

SEQ ID NO: 649 - DNA, 8 bp, Artificial
  synthetic DNA
ttgtggag

SEQ ID NO: 650 - DNA, 8 bp, Artificial
  synthetic DNA
ttagagca

SEQ ID NO: 651 - DNA, 8 bp, Artificial
  synthetic DNA
taactacc

SEQ ID NO: 652 - DNA, 8 bp, Artificial
  synthetic DNA
ctatgagg

SEQ ID NO: 653 - DNA, 8 bp, Artificial
  synthetic DNA
cttctcac

SEQ ID NO: 654 - DNA, 8 bp, Artificial
  synthetic DNA
cgttctct

SEQ ID NO: 655 - DNA, 8 bp, Artificial
  synthetic DNA
gtcactat

SEQ ID NO: 656 - DNA, 8 bp, Artificial
  synthetic DNA
tcgttagc

SEQ ID NO: 657 - DNA, 8 bp, Artificial
  synthetic DNA
atcgtgta

SEQ ID NO: 658 - DNA, 8 bp, Artificial
  synthetic DNA
gagagcaa

SEQ ID NO: 659 - DNA, 8 bp, Artificial
  synthetic DNA
agacgcaa

SEQ ID NO: 660 - DNA, 8 bp, Artificial
  synthetic DNA
tccagtta

SEQ ID NO: 661 - DNA, 8 bp, Artificial
  synthetic DNA
aatgccac

SEQ ID NO: 662 - DNA, 8 bp, Artificial
  synthetic DNA
atcacgtg

SEQ ID NO: 663 - DNA, 8 bp, Artificial
  synthetic DNA
actgtgca

SEQ ID NO: 664 - DNA, 8 bp, Artificial
  synthetic DNA
tcactgca

SEQ ID NO: 665 - DNA, 8 bp, Artificial
  synthetic DNA
gcatccaa

SEQ ID NO: 666 - DNA, 8 bp, Artificial
  synthetic DNA
agcactat

SEQ ID NO: 667 - DNA, 8 bp, Artificial
  synthetic DNA
cgaaggat

SEQ ID NO: 668 - DNA, 8 bp, Artificial
  synthetic DNA
ccttgtgt

SEQ ID NO: 669 - DNA, 8 bp, Artificial
  synthetic DNA
tgcggata

SEQ ID NO: 670 - DNA, 8 bp, Artificial
  synthetic DNA
aggaatgg

SEQ ID NO: 671 - DNA, 8 bp, Artificial
  synthetic DNA
atcgtaac

SEQ ID NO: 672 - DNA, 8 bp, Artificial
  synthetic DNA
gaatgtct

SEQ ID NO: 673 - DNA, 9 bp, Artificial
  synthetic DNA
ttgctacat

SEQ ID NO: 674 - DNA, 9 bp, Artificial
  synthetic DNA
taacgtatg

SEQ ID NO: 675 - DNA, 9 bp, Artificial
  synthetic DNA
cagtatgta

SEQ ID NO: 676 - DNA, 9 bp, Artificial
  synthetic DNA
tcaataacg

SEQ ID NO: 677 - DNA, 9 bp, Artificial
  synthetic DNA
cacacttat

SEQ ID NO: 678 - DNA, 9 bp, Artificial
  synthetic DNA
gactgtaat

SEQ ID NO: 679 - DNA, 9 bp, Artificial
  synthetic DNA
tatacactg

SEQ ID NO: 680 - DNA, 9 bp, Artificial
  synthetic DNA
actgcatta

SEQ ID NO: 681 - DNA, 9 bp, Artificial
  synthetic DNA
acattaagc

SEQ ID NO: 682 - DNA, 9 bp, Artificial
  synthetic DNA
catattacg

SEQ ID NO: 683 - DNA, 9 bp, Artificial
  synthetic DNA
atatctacg

SEQ ID NO: 684 - DNA, 9 bp, Artificial
  synthetic DNA
agtaactgt

SEQ ID NO: 685 - DNA, 9 bp, Artificial
  synthetic DNA
atgacgtta

SEQ ID NO: 686 - DNA, 9 bp, Artificial
  synthetic DNA
attatgcga

SEQ ID NO: 687 - DNA, 9 bp, Artificial
  synthetic DNA
agtatacac

SEQ ID NO: 688 - DNA, 9 bp, Artificial
  synthetic DNA
ttagcgtta

SEQ ID NO: 689 - DNA, 9 bp, Artificial
  synthetic DNA
tatgacact

SEQ ID NO: 690 - DNA, 9 bp, Artificial
  synthetic DNA
attaacgct

SEQ ID NO: 691 - DNA, 9 bp, Artificial
  synthetic DNA
taggacaat

SEQ ID NO: 692 - DNA, 9 bp, Artificial
  synthetic DNA
aagacgtta

SEQ ID NO: 693 - DNA, 9 bp, Artificial
  synthetic DNA
tataagcgt

SEQ ID NO: 694 - DNA, 9 bp, Artificial
  synthetic DNA
atacctggc

SEQ ID NO: 695 - DNA, 9 bp, Artificial
  synthetic DNA
ctcgagatc

SEQ ID NO: 696 - DNA, 9 bp, Artificial
  synthetic DNA
atggtgagg

SEQ ID NO: 697 - DNA, 9 bp, Artificial
  synthetic DNA
atgtcgacg

SEQ ID NO: 698 - DNA, 9 bp, Artificial
  synthetic DNA
gacgtctga

SEQ ID NO: 699 - DNA, 9 bp, Artificial
  synthetic DNA
tacactgcg

SEQ ID NO: 700 - DNA, 9 bp, Artificial
  synthetic DNA
atcgtcagg

SEQ ID NO: 701 - DNA, 9 bp, Artificial
  synthetic DNA
tgcacgtac

SEQ ID NO: 702 - DNA, 9 bp, Artificial
  synthetic DNA
gtcgtgcat

SEQ ID NO: 703 - DNA, 9 bp, Artificial
  synthetic DNA
gagtgttac

SEQ ID NO: 704 - DNA, 9 bp, Artificial
  synthetic DNA
agactgtac

SEQ ID NO: 705 - DNA, 9 bp, Artificial
  synthetic DNA
tgcgactta

SEQ ID NO: 706 - DNA, 9 bp, Artificial
  synthetic DNA
tgtccgtaa

SEQ ID NO: 707 - DNA, 9 bp, Artificial
  synthetic DNA
gtaatcgag

SEQ ID NO: 708 - DNA, 9 bp, Artificial
  synthetic DNA
gtaccttag

SEQ ID NO: 709 - DNA, 9 bp, Artificial
  synthetic DNA
atcacgtgt

SEQ ID NO: 710 - DNA, 9 bp, Artificial
  synthetic DNA
acttagcgt

SEQ ID NO: 711 - DNA, 9 bp, Artificial
  synthetic DNA
gtaatcgtg

SEQ ID NO: 712 - DNA, 9 bp, Artificial
  synthetic DNA
atgccgtta

SEQ ID NO: 713 - DNA, 9 bp, Artificial
  synthetic DNA
ataacgtgc

SEQ ID NO: 714 - DNA, 9 bp, Artificial
  synthetic DNA
ctacgttgt

SEQ ID NO: 715 - DNA, 9 bp, Artificial
  synthetic DNA
tatgacgca

SEQ ID NO: 716 - DNA, 9 bp, Artificial
  synthetic DNA
ccgataaca

SEQ ID NO: 717 - DNA, 9 bp, Artificial
  synthetic DNA
atgcgcata

SEQ ID NO: 718 - DNA, 9 bp, Artificial
  synthetic DNA
gataagcgt

SEQ ID NO: 719 - DNA, 9 bp, Artificial
  synthetic DNA
atatctgcg

SEQ ID NO: 720 - DNA, 9 bp, Artificial
  synthetic DNA
acttagacg

SEQ ID NO: 721 - DNA, 9 bp, Artificial
  synthetic DNA
atcaccgta

SEQ ID NO: 722 - DNA, 9 bp, Artificial
  synthetic DNA
taagacacg

SEQ ID NO: 723 - DNA, 9 bp, Artificial
  synthetic DNA
aatgccgta

SEQ ID NO: 724 - DNA, 9 bp, Artificial
  synthetic DNA
aatcacgtg

SEQ ID NO: 725 - DNA, 9 bp, Artificial
  synthetic DNA
tcgttagtc

SEQ ID NO: 726 - DNA, 9 bp, Artificial
  synthetic DNA
catcatgtc

SEQ ID NO: 727 - DNA, 9 bp, Artificial
  synthetic DNA
taagacggt

SEQ ID NO: 728 - DNA, 9 bp, Artificial
  synthetic DNA
tgcatagtg

SEQ ID NO: 729 - DNA, 9 bp, Artificial
  synthetic DNA
gagcgttat

SEQ ID NO: 730 - DNA, 9 bp, Artificial
  synthetic DNA
tgccttaca

SEQ ID NO: 731 - DNA, 9 bp, Artificial
  synthetic DNA
ttcgcgtta

SEQ ID NO: 732 - DNA, 9 bp, Artificial
  synthetic DNA
gtgttaacg

SEQ ID NO: 733 - DNA, 9 bp, Artificial
  synthetic DNA
gacactgaa

SEQ ID NO: 734 - DNA, 9 bp, Artificial
  synthetic DNA
ctgttatcg

SEQ ID NO: 735 - DNA, 9 bp, Artificial
  synthetic DNA
ggtcgttat

SEQ ID NO: 736 - DNA, 9 bp, Artificial
  synthetic DNA
cgagagtat

SEQ ID NO: 737 - DNA, 9 bp, Artificial
  synthetic DNA
atacagtcc

SEQ ID NO: 738 - DNA, 9 bp, Artificial
  synthetic DNA
aattcacgc

SEQ ID NO: 739 - DNA, 9 bp, Artificial
  synthetic DNA
tatgtgcac

SEQ ID NO: 740 - DNA, 9 bp, Artificial
  synthetic DNA
gatgacgta

SEQ ID NO: 741 - DNA, 9 bp, Artificial
  synthetic DNA
gatgcgata

SEQ ID NO: 742 - DNA, 9 bp, Artificial
  synthetic DNA
gagcgatta

SEQ ID NO: 743 - DNA, 9 bp, Artificial
  synthetic DNA
tgtcacaga

SEQ ID NO: 744 - DNA, 9 bp, Artificial
  synthetic DNA
tactaaccg

SEQ ID NO: 745 - DNA, 9 bp, Artificial
  synthetic DNA
cataacgag

SEQ ID NO: 746 - DNA, 9 bp, Artificial
  synthetic DNA
cgtatacct

SEQ ID NO: 747 - DNA, 9 bp, Artificial
  synthetic DNA
tatcacgtg

SEQ ID NO: 748 - DNA, 9 bp, Artificial
  synthetic DNA
gaacgttac

SEQ ID NO: 749 - DNA, 9 bp, Artificial
  synthetic DNA
gtcgtatac

SEQ ID NO: 750 - DNA, 9 bp, Artificial
  synthetic DNA
atgtcgaca

SEQ ID NO: 751 - DNA, 9 bp, Artificial
  synthetic DNA
atacagcac

SEQ ID NO: 752 - DNA, 9 bp, Artificial
  synthetic DNA
tacttacgc

SEQ ID NO: 753 - DNA, 9 bp, Artificial
  synthetic DNA
aactacggt

SEQ ID NO: 754 - DNA, 9 bp, Artificial
  synthetic DNA
tagaacggt

SEQ ID NO: 755 - DNA, 9 bp, Artificial
  synthetic DNA
gaatgtcac

SEQ ID NO: 756 - DNA, 9 bp, Artificial
  synthetic DNA
tgtacgtct

SEQ ID NO: 757 - DNA, 9 bp, Artificial
  synthetic DNA
aacattgcg

SEQ ID NO: 758 - DNA, 9 bp, Artificial
  synthetic DNA
ttgaacgct

SEQ ID NO: 759 - DNA, 9 bp, Artificial
  synthetic DNA
aatcaggac

SEQ ID NO: 760 - DNA, 9 bp, Artificial
  synthetic DNA
attcgcaca

SEQ ID NO: 761 - DNA, 9 bp, Artificial
  synthetic DNA
ccatgtact

SEQ ID NO: 762 - DNA, 9 bp, Artificial
  synthetic DNA
tgtcctgtt

SEQ ID NO: 763 - DNA, 9 bp, Artificial
  synthetic DNA
taattgcgc

SEQ ID NO: 764 - DNA, 9 bp, Artificial
  synthetic DNA
gatagtgtg

SEQ ID NO: 765 - DNA, 9 bp, Artificial
  synthetic DNA
atagacgca

SEQ ID NO: 766 - DNA, 9 bp, Artificial
  synthetic DNA
tgtaccgtt

SEQ ID NO: 767 - DNA, 9 bp, Artificial
  synthetic DNA
attgtcgca

SEQ ID NO: 768 - DNA, 9 bp, Artificial
  synthetic DNA
gtcacgtaa

SEQ ID NO: 769 - DNA, 11 bp, Artificial
  synthetic DNA
ttacactatgc

SEQ ID NO: 770 - DNA, 11 bp, Artificial
  synthetic DNA
gcgatagtcgt

SEQ ID NO: 771 - DNA, 11 bp, Artificial
  synthetic DNA
ctattcacagt

SEQ ID NO: 772 - DNA, 11 bp, Artificial
  synthetic DNA
agagtcactgt

SEQ ID NO: 773 - DNA, 11 bp, Artificial
  synthetic DNA
agagtcgaagc

SEQ ID NO: 774 - DNA, 11 bp, Artificial
  synthetic DNA
ctgaatatgtg

SEQ ID NO: 775 - DNA, 11 bp, Artificial
  synthetic DNA
actccacagga

SEQ ID NO: 776 - DNA, 11 bp, Artificial
  synthetic DNA
atcctcgtaag

SEQ ID NO: 777 - DNA, 11 bp, Artificial
  synthetic DNA
taccatcgcct

SEQ ID NO: 778 - DNA, 11 bp, Artificial
  synthetic DNA
aacgcctataa

SEQ ID NO: 779 - DNA, 11 bp, Artificial
  synthetic DNA
ctgtcgaactt

SEQ ID NO: 780 - DNA, 11 bp, Artificial
  synthetic DNA
tcagatgtccg

SEQ ID NO: 781 - DNA, 11 bp, Artificial
  synthetic DNA
ctgcttatcgt

SEQ ID NO: 782 - DNA, 11 bp, Artificial
  synthetic DNA
acattcgcaca

SEQ ID NO: 783 - DNA, 11 bp, Artificial
  synthetic DNA
ccttaatgcat

SEQ ID NO: 784 - DNA, 11 bp, Artificial
  synthetic DNA
ggctagctact

SEQ ID NO: 785 - DNA, 11 bp, Artificial
  synthetic DNA
ttccagttggc

SEQ ID NO: 786 - DNA, 11 bp, Artificial
  synthetic DNA
gagtcacaagg

SEQ ID NO: 787 - DNA, 11 bp, Artificial
  synthetic DNA
cagaaggttca

SEQ ID NO: 788 - DNA, 11 bp, Artificial
  synthetic DNA
tcaacgtgcag

SEQ ID NO: 789 - DNA, 11 bp, Artificial
  synthetic DNA
caagcttacta

SEQ ID NO: 790 - DNA, 11 bp, Artificial
  synthetic DNA
agaactcgttg

SEQ ID NO: 791 - DNA, 11 bp, Artificial
  synthetic DNA
ccgatacagag

SEQ ID NO: 792 - DNA, 11 bp, Artificial
  synthetic DNA
gtacgctgatc

SEQ ID NO: 793 - DNA, 11 bp, Artificial
  synthetic DNA
tcctcagtgaa

SEQ ID NO: 794 - DNA, 11 bp, Artificial
  synthetic DNA
gagccaacatt

SEQ ID NO: 795 - DNA, 11 bp, Artificial
  synthetic DNA
gagatcgatgg

SEQ ID NO: 796 - DNA, 11 bp, Artificial
  synthetic DNA
atcgtcagctg

SEQ ID NO: 797 - DNA, 11 bp, Artificial
  synthetic DNA
gaagcacacgt

SEQ ID NO: 798 - DNA, 11 bp, Artificial
  synthetic DNA
atcacgcaacc

SEQ ID NO: 799 - DNA, 11 bp, Artificial
  synthetic DNA
tcgaatagtcg

SEQ ID NO: 800 - DNA, 11 bp, Artificial
  synthetic DNA
tattaccgtct

SEQ ID NO: 801 - DNA, 11 bp, Artificial
  synthetic DNA
cagtcacgaca

SEQ ID NO: 802 - DNA, 11 bp, Artificial
  synthetic DNA
ttactcgacgt

SEQ ID NO: 803 - DNA, 11 bp, Artificial
  synthetic DNA
gcaatgttgaa

SEQ ID NO: 804 - DNA, 11 bp, Artificial
  synthetic DNA
gacacgagcaa

SEQ ID NO: 805 - DNA, 11 bp, Artificial
  synthetic DNA
cgagattacaa

SEQ ID NO: 806 - DNA, 11 bp, Artificial
  synthetic DNA
taccgactaca

SEQ ID NO: 807 - DNA, 11 bp, Artificial
  synthetic DNA
accgttgccat

SEQ ID NO: 808 - DNA, 11 bp, Artificial
  synthetic DNA
atgtaatcgcc

SEQ ID NO: 809 - DNA, 11 bp, Artificial
  synthetic DNA
aagcctgatgt

SEQ ID NO: 810 - DNA, 11 bp, Artificial
  synthetic DNA
aagtaacgtgg

SEQ ID NO: 811 - DNA, 11 bp, Artificial
  synthetic DNA
gtagaggttgg

SEQ ID NO: 812 - DNA, 11 bp, Artificial
  synthetic DNA
ctcttgcctca

SEQ ID NO: 813 - DNA, 11 bp, Artificial
  synthetic DNA
atcgtgaagtg

SEQ ID NO: 814 - DNA, 11 bp, Artificial
  synthetic DNA
accagcactat

SEQ ID NO: 815 - DNA, 11 bp, Artificial
  synthetic DNA
caccagaatgt

SEQ ID NO: 816 - DNA, 11 bp, Artificial
  synthetic DNA
gagtgaacaac

SEQ ID NO: 817 - DNA, 11 bp, Artificial
  synthetic DNA
taacgttacgc

SEQ ID NO: 818 - DNA, 11 bp, Artificial
  synthetic DNA
cttggatcttg

SEQ ID NO: 819 - DNA, 11 bp, Artificial
  synthetic DNA
gttccaacgtt

SEQ ID NO: 820 - DNA, 11 bp, Artificial
  synthetic DNA
caaggaccgta

SEQ ID NO: 821 - DNA, 11 bp, Artificial
  synthetic DNA
gacttcacgca

SEQ ID NO: 822 - DNA, 11 bp, Artificial
  synthetic DNA
cacactactgg

SEQ ID NO: 823 - DNA, 11 bp, Artificial
  synthetic DNA
tcagatgaatc

SEQ ID NO: 824 - DNA, 11 bp, Artificial
  synthetic DNA
tatggatctgg

SEQ ID NO: 825 - DNA, 11 bp, Artificial
  synthetic DNA
tcttaggtgtg

SEQ ID NO: 826 - DNA, 11 bp, Artificial
  synthetic DNA
tgtcagcgtca

SEQ ID NO: 827 - DNA, 11 bp, Artificial
  synthetic DNA
gtctaggacag

SEQ ID NO: 828 - DNA, 11 bp, Artificial
  synthetic DNA
gcctcttcata

SEQ ID NO: 829 - DNA, 11 bp, Artificial
  synthetic DNA
agaagtgttac

SEQ ID NO: 830 - DNA, 11 bp, Artificial
  synthetic DNA
catgaggcttg

SEQ ID NO: 831 - DNA, 11 bp, Artificial
  synthetic DNA
tggattgctca

SEQ ID NO: 832 - DNA, 11 bp, Artificial
  synthetic DNA
atctacctaag

SEQ ID NO: 833 - DNA, 11 bp, Artificial
  synthetic DNA
atgagcagtga

SEQ ID NO: 834 - DNA, 11 bp, Artificial
  synthetic DNA
ccaggagatac

SEQ ID NO: 835 - DNA, 11 bp, Artificial
  synthetic DNA
ccgttatactt

SEQ ID NO: 836 - DNA, 11 bp, Artificial
  synthetic DNA
ctcagtacaag

SEQ ID NO: 837 - DNA, 11 bp, Artificial
  synthetic DNA
ggtgatcgtag

SEQ ID NO: 838 - DNA, 11 bp, Artificial
  synthetic DNA
cgaacgagaca

SEQ ID NO: 839 - DNA, 11 bp, Artificial
  synthetic DNA
actacgagctt

SEQ ID NO: 840 - DNA, 11 bp, Artificial
  synthetic DNA
ttgccacagca

SEQ ID NO: 841 - DNA, 11 bp, Artificial
  synthetic DNA
gtcaactctac

SEQ ID NO: 842 - DNA, 11 bp, Artificial
  synthetic DNA
tggactgtgtc

SEQ ID NO: 843 - DNA, 11 bp, Artificial
  synthetic DNA
ggaatggactt

SEQ ID NO: 844 - DNA, 11 bp, Artificial
  synthetic DNA
cgagaacataa

SEQ ID NO: 845 - DNA, 11 bp, Artificial
  synthetic DNA
acctggtcagt

SEQ ID NO: 846 - DNA, 11 bp, Artificial
  synthetic DNA
cgaacgacaca

SEQ ID NO: 847 - DNA, 11 bp, Artificial
  synthetic DNA
agtctagccat

SEQ ID NO: 848 - DNA, 11 bp, Artificial
  synthetic DNA
aggcctagatg

SEQ ID NO: 849 - DNA, 11 bp, Artificial
  synthetic DNA
ggtgcgttagt

SEQ ID NO: 850 - DNA, 11 bp, Artificial
  synthetic DNA
attgtgtccga

SEQ ID NO: 851 - DNA, 11 bp, Artificial
  synthetic DNA
gcagacattaa

SEQ ID NO: 852 - DNA, 11 bp, Artificial
  synthetic DNA
attggctcatg

SEQ ID NO: 853 - DNA, 11 bp, Artificial
  synthetic DNA
gaggttacatg

SEQ ID NO: 854 - DNA, 11 bp, Artificial
  synthetic DNA
cctataggacc

SEQ ID NO: 855 - DNA, 11 bp, Artificial
  synthetic DNA
ttagacggtct

SEQ ID NO: 856 - DNA, 11 bp, Artificial
  synthetic DNA
gattgacgcac

SEQ ID NO: 857 - DNA, 11 bp, Artificial
  synthetic DNA
aagacacctcg

SEQ ID NO: 858 - DNA, 11 bp, Artificial
  synthetic DNA
tcgaataatcg

SEQ ID NO: 859 - DNA, 11 bp, Artificial
  synthetic DNA
tctatgtcgga

SEQ ID NO: 860 - DNA, 11 bp, Artificial
  synthetic DNA
tcgcatgaacc

SEQ ID NO: 861 - DNA, 11 bp, Artificial
  synthetic DNA
tgttatgtctc

SEQ ID NO: 862 - DNA, 11 bp, Artificial
  synthetic DNA
tggatcctaca

SEQ ID NO: 863 - DNA, 11 bp, Artificial
  synthetic DNA
atcgttcagcc

SEQ ID NO: 864 - DNA, 11 bp, Artificial
  synthetic DNA
taccgcaagca

SEQ ID NO: 865 - DNA, 12 bp, Artificial
  synthetic DNA
gctgttgaaccg

SEQ ID NO: 866 - DNA, 12 bp, Artificial
  synthetic DNA
atactccgagat

SEQ ID NO: 867 - DNA, 12 bp, Artificial
  synthetic DNA
cttaaggagcgc

SEQ ID NO: 868 - DNA, 12 bp, Artificial
  synthetic DNA
tatactacaagc

SEQ ID NO: 869 - DNA, 12 bp, Artificial
  synthetic DNA
tagtggtcgtca

SEQ ID NO: 870 - DNA, 12 bp, Artificial
  synthetic DNA
gtgcttcaggag

SEQ ID NO: 871 - DNA, 12 bp, Artificial
  synthetic DNA
gacgcatacctc

SEQ ID NO: 872 - DNA, 12 bp, Artificial
  synthetic DNA
cctacctgtgga

SEQ ID NO: 873 - DNA, 12 bp, Artificial
  synthetic DNA
gcggtcacatat

SEQ ID NO: 874 - DNA, 12 bp, Artificial
  synthetic DNA
ctgcattcacga

SEQ ID NO: 875 - DNA, 12 bp, Artificial
  synthetic DNA
tggatccttcat

SEQ ID NO: 876 - DNA, 12 bp, Artificial
  synthetic DNA
ttgtgctggact

SEQ ID NO: 877 - DNA, 12 bp, Artificial
  synthetic DNA
attgagagctat

SEQ ID NO: 878 - DNA, 12 bp, Artificial
  synthetic DNA
tcgctaatgtag

SEQ ID NO: 879 - DNA, 12 bp, Artificial
  synthetic DNA
ctactggcacaa

SEQ ID NO: 880 - DNA, 12 bp, Artificial
  synthetic DNA
agagccagtcgt

SEQ ID NO: 881 - DNA, 12 bp, Artificial
  synthetic DNA
aatactggctaa

SEQ ID NO: 882 - DNA, 12 bp, Artificial
  synthetic DNA
ctgcatgcataa

SEQ ID NO: 883 - DNA, 12 bp, Artificial
  synthetic DNA
ttgtcacaactc

SEQ ID NO: 884 - DNA, 12 bp, Artificial
  synthetic DNA
tgctaactctcc

SEQ ID NO: 885 - DNA, 12 bp, Artificial
  synthetic DNA
tctctagttcgg

SEQ ID NO: 886 - DNA, 12 bp, Artificial
  synthetic DNA
ttacgtccgcaa

SEQ ID NO: 887 - DNA, 12 bp, Artificial
  synthetic DNA
gtgttgctacca

SEQ ID NO: 888 - DNA, 12 bp, Artificial
  synthetic DNA
cgcatgtatgcc

SEQ ID NO: 889 - DNA, 12 bp, Artificial
  synthetic DNA
cctgttctgatt

SEQ ID NO: 890 - DNA, 12 bp, Artificial
  synthetic DNA
taagatgcttga

SEQ ID NO: 891 - DNA, 12 bp, Artificial
  synthetic DNA
atatatctcagc

SEQ ID NO: 892 - DNA, 12 bp, Artificial
  synthetic DNA
ttcctcgtggtt

SEQ ID NO: 893 - DNA, 12 bp, Artificial
  synthetic DNA
atgtcgatctag

SEQ ID NO: 894 - DNA, 12 bp, Artificial
  synthetic DNA
catccactaatc

SEQ ID NO: 895 - DNA, 12 bp, Artificial
  synthetic DNA
gcctctggtaac

SEQ ID NO: 896 - DNA, 12 bp, Artificial
  synthetic DNA
agtcaagagatt

SEQ ID NO: 897 - DNA, 12 bp, Artificial
  synthetic DNA
actgaggcgttc

SEQ ID NO: 898 - DNA, 12 bp, Artificial
  synthetic DNA
taaggctgacat

SEQ ID NO: 899 - DNA, 12 bp, Artificial
  synthetic DNA
agttcgcataca

SEQ ID NO: 900 - DNA, 12 bp, Artificial
  synthetic DNA
gcagaattgcga

SEQ ID NO: 901 - DNA, 12 bp, Artificial
  synthetic DNA
ggttatgaagaa

SEQ ID NO: 902 - DNA, 12 bp, Artificial
  synthetic DNA
agaagtcgcctc

SEQ ID NO: 903 - DNA, 12 bp, Artificial
  synthetic DNA
ttcgcgttattg

SEQ ID NO: 904 - DNA, 12 bp, Artificial
  synthetic DNA
tacctggtcggt

SEQ ID NO: 905 - DNA, 12 bp, Artificial
  synthetic DNA
ggttaccgagga

SEQ ID NO: 906 - DNA, 12 bp, Artificial
  synthetic DNA
acacacttctag

SEQ ID NO: 907 - DNA, 12 bp, Artificial
  synthetic DNA
ggaagtgattaa

SEQ ID NO: 908 - DNA, 12 bp, Artificial
  synthetic DNA
tccatcagataa

SEQ ID NO: 909 - DNA, 12 bp, Artificial
  synthetic DNA
tgtctgtatcat

SEQ ID NO: 910 - DNA, 12 bp, Artificial
  synthetic DNA
aattggctatag

SEQ ID NO: 911 - DNA, 12 bp, Artificial
  synthetic DNA
acgtcggaaggt

SEQ ID NO: 912 - DNA, 12 bp, Artificial
  synthetic DNA
aggcatccgttg

SEQ ID NO: 913 - DNA, 12 bp, Artificial
  synthetic DNA
accgtcgcttga

SEQ ID NO: 914 - DNA, 12 bp, Artificial
  synthetic DNA
taccgtcaagtg

SEQ ID NO: 915 - DNA, 12 bp, Artificial
  synthetic DNA
ctcgatatagtt

SEQ ID NO: 916 - DNA, 12 bp, Artificial
  synthetic DNA
cgtcaacgtggt

SEQ ID NO: 917 - DNA, 12 bp, Artificial
  synthetic DNA
tagtcaacgtag

SEQ ID NO: 918 - DNA, 12 bp, Artificial
  synthetic DNA
tgagtaggtcag

SEQ ID NO: 919 - DNA, 12 bp, Artificial
  synthetic DNA
cttggcatgtac

SEQ ID NO: 920 - DNA, 12 bp, Artificial
  synthetic DNA
tgccgagacttc

SEQ ID NO: 921 - DNA, 12 bp, Artificial
  synthetic DNA
ctaagacttaag

SEQ ID NO: 922 - DNA, 12 bp, Artificial
  synthetic DNA
ttctcgtgtgcg

SEQ ID NO: 923 - DNA, 12 bp, Artificial
  synthetic DNA
cacctgcacgat

SEQ ID NO: 924 - DNA, 12 bp, Artificial
  synthetic DNA
attaagcctaag

SEQ ID NO: 925 - DNA, 12 bp, Artificial
  synthetic DNA
ggtggaaccatg

SEQ ID NO: 926 - DNA, 12 bp, Artificial
  synthetic DNA
actaacgcgact

SEQ ID NO: 927 - DNA, 12 bp, Artificial
  synthetic DNA
cagttgtgctat

SEQ ID NO: 928 - DNA, 12 bp, Artificial
  synthetic DNA
acgctgttagca

SEQ ID NO: 929 - DNA, 12 bp, Artificial
  synthetic DNA
gtcaacgctaag

SEQ ID NO: 930 - DNA, 12 bp, Artificial
  synthetic DNA
agcttaggtatg

SEQ ID NO: 931 - DNA, 12 bp, Artificial
  synthetic DNA
cgcaggacgatt

SEQ ID NO: 932 - DNA, 12 bp, Artificial
  synthetic DNA
aaccggctgtct

SEQ ID NO: 933 - DNA, 12 bp, Artificial
  synthetic DNA
gttgctcacgtg

SEQ ID NO: 934 - DNA, 12 bp, Artificial
  synthetic DNA
gaatcttccgcg

SEQ ID NO: 935 - DNA, 12 bp, Artificial
  synthetic DNA
agagcgtacacg

SEQ ID NO: 936 - DNA, 12 bp, Artificial
  synthetic DNA
aaggctaatgtc

SEQ ID NO: 937 - DNA, 12 bp, Artificial
  synthetic DNA
tctatgtagacg

SEQ ID NO: 938 - DNA, 12 bp, Artificial
  synthetic DNA
agacggtctagt

SEQ ID NO: 939 - DNA, 12 bp, Artificial
  synthetic DNA
ttggtcacacgc

SEQ ID NO: 940 - DNA, 12 bp, Artificial
  synthetic DNA
gtcgatatatgg

SEQ ID NO: 941 - DNA, 12 bp, Artificial
  synthetic DNA
aacatggatacg

SEQ ID NO: 942 - DNA, 12 bp, Artificial
  synthetic DNA
ttcgcagttcct

SEQ ID NO: 943 - DNA, 12 bp, Artificial
  synthetic DNA
cgcatgttgtgc

SEQ ID NO: 944 - DNA, 12 bp, Artificial
  synthetic DNA
tgttaagttgga

SEQ ID NO: 945 - DNA, 12 bp, Artificial
  synthetic DNA
caagtgtgatga

SEQ ID NO: 946 - DNA, 12 bp, Artificial
  synthetic DNA
ctggtaccacgt

SEQ ID NO: 947 - DNA, 12 bp, Artificial
  synthetic DNA
cgctaggatcac

SEQ ID NO: 948 - DNA, 12 bp, Artificial
  synthetic DNA
tgctcattacgg

SEQ ID NO: 949 - DNA, 12 bp, Artificial
  synthetic DNA
tgctcagtaaca

SEQ ID NO: 950 - DNA, 12 bp, Artificial
  synthetic DNA
acgatcatagcc

SEQ ID NO: 951 - DNA, 12 bp, Artificial
  synthetic DNA
acgatacgtgga

SEQ ID NO: 952 - DNA, 12 bp, Artificial
  synthetic DNA
gttcgatgatgg

SEQ ID NO: 953 - DNA, 12 bp, Artificial
  synthetic DNA
aagagctgtgcc

SEQ ID NO: 954 - DNA, 12 bp, Artificial
  synthetic DNA
ggttggatcaac

SEQ ID NO: 955 - DNA, 12 bp, Artificial
  synthetic DNA
gcgcgcttatga

SEQ ID NO: 956 - DNA, 12 bp, Artificial
  synthetic DNA
cgtcgatcatca

SEQ ID NO: 957 - DNA, 12 bp, Artificial
  synthetic DNA
gagactgcactc

SEQ ID NO: 958 - DNA, 12 bp, Artificial
  synthetic DNA
gatagatcgcat

SEQ ID NO: 959 - DNA, 12 bp, Artificial
  synthetic DNA
ggccatcatcag

SEQ ID NO: 960 - DNA, 12 bp, Artificial
  synthetic DNA
ggtgttccactg

SEQ ID NO: 961 - DNA, 14 bp, Artificial
  synthetic DNA
agctatacagaggt

SEQ ID NO: 962 - DNA, 14 bp, Artificial
  synthetic DNA
aggccgttctgtct

SEQ ID NO: 963 - DNA, 14 bp, Artificial
  synthetic DNA
cattggtctgctat

SEQ ID NO: 964 - DNA, 14 bp, Artificial
  synthetic DNA
ctacatacgcgcca

SEQ ID NO: 965 - DNA, 14 bp, Artificial
  synthetic DNA
gcttaacggcgctt

SEQ ID NO: 966 - DNA, 14 bp, Artificial
  synthetic DNA
tacgatactccacc

SEQ ID NO: 967 - DNA, 14 bp, Artificial
  synthetic DNA
accggcataagaag

SEQ ID NO: 968 - DNA, 14 bp, Artificial
  synthetic DNA
ggatgcttcgataa

SEQ ID NO: 969 - DNA, 14 bp, Artificial
  synthetic DNA
gtgtacctgaatgt

SEQ ID NO: 970 - DNA, 14 bp, Artificial
  synthetic DNA
cgcggatacacaga

SEQ ID NO: 971 - DNA, 14 bp, Artificial
  synthetic DNA
ttccacggcactgt

SEQ ID NO: 972 - DNA, 14 bp, Artificial
  synthetic DNA
tagccaggcaacaa

SEQ ID NO: 973 - DNA, 14 bp, Artificial
  synthetic DNA
agcgtcaacacgta

SEQ ID NO: 974 - DNA, 14 bp, Artificial
  synthetic DNA
taacgctactcgcg

SEQ ID NO: 975 - DNA, 14 bp, Artificial
  synthetic DNA
tagatagacgatct

SEQ ID NO: 976 - DNA, 14 bp, Artificial
  synthetic DNA
actcttgcaatgct

SEQ ID NO: 977 - DNA, 14 bp, Artificial
  synthetic DNA
actcggttaggtcg

SEQ ID NO: 978 - DNA, 14 bp, Artificial
  synthetic DNA
cattatctacgcat

SEQ ID NO: 979 - DNA, 14 bp, Artificial
  synthetic DNA
cacaccggcgatta

SEQ ID NO: 980 - DNA, 14 bp, Artificial
  synthetic DNA
tacgcagtactgtg

SEQ ID NO: 981 - DNA, 14 bp, Artificial
  synthetic DNA
caagcgcgtgaatg

SEQ ID NO: 982 - DNA, 14 bp, Artificial
  synthetic DNA
gaatggactgacga

SEQ ID NO: 983 - DNA, 14 bp, Artificial
  synthetic DNA
ctagcgctgaagtt

SEQ ID NO: 984 - DNA, 14 bp, Artificial
  synthetic DNA
tgcggcagaccaat

SEQ ID NO: 985 - DNA, 14 bp, Artificial
  synthetic DNA
aaggcatagagatt

SEQ ID NO: 986 - DNA, 14 bp, Artificial
  synthetic DNA
ttctcctcgccatg

SEQ ID NO: 987 - DNA, 14 bp, Artificial
  synthetic DNA
tcattggtcgtgaa

SEQ ID NO: 988 - DNA, 14 bp, Artificial
  synthetic DNA
attacgctatacga

SEQ ID NO: 989 - DNA, 14 bp, Artificial
  synthetic DNA
atgatcctccacgg

SEQ ID NO: 990 - DNA, 14 bp, Artificial
  synthetic DNA
cgtcgttagtaatc

SEQ ID NO: 991 - DNA, 14 bp, Artificial
  synthetic DNA
tgcacatagtctca

SEQ ID NO: 992 - DNA, 14 bp, Artificial
  synthetic DNA
gtcaaggagtcacg

SEQ ID NO: 993 - DNA, 14 bp, Artificial
  synthetic DNA
ggttggaatcttgc

SEQ ID NO: 994 - DNA, 14 bp, Artificial
  synthetic DNA
catcggtgcactca

SEQ ID NO: 995 - DNA, 14 bp, Artificial
  synthetic DNA
aatgcactagacgt

SEQ ID NO: 996 - DNA, 14 bp, Artificial
  synthetic DNA
tacagtcaggctcg

SEQ ID NO: 997 - DNA, 14 bp, Artificial
  synthetic DNA
agagaagcttagcc

SEQ ID NO: 998 - DNA, 14 bp, Artificial
  synthetic DNA
ccataggatcgtat

SEQ ID NO: 999 - DNA, 14 bp, Artificial
  synthetic DNA
ttgtgctacacctg

SEQ ID NO: 1000 - DNA, 14 bp, Artificial
  synthetic DNA
ctccagtaatacta

SEQ ID NO: 1001 - DNA, 14 bp, Artificial
  synthetic DNA
tgatgccgatgtgg

SEQ ID NO: 1002 - DNA, 14 bp, Artificial
  synthetic DNA
gtcataccgcttaa

SEQ ID NO: 1003 - DNA, 14 bp, Artificial
  synthetic DNA
acgttctcttgaga

SEQ ID NO: 1004 - DNA, 14 bp, Artificial
  synthetic DNA
cagccatatcgtgt

SEQ ID NO: 1005 - DNA, 14 bp, Artificial
  synthetic DNA
ttgaacgtagcaat

SEQ ID NO: 1006 - DNA, 14 bp, Artificial
  synthetic DNA
acaatcgcggtaat

SEQ ID NO: 1007 - DNA, 14 bp, Artificial
  synthetic DNA
gttcctgtagatcc

SEQ ID NO: 1008 - DNA, 14 bp, Artificial
  synthetic DNA
agagccttacggca

SEQ ID NO: 1009 - DNA, 14 bp, Artificial
  synthetic DNA
aatatggcgccacc

SEQ ID NO: 1010 - DNA, 14 bp, Artificial
  synthetic DNA
accatataggttcg

SEQ ID NO: 1011 - DNA, 14 bp, Artificial
  synthetic DNA
atgcaccacagctg

SEQ ID NO: 1012 - DNA, 14 bp, Artificial
  synthetic DNA
ctactattgaacag

SEQ ID NO: 1013 - DNA, 14 bp, Artificial
  synthetic DNA
tgccatcactctag

SEQ ID NO: 1014 - DNA, 14 bp, Artificial
  synthetic DNA
gcgaacgagaatcg

SEQ ID NO: 1015 - DNA, 14 bp, Artificial
  synthetic DNA
gaatcaaggagacc

SEQ ID NO: 1016 - DNA, 14 bp, Artificial
  synthetic DNA
caacatctatgcag

SEQ ID NO: 1017 - DNA, 14 bp, Artificial
  synthetic DNA
caatccgtcatgga

SEQ ID NO: 1018 - DNA, 14 bp, Artificial
  synthetic DNA
agctcttagccata

SEQ ID NO: 1019 - DNA, 14 bp, Artificial
  synthetic DNA
aacaaggcaactgg

SEQ ID NO: 1020 - DNA, 14 bp, Artificial
  synthetic DNA
gtcgtcgctcctat

SEQ ID NO: 1021 - DNA, 14 bp, Artificial
  synthetic DNA
gtcatcattagatg

SEQ ID NO: 1022 - DNA, 14 bp, Artificial
  synthetic DNA
gcactaagtagcag

SEQ ID NO: 1023 - DNA, 14 bp, Artificial
  synthetic DNA
accttaccggacct

SEQ ID NO: 1024 - DNA, 14 bp, Artificial
  synthetic DNA
gctcaggtatgtca

SEQ ID NO: 1025 - DNA, 14 bp, Artificial
  synthetic DNA
tgtcacgagttagt

SEQ ID NO: 1026 - DNA, 14 bp, Artificial
  synthetic DNA
cagatgacttacgt

SEQ ID NO: 1027 - DNA, 14 bp, Artificial
  synthetic DNA
gaagtagcgattga

SEQ ID NO: 1028 - DNA, 14 bp, Artificial
  synthetic DNA
gcaggcaatctgta

SEQ ID NO: 1029 - DNA, 14 bp, Artificial
  synthetic DNA
ccttatacaacaag

SEQ ID NO: 1030 - DNA, 14 bp, Artificial
  synthetic DNA
ccttagattgattg

SEQ ID NO: 1031 - DNA, 14 bp, Artificial
  synthetic DNA
agccacgagtgata

SEQ ID NO: 1032 - DNA, 14 bp, Artificial
  synthetic DNA
ggatgactcgtgac

SEQ ID NO: 1033 - DNA, 14 bp, Artificial
  synthetic DNA
cttcgttcgccatt

SEQ ID NO: 1034 - DNA, 14 bp, Artificial
  synthetic DNA
tcttgcgtattgat

SEQ ID NO: 1035 - DNA, 14 bp, Artificial
  synthetic DNA
cttaacgtggtggc

SEQ ID NO: 1036 - DNA, 14 bp, Artificial
  synthetic DNA
tgctgttacggaag

SEQ ID NO: 1037 - DNA, 14 bp, Artificial
  synthetic DNA
ctgaattagttctc

SEQ ID NO: 1038 - DNA, 14 bp, Artificial
  synthetic DNA
cctccaagtacaga

SEQ ID NO: 1039 - DNA, 14 bp, Artificial
  synthetic DNA
ctggtaattcgcgg

SEQ ID NO: 1040 - DNA, 14 bp, Artificial
  synthetic DNA
cgactgcaatctgg

SEQ ID NO: 1041 - DNA, 14 bp, Artificial
  synthetic DNA
tggatcgcgattgg

SEQ ID NO: 1042 - DNA, 14 bp, Artificial
  synthetic DNA
cgactattcctgcg

SEQ ID NO: 1043 - DNA, 14 bp, Artificial
  synthetic DNA
caagtaggtccgtc

SEQ ID NO: 1044 - DNA, 14 bp, Artificial
  synthetic DNA
agtaatcagtgttc

SEQ ID NO: 1045 - DNA, 14 bp, Artificial
  synthetic DNA
ttattctcactacg

SEQ ID NO: 1046 - DNA, 14 bp, Artificial
  synthetic DNA
catgtcttcttcgt

SEQ ID NO: 1047 - DNA, 14 bp, Artificial
  synthetic DNA
aggcacataccatc

SEQ ID NO: 1048 - DNA, 14 bp, Artificial
  synthetic DNA
aggttagaggatgt

SEQ ID NO: 1049 - DNA, 14 bp, Artificial
  synthetic DNA
caactggcaagtgc

SEQ ID NO: 1050 - DNA, 14 bp, Artificial
  synthetic DNA
cgctcacatagagg

SEQ ID NO: 1051 - DNA, 14 bp, Artificial
  synthetic DNA
gcaatgtcgagatc

SEQ ID NO: 1052 - DNA, 14 bp, Artificial
  synthetic DNA
gttctgtggtgctc

SEQ ID NO: 1053 - DNA, 14 bp, Artificial
  synthetic DNA
aagtgatcagacta

SEQ ID NO: 1054 - DNA, 14 bp, Artificial
  synthetic DNA
attgaaggattcca

SEQ ID NO: 1055 - DNA, 14 bp, Artificial
  synthetic DNA
acgccatgctacta

SEQ ID NO: 1056 - DNA, 14 bp, Artificial
  synthetic DNA
ctgaagatgtctgc

SEQ ID NO: 1057 - DNA, 16 bp, Artificial
  synthetic DNA
gacaatctctgccgat

SEQ ID NO: 1058 - DNA, 16 bp, Artificial
  synthetic DNA
ggtccgcctaatgtaa

SEQ ID NO: 1059 - DNA, 16 bp, Artificial
  synthetic DNA
agccacaggcaattcc

SEQ ID NO: 1060 - DNA, 16 bp, Artificial
  synthetic DNA
atctcaagttctcaac

SEQ ID NO: 1061 - DNA, 16 bp, Artificial
  synthetic DNA
tgtaacgcatacgacg

SEQ ID NO: 1062 - DNA, 16 bp, Artificial
  synthetic DNA
tatctcgaataccagc

SEQ ID NO: 1063 - DNA, 16 bp, Artificial
  synthetic DNA
accgcaacacaggcaa

SEQ ID NO: 1064 - DNA, 16 bp, Artificial
  synthetic DNA
ggccagtaacatgact

SEQ ID NO: 1065 - DNA, 16 bp, Artificial
  synthetic DNA
gtgaacagttaaggtg

SEQ ID NO: 1066 - DNA, 16 bp, Artificial
  synthetic DNA
ccaggatccgtattgc

SEQ ID NO: 1067 - DNA, 16 bp, Artificial
  synthetic DNA
gacctagcactagacc

SEQ ID NO: 1068 - DNA, 16 bp, Artificial
  synthetic DNA
cgccatcctattcacg

SEQ ID NO: 1069 - DNA, 16 bp, Artificial
  synthetic DNA
aagtgcagtaatggaa

SEQ ID NO: 1070 - DNA, 16 bp, Artificial
  synthetic DNA
tcaacgcgttcgtcta

SEQ ID NO: 1071 - DNA, 16 bp, Artificial
  synthetic DNA
agcggccactatctaa

SEQ ID NO: 1072 - DNA, 16 bp, Artificial
  synthetic DNA
ctcggcgccatataga

SEQ ID NO: 1073 - DNA, 16 bp, Artificial
  synthetic DNA
cgataacttagaagaa

SEQ ID NO: 1074 - DNA, 16 bp, Artificial
  synthetic DNA
cataggatgtgacgcc

SEQ ID NO: 1075 - DNA, 16 bp, Artificial
  synthetic DNA
ggcttgtcgtcgtatc

SEQ ID NO: 1076 - DNA, 16 bp, Artificial
  synthetic DNA
cttgtctgaatattag

SEQ ID NO: 1077 - DNA, 16 bp, Artificial
  synthetic DNA
acagttcgagtgtcgg

SEQ ID NO: 1078 - DNA, 16 bp, Artificial
  synthetic DNA
ctctaacctgtgacgt

SEQ ID NO: 1079 - DNA, 16 bp, Artificial
  synthetic DNA
cgcgctaattcaacaa

SEQ ID NO: 1080 - DNA, 16 bp, Artificial
  synthetic DNA
actcacgaatgcggca

SEQ ID NO: 1081 - DNA, 16 bp, Artificial
  synthetic DNA
aatcttcggcattcat

SEQ ID NO: 1082 - DNA, 16 bp, Artificial
  synthetic DNA
aagtatcaggatcgcg

SEQ ID NO: 1083 - DNA, 16 bp, Artificial
  synthetic DNA
agtaactctgcagaca

SEQ ID NO: 1084 - DNA, 16 bp, Artificial
  synthetic DNA
ggattgaacattgtgc

SEQ ID NO: 1085 - DNA, 16 bp, Artificial
  synthetic DNA
gtgatgctcacgcatc

SEQ ID NO: 1086 - DNA, 16 bp, Artificial
  synthetic DNA
cgtagcgtaacggata

SEQ ID NO: 1087 - DNA, 16 bp, Artificial
  synthetic DNA
tgcgatgcaccgttag

SEQ ID NO: 1088 - DNA, 16 bp, Artificial
  synthetic DNA
ccagtatgctctcagg

SEQ ID NO: 1089 - DNA, 16 bp, Artificial
  synthetic DNA
aatgacgttgaagcct

SEQ ID NO: 1090 - DNA, 16 bp, Artificial
  synthetic DNA
tcgattctataggagt

SEQ ID NO: 1091 - DNA, 16 bp, Artificial
  synthetic DNA
cgataggttcagctat

SEQ ID NO: 1092 - DNA, 16 bp, Artificial
  synthetic DNA
ccatgttgatagaata

SEQ ID NO: 1093 - DNA, 16 bp, Artificial
  synthetic DNA
gagccacttctacagg

SEQ ID NO: 1094 - DNA, 16 bp, Artificial
  synthetic DNA
gcgaactctcggtaat

SEQ ID NO: 1095 - DNA, 16 bp, Artificial
  synthetic DNA
gacctgagtagctggt

SEQ ID NO: 1096 - DNA, 16 bp, Artificial
  synthetic DNA
cgagtctattagcctg

SEQ ID NO: 1097 - DNA, 16 bp, Artificial
  synthetic DNA
gtagtgccatacacct

SEQ ID NO: 1098 - DNA, 16 bp, Artificial
  synthetic DNA
ccagtggtctatagca

SEQ ID NO: 1099 - DNA, 16 bp, Artificial
  synthetic DNA
gtcagtgcgttattgc

SEQ ID NO: 1100 - DNA, 16 bp, Artificial
  synthetic DNA
agtgtcggagtgacga

SEQ ID NO: 1101 - DNA, 16 bp, Artificial
  synthetic DNA
aatctccgctatagtt

SEQ ID NO: 1102 - DNA, 16 bp, Artificial
  synthetic DNA
cgagtaggtctgactt

SEQ ID NO: 1103 - DNA, 16 bp, Artificial
  synthetic DNA
ctgtcgctctaataac

SEQ ID NO: 1104 - DNA, 16 bp, Artificial
  synthetic DNA
gctgtcaatataactg

SEQ ID NO: 1105 - DNA, 16 bp, Artificial
  synthetic DNA
agctcaagttgaatcc

SEQ ID NO: 1106 - DNA, 16 bp, Artificial
  synthetic DNA
aattcatgctcctaac

SEQ ID NO: 1107 - DNA, 16 bp, Artificial
  synthetic DNA
ccaaggtctggtgata

SEQ ID NO: 1108 - DNA, 16 bp, Artificial
  synthetic DNA
ctccacgtatcttgaa

SEQ ID NO: 1109 - DNA, 16 bp, Artificial
  synthetic DNA
tagccgaacaacactt

SEQ ID NO: 1110 - DNA, 16 bp, Artificial
  synthetic DNA
agtacacgacatatgc

SEQ ID NO: 1111 - DNA, 16 bp, Artificial
  synthetic DNA
acgttctagactcctg

SEQ ID NO: 1112 - DNA, 16 bp, Artificial
  synthetic DNA
cgactcaagcactgct

SEQ ID NO: 1113 - DNA, 16 bp, Artificial
  synthetic DNA
tgaagctcacgattaa

SEQ ID NO: 1114 - DNA, 16 bp, Artificial
  synthetic DNA
tatctaacgtatggta

SEQ ID NO: 1115 - DNA, 16 bp, Artificial
  synthetic DNA
tataccatgttccttg

SEQ ID NO: 1116 - DNA, 16 bp, Artificial
  synthetic DNA
ttcctacgatgacttc

SEQ ID NO: 1117 - DNA, 16 bp, Artificial
  synthetic DNA
ctctccaatatgtgcc

SEQ ID NO: 1118 - DNA, 16 bp, Artificial
  synthetic DNA
gagtagagtcttgcca

SEQ ID NO: 1119 - DNA, 16 bp, Artificial
  synthetic DNA
gcgagatgtggtccta

SEQ ID NO: 1120 - DNA, 16 bp, Artificial
  synthetic DNA
aagctacacggaccac

SEQ ID NO: 1121 - DNA, 16 bp, Artificial
  synthetic DNA
atacaactggcaaccg

SEQ ID NO: 1122 - DNA, 16 bp, Artificial
  synthetic DNA
cggtagatgctatgct

SEQ ID NO: 1123 - DNA, 16 bp, Artificial
  synthetic DNA
tcttgaccggtcatca

SEQ ID NO: 1124 - DNA, 16 bp, Artificial
  synthetic DNA
agatcgtgcatgcgat

SEQ ID NO: 1125 - DNA, 16 bp, Artificial
  synthetic DNA
tcctcgagacagcctt

SEQ ID NO: 1126 - DNA, 16 bp, Artificial
  synthetic DNA
tagccggtaccactta

SEQ ID NO: 1127 - DNA, 16 bp, Artificial
  synthetic DNA
gtaaggcagcgtgcaa

SEQ ID NO: 1128 - DNA, 16 bp, Artificial
  synthetic DNA
tagtctgctcctggtc

SEQ ID NO: 1129 - DNA, 16 bp, Artificial
  synthetic DNA
tggattatagcagcag

SEQ ID NO: 1130 - DNA, 16 bp, Artificial
  synthetic DNA
aagaatgatcagacat

SEQ ID NO: 1131 - DNA, 16 bp, Artificial
  synthetic DNA
cagcgctatatacctc

SEQ ID NO: 1132 - DNA, 16 bp, Artificial
  synthetic DNA
gagtagtacctccacc

SEQ ID NO: 1133 - DNA, 16 bp, Artificial
  synthetic DNA
gacgtgatcctctaga

SEQ ID NO: 1134 - DNA, 16 bp, Artificial
  synthetic DNA
gttccgttcactacga

SEQ ID NO: 1135 - DNA, 16 bp, Artificial
  synthetic DNA
tgcaagcaccaggatg

SEQ ID NO: 1136 - DNA, 16 bp, Artificial
  synthetic DNA
ttagttggcggctgag

SEQ ID NO: 1137 - DNA, 16 bp, Artificial
  synthetic DNA
cagatgcagacatacg

SEQ ID NO: 1138 - DNA, 16 bp, Artificial
  synthetic DNA
gacgcttgatgattat

SEQ ID NO: 1139 - DNA, 16 bp, Artificial
  synthetic DNA
tggatcacgactagga

SEQ ID NO: 1140 - DNA, 16 bp, Artificial
  synthetic DNA
ctcgtcggtataacgc

SEQ ID NO: 1141 - DNA, 16 bp, Artificial
  synthetic DNA
aagcacggatgcgatt

SEQ ID NO: 1142 - DNA, 16 bp, Artificial
  synthetic DNA
agatcttccggtgaac

SEQ ID NO: 1143 - DNA, 16 bp, Artificial
  synthetic DNA
ggacaatagcaacctg

SEQ ID NO: 1144 - DNA, 16 bp, Artificial
  synthetic DNA
gataatcggttccaat

SEQ ID NO: 1145 - DNA, 16 bp, Artificial
  synthetic DNA
ctcaagctacagttgt

SEQ ID NO: 1146 - DNA, 16 bp, Artificial
  synthetic DNA
gttggcatgatgtaga

SEQ ID NO: 1147 - DNA, 16 bp, Artificial
  synthetic DNA
cagcatgaggtaagtg

SEQ ID NO: 1148 - DNA, 16 bp, Artificial
  synthetic DNA
gcctcatcacacgtca

SEQ ID NO: 1149 - DNA, 16 bp, Artificial
  synthetic DNA
tcgatactacacatcg

SEQ ID NO: 1150 - DNA, 16 bp, Artificial
  synthetic DNA
tacacgaggcttgatc

SEQ ID NO: 1151 - DNA, 16 bp, Artificial
  synthetic DNA
ttctcgtgtccgcatt

SEQ ID NO: 1152 - DNA, 16 bp, Artificial
  synthetic DNA
ggtgaagcaacagcat

SEQ ID NO: 1153 - DNA, 18 bp, Artificial
  synthetic DNA
cgaaccgactgtacagtt

SEQ ID NO: 1154 - DNA, 18 bp, Artificial
  synthetic DNA
ccgactgcggataagtta

SEQ ID NO: 1155 - DNA, 18 bp, Artificial
  synthetic DNA
cgacaggtaggtaagcag

SEQ ID NO: 1156 - DNA, 18 bp, Artificial
  synthetic DNA
tgatacgttggtatacag

SEQ ID NO: 1157 - DNA, 18 bp, Artificial
  synthetic DNA
ctactatagaatacgtag

SEQ ID NO: 1158 - DNA, 18 bp, Artificial
  synthetic DNA
agactgtggcaatggcat

SEQ ID NO: 1159 - DNA, 18 bp, Artificial
  synthetic DNA
ggaagactgatacaacga

SEQ ID NO: 1160 - DNA, 18 bp, Artificial
  synthetic DNA
tatgcacatatagcgctt

SEQ ID NO: 1161 - DNA, 18 bp, Artificial
  synthetic DNA
catggtaatcgaccgagg

SEQ ID NO: 1162 - DNA, 18 bp, Artificial
  synthetic DNA
gtcattgccgtcattgcc

SEQ ID NO: 1163 - DNA, 18 bp, Artificial
  synthetic DNA
cctaagaactccgaagct

SEQ ID NO: 1164 - DNA, 18 bp, Artificial
  synthetic DNA
tcgctcaccgtactagga

SEQ ID NO: 1165 - DNA, 18 bp, Artificial
  synthetic DNA
tattactgtcacagcagg

SEQ ID NO: 1166 - DNA, 18 bp, Artificial
  synthetic DNA
tgagacaggctacgagtc

SEQ ID NO: 1167 - DNA, 18 bp, Artificial
  synthetic DNA
aagctatgcgaacacgtt

SEQ ID NO: 1168 - DNA, 18 bp, Artificial
  synthetic DNA
aacggaggagtgagccaa

SEQ ID NO: 1169 - DNA, 18 bp, Artificial
  synthetic DNA
ccactatggacatcatgg

SEQ ID NO: 1170 - DNA, 18 bp, Artificial
  synthetic DNA
atggtggtggatagctcg

SEQ ID NO: 1171 - DNA, 18 bp, Artificial
  synthetic DNA
tcaccggttacacatcgc

SEQ ID NO: 1172 - DNA, 18 bp, Artificial
  synthetic DNA
aagatactgagatatgga

SEQ ID NO: 1173 - DNA, 18 bp, Artificial
  synthetic DNA
gacctgttcttgaactag

SEQ ID NO: 1174 - DNA, 18 bp, Artificial
  synthetic DNA
aagtagagctctcggtta

SEQ ID NO: 1175 - DNA, 18 bp, Artificial
  synthetic DNA
ctatgttcttactctctt

SEQ ID NO: 1176 - DNA, 18 bp, Artificial
  synthetic DNA
caaggctataagcggtta

SEQ ID NO: 1177 - DNA, 18 bp, Artificial
  synthetic DNA
gaagctaattaaccgata

SEQ ID NO: 1178 - DNA, 18 bp, Artificial
  synthetic DNA
ttcacgtctgccaagcac

SEQ ID NO: 1179 - DNA, 18 bp, Artificial
  synthetic DNA
atcgtatagatcgagaca

SEQ ID NO: 1180 - DNA, 18 bp, Artificial
  synthetic DNA
gtcacagattcacatcat

SEQ ID NO: 1181 - DNA, 18 bp, Artificial
  synthetic DNA
gtgcctgtgaactatcag

SEQ ID NO: 1182 - DNA, 18 bp, Artificial
  synthetic DNA
cagcgtacaagatagtcg

SEQ ID NO: 1183 - DNA, 18 bp, Artificial
  synthetic DNA
gcatggcatggtagacct

SEQ ID NO: 1184 - DNA, 18 bp, Artificial
  synthetic DNA
ggtatgctactcttcgca

SEQ ID NO: 1185 - DNA, 18 bp, Artificial
  synthetic DNA
atgttcagtcacaagcga

SEQ ID NO: 1186 - DNA, 18 bp, Artificial
  synthetic DNA
taggaagtgtgtaatagc

SEQ ID NO: 1187 - DNA, 18 bp, Artificial
  synthetic DNA
aatccatgtagctgtacg

SEQ ID NO: 1188 - DNA, 18 bp, Artificial
  synthetic DNA
ccagattcactggcatag

SEQ ID NO: 1189 - DNA, 18 bp, Artificial
  synthetic DNA
ttgtctctacgtaatatc

SEQ ID NO: 1190 - DNA, 18 bp, Artificial
  synthetic DNA
gtggtgcttgtgacaatt

SEQ ID NO: 1191 - DNA, 18 bp, Artificial
  synthetic DNA
cagcctacttggctgaga

SEQ ID NO: 1192 - DNA, 18 bp, Artificial
  synthetic DNA
tactcaatgcatctgtgt

SEQ ID NO: 1193 - DNA, 18 bp, Artificial
  synthetic DNA
tgtagagagacgaatata

SEQ ID NO: 1194 - DNA, 18 bp, Artificial
  synthetic DNA
gcctacaaccatcctact

SEQ ID NO: 1195 - DNA, 18 bp, Artificial
  synthetic DNA
gcgtggcattgagattca

SEQ ID NO: 1196 - DNA, 18 bp, Artificial
  synthetic DNA
gcatgccagctaactgag

SEQ ID NO: 1197 - DNA, 18 bp, Artificial
  synthetic DNA
gcgagtaatccggttgga

SEQ ID NO: 1198 - DNA, 18 bp, Artificial
  synthetic DNA
gcctctaccagaacgtca

SEQ ID NO: 1199 - DNA, 18 bp, Artificial
  synthetic DNA
gtcagcagaagactgacc

SEQ ID NO: 1200 - DNA, 18 bp, Artificial
  synthetic DNA
gataacagacgtagcagg

SEQ ID NO: 1201 - DNA, 18 bp, Artificial
  synthetic DNA
caggagatcgcatgtcgt

SEQ ID NO: 1202 - DNA, 18 bp, Artificial
  synthetic DNA
ctggaaggaatggagcca

SEQ ID NO: 1203 - DNA, 18 bp, Artificial
  synthetic DNA
attggttctctaccacaa

SEQ ID NO: 1204 - DNA, 18 bp, Artificial
  synthetic DNA
ctcattgttgacggctca

SEQ ID NO: 1205 - DNA, 18 bp, Artificial
  synthetic DNA
ttcaggactgtagttcat

SEQ ID NO: 1206 - DNA, 18 bp, Artificial
  synthetic DNA
agaccgcactaactcaag

SEQ ID NO: 1207 - DNA, 18 bp, Artificial
  synthetic DNA
ggaatattgtgcagaccg

SEQ ID NO: 1208 - DNA, 18 bp, Artificial
  synthetic DNA
cctattactaatagctca

SEQ ID NO: 1209 - DNA, 18 bp, Artificial
  synthetic DNA
atggcatgagtacttcgg

SEQ ID NO: 1210 - DNA, 18 bp, Artificial
  synthetic DNA
gacacgtatgcgtctagc

SEQ ID NO: 1211 - DNA, 18 bp, Artificial
  synthetic DNA
gaaggtacggaatctgtt

SEQ ID NO: 1212 - DNA, 18 bp, Artificial
  synthetic DNA
tataacgtccgacactgt

SEQ ID NO: 1213 - DNA, 18 bp, Artificial
  synthetic DNA
gctaatacattaccgccg

SEQ ID NO: 1214 - DNA, 18 bp, Artificial
  synthetic DNA
gaagccaacactcctgac

SEQ ID NO: 1215 - DNA, 18 bp, Artificial
  synthetic DNA
cgaataacgagctgtgat

SEQ ID NO: 1216 - DNA, 18 bp, Artificial
  synthetic DNA
gcctaccgatcgcactta

SEQ ID NO: 1217 - DNA, 18 bp, Artificial
  synthetic DNA
ctgaggagaatagcctgc

SEQ ID NO: 1218 - DNA, 18 bp, Artificial
  synthetic DNA
cagcatggacagtacttc

SEQ ID NO: 1219 - DNA, 18 bp, Artificial
  synthetic DNA
ggtatagagccttcctta

SEQ ID NO: 1220 - DNA, 18 bp, Artificial
  synthetic DNA
cgctctgcatatatagca

SEQ ID NO: 1221 - DNA, 18 bp, Artificial
  synthetic DNA
cggctctactatgctcgt

SEQ ID NO: 1222 - DNA, 18 bp, Artificial
  synthetic DNA
cctaatgcgaagctcacc

SEQ ID NO: 1223 - DNA, 18 bp, Artificial
  synthetic DNA
acaaccggtgaggcagta

SEQ ID NO: 1224 - DNA, 18 bp, Artificial
  synthetic DNA
ttggttcgaaccaaccgc

SEQ ID NO: 1225 - DNA, 18 bp, Artificial
  synthetic DNA
atactaggttgaactaag

SEQ ID NO: 1226 - DNA, 18 bp, Artificial
  synthetic DNA
gcgttgagagtaacatat

SEQ ID NO: 1227 - DNA, 18 bp, Artificial
  synthetic DNA
agttgtataataagcgtc

SEQ ID NO: 1228 - DNA, 18 bp, Artificial
  synthetic DNA
gtatgatgccgtccaatt

SEQ ID NO: 1229 - DNA, 18 bp, Artificial
  synthetic DNA
ggactctctgaagagtct

SEQ ID NO: 1230 - DNA, 18 bp, Artificial
  synthetic DNA
ggactctcttgacttgaa

SEQ ID NO: 1231 - DNA, 18 bp, Artificial
  synthetic DNA
gataacagtgcttcgtcc

SEQ ID NO: 1232 - DNA, 18 bp, Artificial
  synthetic DNA
ggccattatagatgaact

SEQ ID NO: 1233 - DNA, 18 bp, Artificial
  synthetic DNA
atagagagcacagagcag

SEQ ID NO: 1234 - DNA, 18 bp, Artificial
  synthetic DNA
gtgtgagtgtatcataac

SEQ ID NO: 1235 - DNA, 18 bp, Artificial
  synthetic DNA
ataaccttagtgcgcgtc

SEQ ID NO: 1236 - DNA, 18 bp, Artificial
  synthetic DNA
ccgactgatatgcatgga

SEQ ID NO: 1237 - DNA, 18 bp, Artificial
  synthetic DNA
ggatatctgatcgcatca

SEQ ID NO: 1238 - DNA, 18 bp, Artificial
  synthetic DNA
cagcattaacgaggcgaa

SEQ ID NO: 1239 - DNA, 18 bp, Artificial
  synthetic DNA
gcgaggcctacatattcg

SEQ ID NO: 1240 - DNA, 18 bp, Artificial
  synthetic DNA
cgataagtggtaaggtct

SEQ ID NO: 1241 - DNA, 18 bp, Artificial
  synthetic DNA
agatcctgagtcgagcaa

SEQ ID NO: 1242 - DNA, 18 bp, Artificial
  synthetic DNA
aagatataacgagaccga

SEQ ID NO: 1243 - DNA, 18 bp, Artificial
  synthetic DNA
ccgactgattgagaacgt

SEQ ID NO: 1244 - DNA, 18 bp, Artificial
  synthetic DNA
tcggcttatatgacacgt

SEQ ID NO: 1245 - DNA, 18 bp, Artificial
  synthetic DNA
aataacgtacgccggagg

SEQ ID NO: 1246 - DNA, 18 bp, Artificial
  synthetic DNA
aacacagcattgcgcacg

SEQ ID NO: 1247 - DNA, 18 bp, Artificial
  synthetic DNA
gtagtctgacagcaacaa

SEQ ID NO: 1248 - DNA, 18 bp, Artificial
  synthetic DNA
agaatgacttgagctgct

SEQ ID NO: 1249 - DNA, 20 bp, Artificial
  synthetic DNA
actggtagtaacgtccacct

SEQ ID NO: 1250 - DNA, 20 bp, Artificial
  synthetic DNA
agactggttgttattcgcct

SEQ ID NO: 1251 - DNA, 20 bp, Artificial
  synthetic DNA
tatcattgacagcgagctca

SEQ ID NO: 1252 - DNA, 20 bp, Artificial
  synthetic DNA
tggagtctgaagaaggactc

SEQ ID NO: 1253 - DNA, 20 bp, Artificial
  synthetic DNA
catctggactacggcaacga

SEQ ID NO: 1254 - DNA, 20 bp, Artificial
  synthetic DNA
aactgtcataagacagacaa

SEQ ID NO: 1255 - DNA, 20 bp, Artificial
  synthetic DNA
cctcaacatgacatacaccg

SEQ ID NO: 1256 - DNA, 20 bp, Artificial
  synthetic DNA
caataccgttcgcgattcta

SEQ ID NO: 1257 - DNA, 20 bp, Artificial
  synthetic DNA
gcgtctacgttgattcggcc

SEQ ID NO: 1258 - DNA, 20 bp, Artificial
  synthetic DNA
tgaacagaggcacttgcagg

SEQ ID NO: 1259 - DNA, 20 bp, Artificial
  synthetic DNA
cgactagaacctactactgc

SEQ ID NO: 1260 - DNA, 20 bp, Artificial
  synthetic DNA
gcaccgcacgtggagagata

SEQ ID NO: 1261 - DNA, 20 bp, Artificial
  synthetic DNA
ctgagagaccgactgatgcg

SEQ ID NO: 1262 - DNA, 20 bp, Artificial
  synthetic DNA
tcgtccttctacttaatgat

SEQ ID NO: 1263 - DNA, 20 bp, Artificial
  synthetic DNA
caagctataccatccgaatt

SEQ ID NO: 1264 - DNA, 20 bp, Artificial
  synthetic DNA
caatacgtatagtcttagat

SEQ ID NO: 1265 - DNA, 20 bp, Artificial
  synthetic DNA
ccatccacagtgacctatgt

SEQ ID NO: 1266 - DNA, 20 bp, Artificial
  synthetic DNA
tatccgttggagaaggttca

SEQ ID NO: 1267 - DNA, 20 bp, Artificial
  synthetic DNA
cgcctaggtacctgagtacg

SEQ ID NO: 1268 - DNA, 20 bp, Artificial
  synthetic DNA
cagagtgctcgtgttcgcga

SEQ ID NO: 1269 - DNA, 20 bp, Artificial
  synthetic DNA
cgcttggacatccttaagaa

SEQ ID NO: 1270 - DNA, 20 bp, Artificial
  synthetic DNA
gaccgcatgattagtcttac

SEQ ID NO: 1271 - DNA, 20 bp, Artificial
  synthetic DNA
cttggccgtagtcactcagt

SEQ ID NO: 1272 - DNA, 20 bp, Artificial
  synthetic DNA
gatagcgatattcagttcgc

SEQ ID NO: 1273 - DNA, 20 bp, Artificial
  synthetic DNA
atccaacactaagacaacca

SEQ ID NO: 1274 - DNA, 20 bp, Artificial
  synthetic DNA
ccattctgttgcgtgtcctc

SEQ ID NO: 1275 - DNA, 20 bp, Artificial
  synthetic DNA
acattctgtacgcttgcagc

SEQ ID NO: 1276 - DNA, 20 bp, Artificial
  synthetic DNA
tgctgaacgccaatcgctta

SEQ ID NO: 1277 - DNA, 20 bp, Artificial
  synthetic DNA
tcctctacaagaatattgcg

SEQ ID NO: 1278 - DNA, 20 bp, Artificial
  synthetic DNA
cgaccaacgcagcctgattc

SEQ ID NO: 1279 - DNA, 20 bp, Artificial
  synthetic DNA
attgcgagcttgagtagcgc

SEQ ID NO: 1280 - DNA, 20 bp, Artificial
  synthetic DNA
aaggtgcgagcataggaatc

SEQ ID NO: 1281 - DNA, 20 bp, Artificial
  synthetic DNA
cacttaagtgtgatatagat

SEQ ID NO: 1282 - DNA, 20 bp, Artificial
  synthetic DNA
atcggtatgctgacctagac

SEQ ID NO: 1283 - DNA, 20 bp, Artificial
  synthetic DNA
tacaatctcgaatgcaggat

SEQ ID NO: 1284 - DNA, 20 bp, Artificial
  synthetic DNA
ccatatgaagcgcagccgtc

SEQ ID NO: 1285 - DNA, 20 bp, Artificial
  synthetic DNA
cgtctcgtggacattcgagg

SEQ ID NO: 1286 - DNA, 20 bp, Artificial
  synthetic DNA
ccgagtacagaagcgtggaa

SEQ ID NO: 1287 - DNA, 20 bp, Artificial
  synthetic DNA
ttacgtggtcgacaggcagt

SEQ ID NO: 1288 - DNA, 20 bp, Artificial
  synthetic DNA
agctgcaatctgcatgatta

SEQ ID NO: 1289 - DNA, 20 bp, Artificial
  synthetic DNA
acctgccgaagcagcctaca

SEQ ID NO: 1290 - DNA, 20 bp, Artificial
  synthetic DNA
aacatgataaccacatggtt

SEQ ID NO: 1291 - DNA, 20 bp, Artificial
  synthetic DNA
atccgactgattgaattacc

SEQ ID NO: 1292 - DNA, 20 bp, Artificial
  synthetic DNA
tcacgctgactcttatcagg

SEQ ID NO: 1293 - DNA, 20 bp, Artificial
  synthetic DNA
gcgcgctcgaagtacaacat

SEQ ID NO: 1294 - DNA, 20 bp, Artificial
  synthetic DNA
acagccagatgcgttgttcc

SEQ ID NO: 1295 - DNA, 20 bp, Artificial
  synthetic DNA
ggagctctgacctgcaagaa

SEQ ID NO: 1296 - DNA, 20 bp, Artificial
  synthetic DNA
aacattagcctcaagtaaga

SEQ ID NO: 1297 - DNA, 20 bp, Artificial
  synthetic DNA
tgtgattatgccgaatgagg

SEQ ID NO: 1298 - DNA, 20 bp, Artificial
  synthetic DNA
gagtaataatccaatcagta

SEQ ID NO: 1299 - DNA, 20 bp, Artificial
  synthetic DNA
ctccttggcgacagctgaac

SEQ ID NO: 1300 - DNA, 20 bp, Artificial
  synthetic DNA
ttacgcacacatacacagac

SEQ ID NO: 1301 - DNA, 20 bp, Artificial
  synthetic DNA
acgccgtatggcgacttagg

SEQ ID NO: 1302 - DNA, 20 bp, Artificial
  synthetic DNA
agaacgacaattacgatggc

SEQ ID NO: 1303 - DNA, 20 bp, Artificial
  synthetic DNA
tgctaacgtaccactgccac

SEQ ID NO: 1304 - DNA, 20 bp, Artificial
  synthetic DNA
catccagaatgtctatcata

SEQ ID NO: 1305 - DNA, 20 bp, Artificial
  synthetic DNA
ggagaacgcctatagcactc

SEQ ID NO: 1306 - DNA, 20 bp, Artificial
  synthetic DNA
acctcttgtgacggccagtc

SEQ ID NO: 1307 - DNA, 20 bp, Artificial
  synthetic DNA
tgccataacttggcataaga

SEQ ID NO: 1308 - DNA, 20 bp, Artificial
  synthetic DNA
acaattgtctgaccacgctc

SEQ ID NO: 1309 - DNA, 20 bp, Artificial
  synthetic DNA
tcgtcaccttcacagaacga

SEQ ID NO: 1310 - DNA, 20 bp, Artificial
  synthetic DNA
agcagcagatgatgatccaa

SEQ ID NO: 1311 - DNA, 20 bp, Artificial
  synthetic DNA
tcgtgccttggattccagga

SEQ ID NO: 1312 - DNA, 20 bp, Artificial
  synthetic DNA
tgttatagccacgatactat

SEQ ID NO: 1313 - DNA, 20 bp, Artificial
  synthetic DNA
aatctcacctgtaccttccg

SEQ ID NO: 1314 - DNA, 20 bp, Artificial
  synthetic DNA
gagtagcggaagcgttagcg

SEQ ID NO: 1315 - DNA, 20 bp, Artificial
  synthetic DNA
aatactccggcgaggtatac

SEQ ID NO: 1316 - DNA, 20 bp, Artificial
  synthetic DNA
ttcgcatccttgcacgaaca

SEQ ID NO: 1317 - DNA, 20 bp, Artificial
  synthetic DNA
aaccggctaatactactggc

SEQ ID NO: 1318 - DNA, 20 bp, Artificial
  synthetic DNA
ctagcatcttagacaccaga

SEQ ID NO: 1319 - DNA, 20 bp, Artificial
  synthetic DNA
tagttgcgtgatacaagata

SEQ ID NO: 1320 - DNA, 20 bp, Artificial
  synthetic DNA
tcgtctcgacacagttggtc

SEQ ID NO: 1321 - DNA, 20 bp, Artificial
  synthetic DNA
tccgttcgcgtgcgaactga

SEQ ID NO: 1322 - DNA, 20 bp, Artificial
  synthetic DNA
tctgactctggtgtacagtc

SEQ ID NO: 1323 - DNA, 20 bp, Artificial
  synthetic DNA
acagcgcaattatatcctgt

SEQ ID NO: 1324 - DNA, 20 bp, Artificial
  synthetic DNA
agatccgtacgtgagactag

SEQ ID NO: 1325 - DNA, 20 bp, Artificial
  synthetic DNA
tacattgaagcatccgaaca

SEQ ID NO: 1326 - DNA, 20 bp, Artificial
  synthetic DNA
ctcctgagagatcaacgcca

SEQ ID NO: 1327 - DNA, 20 bp, Artificial
  synthetic DNA
tcacctcgaatgagttcgtt

SEQ ID NO: 1328 - DNA, 20 bp, Artificial
  synthetic DNA
tagcgacttaaggtccaagc

SEQ ID NO: 1329 - DNA, 20 bp, Artificial
  synthetic DNA
agtacgtattgccgtgcaag

SEQ ID NO: 1330 - DNA, 20 bp, Artificial
  synthetic DNA
agccacgaaccgacgtcata

SEQ ID NO: 1331 - DNA, 20 bp, Artificial
  synthetic DNA
tgatgtgtacgctactacta

SEQ ID NO: 1332 - DNA, 20 bp, Artificial
  synthetic DNA
ccactgtgtgcagcagacga

SEQ ID NO: 1333 - DNA, 20 bp, Artificial
  synthetic DNA
ctattgtacagcgaacgctg

SEQ ID NO: 1334 - DNA, 20 bp, Artificial
  synthetic DNA
ctccgatatcgcacggatcg

SEQ ID NO: 1335 - DNA, 20 bp, Artificial
  synthetic DNA
aacttatcgtcggacgcatg

SEQ ID NO: 1336 - DNA, 20 bp, Artificial
  synthetic DNA
tatcctaattcgtgccggtc

SEQ ID NO: 1337 - DNA, 20 bp, Artificial
  synthetic DNA
acagccttcctgtgtggact

SEQ ID NO: 1338 - DNA, 20 bp, Artificial
  synthetic DNA
cctccgtgaggatcgtacca

SEQ ID NO: 1339 - DNA, 20 bp, Artificial
  synthetic DNA
gctctaagtaacagaactaa

SEQ ID NO: 1340 - DNA, 20 bp, Artificial
  synthetic DNA
gacttaccgcgcgttctggt

SEQ ID NO: 1341 - DNA, 20 bp, Artificial
  synthetic DNA
tctgaggatacacatgtgga

SEQ ID NO: 1342 - DNA, 20 bp, Artificial
  synthetic DNA
tgtaatcacactggtgtcgg

SEQ ID NO: 1343 - DNA, 20 bp, Artificial
  synthetic DNA
cactaggcggcagacataca

SEQ ID NO: 1344 - DNA, 20 bp, Artificial
  synthetic DNA
ctagagcacagtaccacgtt

SEQ ID NO: 1345 - DNA, 22 bp, Artificial
  synthetic DNA
ttcagaggtctacgcttccggt

SEQ ID NO: 1346 - DNA, 22 bp, Artificial
  synthetic DNA
aacacagactgcgttatgccaa

SEQ ID NO: 1347 - DNA, 22 bp, Artificial
  synthetic DNA
tgctgagttctatacagcagtg

SEQ ID NO: 1348 - DNA, 22 bp, Artificial
  synthetic DNA
acctattatatgatagcgtcat

SEQ ID NO: 1349 - DNA, 22 bp, Artificial
  synthetic DNA
atcgtgagctacagtgaatgca

SEQ ID NO: 1350 - DNA, 22 bp, Artificial
  synthetic DNA
cgtgatgtatccggccttgcag

SEQ ID NO: 1351 - DNA, 22 bp, Artificial
  synthetic DNA
tcttctggtcctagagttgtgc

SEQ ID NO: 1352 - DNA, 22 bp, Artificial
  synthetic DNA
tgatgtcggcggcggatcagat

SEQ ID NO: 1353 - DNA, 22 bp, Artificial
  synthetic DNA
tcggccttagcgttcagcatcc

SEQ ID NO: 1354 - DNA, 22 bp, Artificial
  synthetic DNA
ttaagtaggtcagccactgcac

SEQ ID NO: 1355 - DNA, 22 bp, Artificial
  synthetic DNA
ccaggtgagttgatctgacacc

SEQ ID NO: 1356 - DNA, 22 bp, Artificial
  synthetic DNA
tatactattactgtgttcgatc

SEQ ID NO: 1357 - DNA, 22 bp, Artificial
  synthetic DNA
ccgcagtatgtctagtgttgtc

SEQ ID NO: 1358 - DNA, 22 bp, Artificial
  synthetic DNA
gtctaccgcgtacgaagctctc

SEQ ID NO: 1359 - DNA, 22 bp, Artificial
  synthetic DNA
atgcgagtccgtggtcgatcct

SEQ ID NO: 1360 - DNA, 22 bp, Artificial
  synthetic DNA
tggtagattggtgtgagaacta

SEQ ID NO: 1361 - DNA, 22 bp, Artificial
  synthetic DNA
aggttcgtcgatcaactgctaa

SEQ ID NO: 1362 - DNA, 22 bp, Artificial
  synthetic DNA
acgacaagcatcctgcgatatc

SEQ ID NO: 1363 - DNA, 22 bp, Artificial
  synthetic DNA
ttgaatcacagagagcgtgatt

SEQ ID NO: 1364 - DNA, 22 bp, Artificial
  synthetic DNA
gtacttagtgcttacgtcagct

SEQ ID NO: 1365 - DNA, 22 bp, Artificial
  synthetic DNA
gattattaaggccaagctcata

SEQ ID NO: 1366 - DNA, 22 bp, Artificial
  synthetic DNA
gcatgcagagacgtactcatcg

SEQ ID NO: 1367 - DNA, 22 bp, Artificial
  synthetic DNA
tagcggatggtgtcctggcact

SEQ ID NO: 1368 - DNA, 22 bp, Artificial
  synthetic DNA
tacggctgccaacttaataact

SEQ ID NO: 1369 - DNA, 22 bp, Artificial
  synthetic DNA
ctcatatgacaacttctatagt

SEQ ID NO: 1370 - DNA, 22 bp, Artificial
  synthetic DNA
caagcaatagttgtcggccacc

SEQ ID NO: 1371 - DNA, 22 bp, Artificial
  synthetic DNA
ttcagcaatccgtactgctaga

SEQ ID NO: 1372 - DNA, 22 bp, Artificial
  synthetic DNA
tgagacgttgctgacattctcc

SEQ ID NO: 1373 - DNA, 22 bp, Artificial
  synthetic DNA
gttccgatgagttagatgtata

SEQ ID NO: 1374 - DNA, 22 bp, Artificial
  synthetic DNA
ttgacgcttggaggagtacaag

SEQ ID NO: 1375 - DNA, 22 bp, Artificial
  synthetic DNA
ttcatgttacctccacattgtg

SEQ ID NO: 1376 - DNA, 22 bp, Artificial
  synthetic DNA
gagcacgtgccagattgcaacc

SEQ ID NO: 1377 - DNA, 22 bp, Artificial
  synthetic DNA
ggtcgacaagcacaagccttct

SEQ ID NO: 1378 - DNA, 22 bp, Artificial
  synthetic DNA
taggcaggtaagatgaccgact

SEQ ID NO: 1379 - DNA, 22 bp, Artificial
  synthetic DNA
cgaggcatgccaagtcgccaat

SEQ ID NO: 1380 - DNA, 22 bp, Artificial
  synthetic DNA
agtgttgataggcggatgagag

SEQ ID NO: 1381 - DNA, 22 bp, Artificial
  synthetic DNA
ttcggtctagacctctcacaat

SEQ ID NO: 1382 - DNA, 22 bp, Artificial
  synthetic DNA
gtgacgctcatatcttgccacc

SEQ ID NO: 1383 - DNA, 22 bp, Artificial
  synthetic DNA
gatgtaattctacgcgcggact

SEQ ID NO: 1384 - DNA, 22 bp, Artificial
  synthetic DNA
gatggcgatgttgcattacatg

SEQ ID NO: 1385 - DNA, 22 bp, Artificial
  synthetic DNA
tatgctctgaattaacgtagaa

SEQ ID NO: 1386 - DNA, 22 bp, Artificial
  synthetic DNA
aggcaatatggtgatccgtagc

SEQ ID NO: 1387 - DNA, 22 bp, Artificial
  synthetic DNA
tgacagcgatgcatacagtagt

SEQ ID NO: 1388 - DNA, 22 bp, Artificial
  synthetic DNA
ttctgctaacggtatccaatac

SEQ ID NO: 1389 - DNA, 22 bp, Artificial
  synthetic DNA
gagtcgtccatacgatctagga

SEQ ID NO: 1390 - DNA, 22 bp, Artificial
  synthetic DNA
agacggactcaacgccaattcc

SEQ ID NO: 1391 - DNA, 22 bp, Artificial
  synthetic DNA
gtagtgttgagcggaccgagct

SEQ ID NO: 1392 - DNA, 22 bp, Artificial
  synthetic DNA
aatataactagatcatagccag

SEQ ID NO: 1393 - DNA, 22 bp, Artificial
  synthetic DNA
tcaatcggagaatacagaacgt

SEQ ID NO: 1394 - DNA, 22 bp, Artificial
  synthetic DNA
atctccgtcgtccgaaccaaca

SEQ ID NO: 1395 - DNA, 22 bp, Artificial
  synthetic DNA
taggcgttcagcggtatgctta

SEQ ID NO: 1396 - DNA, 22 bp, Artificial
  synthetic DNA
tgcgtgctatacaacctatacg

SEQ ID NO: 1397 - DNA, 22 bp, Artificial
  synthetic DNA
atggccggcatacatctgtatg

SEQ ID NO: 1398 - DNA, 22 bp, Artificial
  synthetic DNA
tgatgctgacataacactgaat

SEQ ID NO: 1399 - DNA, 22 bp, Artificial
  synthetic DNA
atccaaggtacctgaacatcct

SEQ ID NO: 1400 - DNA, 22 bp, Artificial
  synthetic DNA
tagtgacgaccaggtgagcctc

SEQ ID NO: 1401 - DNA, 22 bp, Artificial
  synthetic DNA
aggaggatccgtcaagtcgacc

SEQ ID NO: 1402 - DNA, 22 bp, Artificial
  synthetic DNA
agagtatgccagatcgtgaggc

SEQ ID NO: 1403 - DNA, 22 bp, Artificial
  synthetic DNA
ccactcactaggatggctgcgt

SEQ ID NO: 1404 - DNA, 22 bp, Artificial
  synthetic DNA
tatccaacctgttatagcgatt

SEQ ID NO: 1405 - DNA, 22 bp, Artificial
  synthetic DNA
tcttgcagtgagttgagtctgc

SEQ ID NO: 1406 - DNA, 22 bp, Artificial
  synthetic DNA
ccactgttgtacatacacctgg

SEQ ID NO: 1407 - DNA, 22 bp, Artificial
  synthetic DNA
atgcgcgtaggccactaagtcc

SEQ ID NO: 1408 - DNA, 22 bp, Artificial
  synthetic DNA
acagcggtctacaaccgactgc

SEQ ID NO: 1409 - DNA, 22 bp, Artificial
  synthetic DNA
tcgcgctccagacaattgcagc

SEQ ID NO: 1410 - DNA, 22 bp, Artificial
  synthetic DNA
ccggtagaccaggagtggtcat

SEQ ID NO: 1411 - DNA, 22 bp, Artificial
  synthetic DNA
atctcctaacctagagccatct

SEQ ID NO: 1412 - DNA, 22 bp, Artificial
  synthetic DNA
ccacatcgaatctaacaactac

SEQ ID NO: 1413 - DNA, 22 bp, Artificial
  synthetic DNA
tagtcttattgaatacgtccta

SEQ ID NO: 1414 - DNA, 22 bp, Artificial
  synthetic DNA
tccttaagccttggaactggcg

SEQ ID NO: 1415 - DNA, 22 bp, Artificial
  synthetic DNA
ccgtgatggattgacgtagagg

SEQ ID NO: 1416 - DNA, 22 bp, Artificial
  synthetic DNA
gcctggataacagatgtcttag

SEQ ID NO: 1417 - DNA, 22 bp, Artificial
  synthetic DNA
ctcgacctataatcttctgcca

SEQ ID NO: 1418 - DNA, 22 bp, Artificial
  synthetic DNA
agctacttctccttcctaatca

SEQ ID NO: 1419 - DNA, 22 bp, Artificial
  synthetic DNA
acacgctattgccttccagtta

SEQ ID NO: 1420 - DNA, 22 bp, Artificial
  synthetic DNA
aagcctgtgcatgcaatgagaa

SEQ ID NO: 1421 - DNA, 22 bp, Artificial
  synthetic DNA
tcgttggttatagcacaacttc

SEQ ID NO: 1422 - DNA, 22 bp, Artificial
  synthetic DNA
gcgatgccttccaacataccaa

SEQ ID NO: 1423 - DNA, 22 bp, Artificial
  synthetic DNA
ccaccgttagcacgtgctacgt

SEQ ID NO: 1424 - DNA, 22 bp, Artificial
  synthetic DNA
gttaccacaatgccgccatcaa

SEQ ID NO: 1425 - DNA, 22 bp, Artificial
  synthetic DNA
ggtgcattaagaacgaactacc

SEQ ID NO: 1426 - DNA, 22 bp, Artificial
  synthetic DNA
tccttccggataatgccgattc

SEQ ID NO: 1427 - DNA, 22 bp, Artificial
  synthetic DNA
aaccgcaacttctagcggaaga

SEQ ID NO: 1428 - DNA, 22 bp, Artificial
  synthetic DNA
tccttaagcagttgaacctagg

SEQ ID NO: 1429 - DNA, 22 bp, Artificial
  synthetic DNA
tactaagtcagataagatcaga

SEQ ID NO: 1430 - DNA, 22 bp, Artificial
  synthetic DNA
ttcgccataactagatgaatgc

SEQ ID NO: 1431 - DNA, 22 bp, Artificial
  synthetic DNA
aagaagttagacgcggtggctg

SEQ ID NO: 1432 - DNA, 22 bp, Artificial
  synthetic DNA
gtatctgatcgaagagcggtgg

SEQ ID NO: 1433 - DNA, 22 bp, Artificial
  synthetic DNA
tcaagagctacgaagtaagtcc

SEQ ID NO: 1434 - DNA, 22 bp, Artificial
  synthetic DNA
cgagtacacagcagcataccta

SEQ ID NO: 1435 - DNA, 22 bp, Artificial
  synthetic DNA
ctcgataagttactctgctaga

SEQ ID NO: 1436 - DNA, 22 bp, Artificial
  synthetic DNA
atggtgctggttctccgtctgt

SEQ ID NO: 1437 - DNA, 22 bp, Artificial
  synthetic DNA
tcaagcggtccaaggctgagac

SEQ ID NO: 1438 - DNA, 22 bp, Artificial
  synthetic DNA
tgtcctgctctgttgctaccgt

SEQ ID NO: 1439 - DNA, 22 bp, Artificial
  synthetic DNA
agtcatatcgcgtcacacgttg

SEQ ID NO: 1440 - DNA, 22 bp, Artificial
  synthetic DNA
ggtgaataaggacatgagaagc

SEQ ID NO: 1441 - DNA, 24 bp, Artificial
  synthetic DNA
cctgatcttatctagtagagactc

SEQ ID NO: 1442 - DNA, 24 bp, Artificial
  synthetic DNA
ttctgtgtaggtgtgccaatcacc

SEQ ID NO: 1443 - DNA, 24 bp, Artificial
  synthetic DNA
gacttccagatgcttaagacgaca

SEQ ID NO: 1444 - DNA, 24 bp, Artificial
  synthetic DNA
gtccttcgacggagaacatccgag

SEQ ID NO: 1445 - DNA, 24 bp, Artificial
  synthetic DNA
cttggttagtgtaccgtcaacgtc

SEQ ID NO: 1446 - DNA, 24 bp, Artificial
  synthetic DNA
aagcggcatgtgcctaatcgacgt

SEQ ID NO: 1447 - DNA, 24 bp, Artificial
  synthetic DNA
cgaccgtcgttacacggaatccga

SEQ ID NO: 1448 - DNA, 24 bp, Artificial
  synthetic DNA
tcgcaagtgtgccgttctgttcat

SEQ ID NO: 1449 - DNA, 24 bp, Artificial
  synthetic DNA
cgtactgaagttcggagtcgccgt

SEQ ID NO: 1450 - DNA, 24 bp, Artificial
  synthetic DNA
ccactacagaatggtagcagatca

SEQ ID NO: 1451 - DNA, 24 bp, Artificial
  synthetic DNA
agtaggagagaggcctacacaaca

SEQ ID NO: 1452 - DNA, 24 bp, Artificial
  synthetic DNA
agccaagatactcgttcggtatgg

SEQ ID NO: 1453 - DNA, 24 bp, Artificial
  synthetic DNA
gttccgagtacattgaatcctggc

SEQ ID NO: 1454 - DNA, 24 bp, Artificial
  synthetic DNA
aggcgtacgagttattgccagagg

SEQ ID NO: 1455 - DNA, 24 bp, Artificial
  synthetic DNA
gtggcatcacacatatctcagcat

SEQ ID NO: 1456 - DNA, 24 bp, Artificial
  synthetic DNA
gagaccgatatgttgatgccagaa

SEQ ID NO: 1457 - DNA, 24 bp, Artificial
  synthetic DNA
caactgtagccagtcgattgctat

SEQ ID NO: 1458 - DNA, 24 bp, Artificial
  synthetic DNA
tatcaatgcaatgagaggatgcag

SEQ ID NO: 1459 - DNA, 24 bp, Artificial
  synthetic DNA
gtatgctcggctccaagtactgtt

SEQ ID NO: 1460 - DNA, 24 bp, Artificial
  synthetic DNA
agagactcttataggcttgacgga

SEQ ID NO: 1461 - DNA, 24 bp, Artificial
  synthetic DNA
acttaacagatatggatcatcgcc

SEQ ID NO: 1462 - DNA, 24 bp, Artificial
  synthetic DNA
aatcagagcgagtctcgcttcagg

SEQ ID NO: 1463 - DNA, 24 bp, Artificial
  synthetic DNA
accaccgaggaacaggtgcgacaa

SEQ ID NO: 1464 - DNA, 24 bp, Artificial
  synthetic DNA
tggtacatgtcaaccgtaagcctg

SEQ ID NO: 1465 - DNA, 24 bp, Artificial
  synthetic DNA
cgtgccgcggtgttcttgtatatg

SEQ ID NO: 1466 - DNA, 24 bp, Artificial
  synthetic DNA
gacaagcgcgcgtgagacatatca

SEQ ID NO: 1467 - DNA, 24 bp, Artificial
  synthetic DNA
agtgcactccgaacaagagttagt

SEQ ID NO: 1468 - DNA, 24 bp, Artificial
  synthetic DNA
cctcattaccgcgttaggagtccg

SEQ ID NO: 1469 - DNA, 24 bp, Artificial
  synthetic DNA
tgcttattgcttagttgctatctc

SEQ ID NO: 1470 - DNA, 24 bp, Artificial
  synthetic DNA
gcgtgatcctgttctattcgttag

SEQ ID NO: 1471 - DNA, 24 bp, Artificial
  synthetic DNA
ggccagaactatgacgagtataag

SEQ ID NO: 1472 - DNA, 24 bp, Artificial
  synthetic DNA
gatggcgactatctaattgcaatg

SEQ ID NO: 1473 - DNA, 24 bp, Artificial
  synthetic DNA
tagtaaccatagctctgtacaact

SEQ ID NO: 1474 - DNA, 24 bp, Artificial
  synthetic DNA
cgtgatcgccaatacacatgtcgc

SEQ ID NO: 1475 - DNA, 24 bp, Artificial
  synthetic DNA
taataacggatcgatatgcacgcg

SEQ ID NO: 1476 - DNA, 24 bp, Artificial
  synthetic DNA
atcatcgcgctaatactatctgaa

SEQ ID NO: 1477 - DNA, 24 bp, Artificial
  synthetic DNA
cacgtgcgtgcaggtcactagtat

SEQ ID NO: 1478 - DNA, 24 bp, Artificial
  synthetic DNA
aggtccaatgccgagcgatcagaa

SEQ ID NO: 1479 - DNA, 24 bp, Artificial
  synthetic DNA
cagcataacaacgagccaggtcag

SEQ ID NO: 1480 - DNA, 24 bp, Artificial
  synthetic DNA
atggcgtccaatactccgacctat

SEQ ID NO: 1481 - DNA, 24 bp, Artificial
  synthetic DNA
aggaacatcgtgaataatgaagac

SEQ ID NO: 1482 - DNA, 24 bp, Artificial
  synthetic DNA
tctcgacgttcatgtaattaagga

SEQ ID NO: 1483 - DNA, 24 bp, Artificial
  synthetic DNA
tcgcggttaaccttacttagacga

SEQ ID NO: 1484 - DNA, 24 bp, Artificial
  synthetic DNA
atcatatctacggctctggcgccg

SEQ ID NO: 1485 - DNA, 24 bp, Artificial
  synthetic DNA
gcagatggagaccagaggtacagg

SEQ ID NO: 1486 - DNA, 24 bp, Artificial
  synthetic DNA
agacagaagattaccacgtgctat

SEQ ID NO: 1487 - DNA, 24 bp, Artificial
  synthetic DNA
ccacggacaacatgccgcttaact

SEQ ID NO: 1488 - DNA, 24 bp, Artificial
  synthetic DNA
cttgaagtctcaagctatgagaga

SEQ ID NO: 1489 - DNA, 24 bp, Artificial
  synthetic DNA
acagcagtcgtgcttaggtcactg

SEQ ID NO: 1490 - DNA, 24 bp, Artificial
  synthetic DNA
aggtgttaatgaacgtaggtgaga

SEQ ID NO: 1491 - DNA, 24 bp, Artificial
  synthetic DNA
agccactatgttcaaggctgagcc

SEQ ID NO: 1492 - DNA, 24 bp, Artificial
  synthetic DNA
gcaggcggtgtcgtgtgacaatga

SEQ ID NO: 1493 - DNA, 24 bp, Artificial
  synthetic DNA
agccattgctacagaggttactta

SEQ ID NO: 1494 - DNA, 24 bp, Artificial
  synthetic DNA
acaatcgaacctacactgagtccg

SEQ ID NO: 1495 - DNA, 24 bp, Artificial
  synthetic DNA
ccgatctcaataggtaccacgaac

SEQ ID NO: 1496 - DNA, 24 bp, Artificial
  synthetic DNA
gatacgtggcgctatgctaattaa

SEQ ID NO: 1497 - DNA, 24 bp, Artificial
  synthetic DNA
agagagatggcacacattgacgtc

SEQ ID NO: 1498 - DNA, 24 bp, Artificial
  synthetic DNA
ctcaactcatccttgtagccgatg

SEQ ID NO: 1499 - DNA, 24 bp, Artificial
  synthetic DNA
gtggaataacgcgatacgactctt

SEQ ID NO: 1500 - DNA, 24 bp, Artificial
  synthetic DNA
atctaccatgcgaatgctctctag

SEQ ID NO: 1501 - DNA, 24 bp, Artificial
  synthetic DNA
atacgcacgcctgacacaaggacc

SEQ ID NO: 1502 - DNA, 24 bp, Artificial
  synthetic DNA
gtccactctcagtgtgtagagtcc

SEQ ID NO: 1503 - DNA, 24 bp, Artificial
  synthetic DNA
aatatatccagattctctgtgcag

SEQ ID NO: 1504 - DNA, 24 bp, Artificial
  synthetic DNA
ccttccgccacatgttcgacaagg

SEQ ID NO: 1505 - DNA, 24 bp, Artificial
  synthetic DNA
actgtgccatcatccgaggagcca

SEQ ID NO: 1506 - DNA, 24 bp, Artificial
  synthetic DNA
tctatgccgctatggcgtcgtgta

SEQ ID NO: 1507 - DNA, 24 bp, Artificial
  synthetic DNA
cgtaacctaaggtaatatgtctgc

SEQ ID NO: 1508 - DNA, 24 bp, Artificial
  synthetic DNA
tactgaccgtatcaagattactaa

SEQ ID NO: 1509 - DNA, 24 bp, Artificial
  synthetic DNA
tcatcggagcgccatacggtacgt

SEQ ID NO: 1510 - DNA, 24 bp, Artificial
  synthetic DNA
gcaagaggaatgaacgaagtgatt

SEQ ID NO: 1511 - DNA, 24 bp, Artificial
  synthetic DNA
ggctgattgacatcctgacttagt

SEQ ID NO: 1512 - DNA, 24 bp, Artificial
  synthetic DNA
aaggcgctagattggattaacgta

SEQ ID NO: 1513 - DNA, 24 bp, Artificial
  synthetic DNA
gctagctagaagaataggattcgt

SEQ ID NO: 1514 - DNA, 24 bp, Artificial
  synthetic DNA
caggtgacggcctctataactcat

SEQ ID NO: 1515 - DNA, 24 bp, Artificial
  synthetic DNA
caggttacacataccactatcttc

SEQ ID NO: 1516 - DNA, 24 bp, Artificial
  synthetic DNA
ttgctacgtaccgtcttaatccgt

SEQ ID NO: 1517 - DNA, 24 bp, Artificial
  synthetic DNA
ctcaacatgtcttgcaagcttcga

SEQ ID NO: 1518 - DNA, 24 bp, Artificial
  synthetic DNA
ggtgcggtacgtagaaccagatca

SEQ ID NO: 1519 - DNA, 24 bp, Artificial
  synthetic DNA
aatgctctccaagatcctgaccta

SEQ ID NO: 1520 - DNA, 24 bp, Artificial
  synthetic DNA
gcttcgcaggtctggatgatggag

SEQ ID NO: 1521 - DNA, 24 bp, Artificial
  synthetic DNA
acattgaccagacagcaccttgcg

SEQ ID NO: 1522 - DNA, 24 bp, Artificial
  synthetic DNA
aggtatcaatgtgcttaataggcg

SEQ ID NO: 1523 - DNA, 24 bp, Artificial
  synthetic DNA
tccggacacacgattagtaacgga

SEQ ID NO: 1524 - DNA, 24 bp, Artificial
  synthetic DNA
tacgaagtactacagatcggtcag

SEQ ID NO: 1525 - DNA, 24 bp, Artificial
  synthetic DNA
aattgtcagacgaatactgctgga

SEQ ID NO: 1526 - DNA, 24 bp, Artificial
  synthetic DNA
tgaatcatgagccagaggttatgc

SEQ ID NO: 1527 - DNA, 24 bp, Artificial
  synthetic DNA
cacaagacacgtcattaacatcaa

SEQ ID NO: 1528 - DNA, 24 bp, Artificial
  synthetic DNA
gaatgactacattactccgccagg

SEQ ID NO: 1529 - DNA, 24 bp, Artificial
  synthetic DNA
agccagagatactggaacttgact

SEQ ID NO: 1530 - DNA, 24 bp, Artificial
  synthetic DNA
tatcagacacatcacaatggatac

SEQ ID NO: 1531 - DNA, 24 bp, Artificial
  synthetic DNA
ctaggacaccgctagtcggttgaa

SEQ ID NO: 1532 - DNA, 24 bp, Artificial
  synthetic DNA
gtataactgcgtgtcctggtgtat

SEQ ID NO: 1533 - DNA, 24 bp, Artificial
  synthetic DNA
atgcaatactaaggtggacctccg

SEQ ID NO: 1534 - DNA, 24 bp, Artificial
  synthetic DNA
atgcagacgcttgcgataagtcat

SEQ ID NO: 1535 - DNA, 24 bp, Artificial
  synthetic DNA
ttgctcgatacacgtagaccagtg

SEQ ID NO: 1536 - DNA, 24 bp, Artificial
  synthetic DNA
tactggaggacgattgtctatcat

SEQ ID NO: 1537 - DNA, 26 bp, Artificial
  synthetic DNA
actaaggcacgctgattcgagcatta

SEQ ID NO: 1538 - DNA, 26 bp, Artificial
  synthetic DNA
cggattctggcacgtacaagtagcag

SEQ ID NO: 1539 - DNA, 26 bp, Artificial
  synthetic DNA
ttatggctccagatctagtcaccagc

SEQ ID NO: 1540 - DNA, 26 bp, Artificial
  synthetic DNA
catacactccaggcatgtatgatagg

SEQ ID NO: 1541 - DNA, 26 bp, Artificial
  synthetic DNA
agttgtaagccaacgagtgtagcgta

SEQ ID NO: 1542 - DNA, 26 bp, Artificial
  synthetic DNA
gtatcagctccttcctctgattccgg

SEQ ID NO: 1543 - DNA, 26 bp, Artificial
  synthetic DNA
aacatacagaatgtctatggtcagct

SEQ ID NO: 1544 - DNA, 26 bp, Artificial
  synthetic DNA
gactcatattcatgttcagtatagag

SEQ ID NO: 1545 - DNA, 26 bp, Artificial
  synthetic DNA
agagtgaacgaacgtgaccgacgctc

SEQ ID NO: 1546 - DNA, 26 bp, Artificial
  synthetic DNA
aattggcgtccttgccacaacatctt

SEQ ID NO: 1547 - DNA, 26 bp, Artificial
  synthetic DNA
tcgtagacgcctcgtacatccgagat

SEQ ID NO: 1548 - DNA, 26 bp, Artificial
  synthetic DNA
ccggctcgtgaggcgataatcatata

SEQ ID NO: 1549 - DNA, 26 bp, Artificial
  synthetic DNA
agtcctgatcacgaccacgactcacg

SEQ ID NO: 1550 - DNA, 26 bp, Artificial
  synthetic DNA
ggcactcaatcctccatggagaagct

SEQ ID NO: 1551 - DNA, 26 bp, Artificial
  synthetic DNA
tcatcattcctcacgttcaccggtga

SEQ ID NO: 1552 - DNA, 26 bp, Artificial
  synthetic DNA
tcaactctgtgctaaccggtcgtaca

SEQ ID NO: 1553 - DNA, 26 bp, Artificial
  synthetic DNA
tgttcttatgcattaatgccaggctt

SEQ ID NO: 1554 - DNA, 26 bp, Artificial
  synthetic DNA
gattcacgacctcaacagcatcactc

SEQ ID NO: 1555 - DNA, 26 bp, Artificial
  synthetic DNA
ggcgagttcgaccagaatgctggaca

SEQ ID NO: 1556 - DNA, 26 bp, Artificial
  synthetic DNA
ttccgtatacaatgcgattaagatct

SEQ ID NO: 1557 - DNA, 26 bp, Artificial
  synthetic DNA
gagtaatccgtaaccggccaacgttg

SEQ ID NO: 1558 - DNA, 26 bp, Artificial
  synthetic DNA
cgcttccatcatggtacggtacgtat

SEQ ID NO: 1559 - DNA, 26 bp, Artificial
  synthetic DNA
ccgtcgtggtgtgttgactggtcaac

SEQ ID NO: 1560 - DNA, 26 bp, Artificial
  synthetic DNA
tattcgcatctccgtattagttgtag

SEQ ID NO: 1561 - DNA, 26 bp, Artificial
  synthetic DNA
tattattgtattctaggcggtgcaac

SEQ ID NO: 1562 - DNA, 26 bp, Artificial
  synthetic DNA
aggctgcctacttcctcgtcatctcg

SEQ ID NO: 1563 - DNA, 26 bp, Artificial
  synthetic DNA
gtaacatacggctcatcgaatgcatc

SEQ ID NO: 1564 - DNA, 26 bp, Artificial
  synthetic DNA
ttatggcacggatattaccgtacgcc

SEQ ID NO: 1565 - DNA, 26 bp, Artificial
  synthetic DNA
atagcacttcctctaatgctctgctg

SEQ ID NO: 1566 - DNA, 26 bp, Artificial
  synthetic DNA
tcacaggcaatagcctaatattatat

SEQ ID NO: 1567 - DNA, 26 bp, Artificial
  synthetic DNA
ggcggatgttcgttaatattataagg

SEQ ID NO: 1568 - DNA, 26 bp, Artificial
  synthetic DNA
tgcaatagccgttgtctctgccagcg

SEQ ID NO: 1569 - DNA, 26 bp, Artificial
  synthetic DNA
tacagcgcgttggcgagtactgatag

SEQ ID NO: 1570 - DNA, 26 bp, Artificial
  synthetic DNA
tgcagttagtaccttctcacgccaac

SEQ ID NO: 1571 - DNA, 26 bp, Artificial
  synthetic DNA
ccattggctacctagcagactctacc

SEQ ID NO: 1572 - DNA, 26 bp, Artificial
  synthetic DNA
aacagtagctcgcgtcttgctctcgt

SEQ ID NO: 1573 - DNA, 26 bp, Artificial
  synthetic DNA
gcagtccatcagctctcgcttataga

SEQ ID NO: 1574 - DNA, 26 bp, Artificial
  synthetic DNA
tatctctctgtcgccagcttgaccaa

SEQ ID NO: 1575 - DNA, 26 bp, Artificial
  synthetic DNA
cagactgttcaagcttgctgtaggag

SEQ ID NO: 1576 - DNA, 26 bp, Artificial
  synthetic DNA
taaccggaactcgttcagcaacattc

SEQ ID NO: 1577 - DNA, 26 bp, Artificial
  synthetic DNA
tcaattatgcatgtcgtccgatctct

SEQ ID NO: 1578 - DNA, 26 bp, Artificial
  synthetic DNA
ttgtctaagtcaacctgtggataatc

SEQ ID NO: 1579 - DNA, 26 bp, Artificial
  synthetic DNA
tctaagagtggtatgaccaggagtcc

SEQ ID NO: 1580 - DNA, 26 bp, Artificial
  synthetic DNA
tcgtagtactactggaacaggtaatc

SEQ ID NO: 1581 - DNA, 26 bp, Artificial
  synthetic DNA
atgtcaacattctaatcatctctcgg

SEQ ID NO: 1582 - DNA, 26 bp, Artificial
  synthetic DNA
agcgcgcaactgttacggtgatccga

SEQ ID NO: 1583 - DNA, 26 bp, Artificial
  synthetic DNA
gcgatagaataatggtgtcacacacg

SEQ ID NO: 1584 - DNA, 26 bp, Artificial
  synthetic DNA
aaggctgcgatgagaggcgtacatcg

SEQ ID NO: 1585 - DNA, 26 bp, Artificial
  synthetic DNA
ggttcatggtctcagtcgtgatcgcg

SEQ ID NO: 1586 - DNA, 26 bp, Artificial
  synthetic DNA
tagtgactctatgtcacctcggagcc

SEQ ID NO: 1587 - DNA, 26 bp, Artificial
  synthetic DNA
atgtgatagcaatggcacctctagtc

SEQ ID NO: 1588 - DNA, 26 bp, Artificial
  synthetic DNA
tcgcgaagtgtaatgcatcatccgct

SEQ ID NO: 1589 - DNA, 26 bp, Artificial
  synthetic DNA
atgtggcgacgatccaagttcaacgc

SEQ ID NO: 1590 - DNA, 26 bp, Artificial
  synthetic DNA
accttgtatgagtcggagtgtccggc

SEQ ID NO: 1591 - DNA, 26 bp, Artificial
  synthetic DNA
acctcaagagagtagacagttgagtt

SEQ ID NO: 1592 - DNA, 26 bp, Artificial
  synthetic DNA
ggtgtaatcctgtgtgcgaagctggt

SEQ ID NO: 1593 - DNA, 26 bp, Artificial
  synthetic DNA
atagcggaactgtacgacgctccagt

SEQ ID NO: 1594 - DNA, 26 bp, Artificial
  synthetic DNA
aagcacgagtcgaccattagcctgga

SEQ ID NO: 1595 - DNA, 26 bp, Artificial
  synthetic DNA
attccggtaacatcagaaggtacaat

SEQ ID NO: 1596 - DNA, 26 bp, Artificial
  synthetic DNA
gtgcaacggcagtccagtatcctggt

SEQ ID NO: 1597 - DNA, 26 bp, Artificial
  synthetic DNA
ccatcttatacacggtgaccgaagat

SEQ ID NO: 1598 - DNA, 26 bp, Artificial
  synthetic DNA
gcacttaatcaagcttgagtgatgct

SEQ ID NO: 1599 - DNA, 26 bp, Artificial
  synthetic DNA
agtattacgtgagtacgaagatagca

SEQ ID NO: 1600 - DNA, 26 bp, Artificial
  synthetic DNA
ttcttaggttaagttccttctggacc

SEQ ID NO: 1601 - DNA, 26 bp, Artificial
  synthetic DNA
gtccttgctagacactgaccgttgct

SEQ ID NO: 1602 - DNA, 26 bp, Artificial
  synthetic DNA
gccgctatgtgtgctgcatcctaagc

SEQ ID NO: 1603 - DNA, 26 bp, Artificial
  synthetic DNA
ccatcaataacagacttatgttgtga

SEQ ID NO: 1604 - DNA, 26 bp, Artificial
  synthetic DNA
cgcgtgtgcttacaagtgctaacaag

SEQ ID NO: 1605 - DNA, 26 bp, Artificial
  synthetic DNA
cgatatgtgttcgcaataagagagcc

SEQ ID NO: 1606 - DNA, 26 bp, Artificial
  synthetic DNA
cgcggatgtgagcggctcaattagca

SEQ ID NO: 1607 - DNA, 26 bp, Artificial
  synthetic DNA
gctgcatgactatcggatggaggcat

SEQ ID NO: 1608 - DNA, 26 bp, Artificial
  synthetic DNA
ctatgccgtgtatggtacgagtggcg

SEQ ID NO: 1609 - DNA, 26 bp, Artificial
  synthetic DNA
ccggctggagttcattacgtaggctg

SEQ ID NO: 1610 - DNA, 26 bp, Artificial
  synthetic DNA
tgtaggcctactgagctagtattaga

SEQ ID NO: 1611 - DNA, 26 bp, Artificial
  synthetic DNA
ccgtcaagtgactattcttctaatct

SEQ ID NO: 1612 - DNA, 26 bp, Artificial
  synthetic DNA
ggtcttacgccagagactgcgcttct

SEQ ID NO: 1613 - DNA, 26 bp, Artificial
  synthetic DNA
cgaagtgtgattattaactgtaatct

SEQ ID NO: 1614 - DNA, 26 bp, Artificial
  synthetic DNA
gcacgcgtggccgtaagcatcgatta

SEQ ID NO: 1615 - DNA, 26 bp, Artificial
  synthetic DNA
atcctgcgtcggaacgtactatagct

SEQ ID NO: 1616 - DNA, 26 bp, Artificial
  synthetic DNA
agtatcatcatatccattcgcagtac

SEQ ID NO: 1617 - DNA, 26 bp, Artificial
  synthetic DNA
agtcctgacgttcatatatagactcc

SEQ ID NO: 1618 - DNA, 26 bp, Artificial
  synthetic DNA
cttgcagtaatctgaatctgaaggtt

SEQ ID NO: 1619 - DNA, 26 bp, Artificial
  synthetic DNA
ataacttggttccagtaacgcatagt

SEQ ID NO: 1620 - DNA, 26 bp, Artificial
  synthetic DNA
gataaggatatggctgtagcgaagtg

SEQ ID NO: 1621 - DNA, 26 bp, Artificial
  synthetic DNA
gtggagcgttacagacatgctgaaca

SEQ ID NO: 1622 - DNA, 26 bp, Artificial
  synthetic DNA
cgcttccggcaggcgtcatataagtc

SEQ ID NO: 1623 - DNA, 26 bp, Artificial
  synthetic DNA
ataacattctaacctctataagccga

SEQ ID NO: 1624 - DNA, 26 bp, Artificial
  synthetic DNA
acgatctatgatccatatggacttcc

SEQ ID NO: 1625 - DNA, 26 bp, Artificial
  synthetic DNA
tgaagctcagatatcatgcctcgagc

SEQ ID NO: 1626 - DNA, 26 bp, Artificial
  synthetic DNA
agacttcaccgcaataactcgtagat

SEQ ID NO: 1627 - DNA, 26 bp, Artificial
  synthetic DNA
agactaagacatacgccatcaccgct

SEQ ID NO: 1628 - DNA, 26 bp, Artificial
  synthetic DNA
tgtagcgtgatgtatcgtaattctgt

SEQ ID NO: 1629 - DNA, 26 bp, Artificial
  synthetic DNA
tgtgctattggcacctcacgctgacc

SEQ ID NO: 1630 - DNA, 26 bp, Artificial
  synthetic DNA
tgtagataagtatccagcgactctct

SEQ ID NO: 1631 - DNA, 26 bp, Artificial
  synthetic DNA
aattcgccaattgtgtgtaggcgcaa

SEQ ID NO: 1632 - DNA, 26 bp, Artificial
  synthetic DNA
cgattatgagtacttgtagaccagct

SEQ ID NO: 1633 - DNA, 28 bp, Artificial
  synthetic DNA
ttgcaagaacaacgtatctcatatgaac

SEQ ID NO: 1634 - DNA, 28 bp, Artificial
  synthetic DNA
caccgtgctgttattacttggtattcgg

SEQ ID NO: 1635 - DNA, 28 bp, Artificial
  synthetic DNA
cacgtgtattgttgcaccagaacgacaa

SEQ ID NO: 1636 - DNA, 28 bp, Artificial
  synthetic DNA
atgcacgtaattacttccggagaagacg

SEQ ID NO: 1637 - DNA, 28 bp, Artificial
  synthetic DNA
tatgttgtctgatatggttcatgtggca

SEQ ID NO: 1638 - DNA, 28 bp, Artificial
  synthetic DNA
agcgcgactagttgatgccaacattgta

SEQ ID NO: 1639 - DNA, 28 bp, Artificial
  synthetic DNA
ataggcaggtccaggctcggaacaagtc

SEQ ID NO: 1640 - DNA, 28 bp, Artificial
  synthetic DNA
gcggtagtcggtcaagaactagaaccgt

SEQ ID NO: 1641 - DNA, 28 bp, Artificial
  synthetic DNA
actatacactctagctattaggaagcat

SEQ ID NO: 1642 - DNA, 28 bp, Artificial
  synthetic DNA
gatcatcttgcttctcctgtggagataa

SEQ ID NO: 1643 - DNA, 28 bp, Artificial
  synthetic DNA
ctactacgagtccataactgatagcctc

SEQ ID NO: 1644 - DNA, 28 bp, Artificial
  synthetic DNA
gcacagacacctgtcctatctagcagga

SEQ ID NO: 1645 - DNA, 28 bp, Artificial
  synthetic DNA
aagcgaggcgcgaaggagatggaaggat

SEQ ID NO: 1646 - DNA, 28 bp, Artificial
  synthetic DNA
ctgaagacgccagtctggataggtgcct

SEQ ID NO: 1647 - DNA, 28 bp, Artificial
  synthetic DNA
gtaagctctgtccttcgagattgataag

SEQ ID NO: 1648 - DNA, 28 bp, Artificial
  synthetic DNA
ggttagagagattattgtgcgcatccat

SEQ ID NO: 1649 - DNA, 28 bp, Artificial
  synthetic DNA
ccaggaggacctatgatcttgccgccat

SEQ ID NO: 1650 - DNA, 28 bp, Artificial
  synthetic DNA
actattcgagctactgtatgtgtatccg

SEQ ID NO: 1651 - DNA, 28 bp, Artificial
  synthetic DNA
gacatcgcgatacgtaactccggagtgt

SEQ ID NO: 1652 - DNA, 28 bp, Artificial
  synthetic DNA
ccgcaattcgtctatatattctagcata

SEQ ID NO: 1653 - DNA, 28 bp, Artificial
  synthetic DNA
ctacacttgaggttgatgctcaagatca

SEQ ID NO: 1654 - DNA, 28 bp, Artificial
  synthetic DNA
cgatcagttctagttcaccgcggacaat

SEQ ID NO: 1655 - DNA, 28 bp, Artificial
  synthetic DNA
aagaatgatgattggccgcgaaccaagc

SEQ ID NO: 1656 - DNA, 28 bp, Artificial
  synthetic DNA
cacgaccggaactagactcctaccaatt

SEQ ID NO: 1657 - DNA, 28 bp, Artificial
  synthetic DNA
agttgcctgtgagtgaggctactatctc

SEQ ID NO: 1658 - DNA, 28 bp, Artificial
  synthetic DNA
gattcttccgatgatcatgccactacaa

SEQ ID NO: 1659 - DNA, 28 bp, Artificial
  synthetic DNA
cgctgaagtgaactatgcaagcaccgca

SEQ ID NO: 1660 - DNA, 28 bp, Artificial
  synthetic DNA
attatcgtgatggtgagactgagctcgt

SEQ ID NO: 1661 - DNA, 28 bp, Artificial
  synthetic DNA
cgaggccactctgagccaggtaagtatc

SEQ ID NO: 1662 - DNA, 28 bp, Artificial
  synthetic DNA
tgccgaggacagccgatcacatcttcgt

SEQ ID NO: 1663 - DNA, 28 bp, Artificial
  synthetic DNA
gttgacatgaaggttatcgtcgatattc

SEQ ID NO: 1664 - DNA, 28 bp, Artificial
  synthetic DNA
gtggtccaggtcaagctctgatcgaatg

SEQ ID NO: 1665 - DNA, 28 bp, Artificial
  synthetic DNA
ccagtccggtgtactcagacctaataac

SEQ ID NO: 1666 - DNA, 28 bp, Artificial
  synthetic DNA
cgagacactgcatgagcgtagtcttatt

SEQ ID NO: 1667 - DNA, 28 bp, Artificial
  synthetic DNA
gacggcttgtatacttctctacggtctg

SEQ ID NO: 1668 - DNA, 28 bp, Artificial
  synthetic DNA
ttagctggatggaagccatattccgtag

SEQ ID NO: 1669 - DNA, 28 bp, Artificial
  synthetic DNA
cagcctacacttgattactcaacaactc

SEQ ID NO: 1670 - DNA, 28 bp, Artificial
  synthetic DNA
gtacgtagtgtcacgcgcctacgttcgt

SEQ ID NO: 1671 - DNA, 28 bp, Artificial
  synthetic DNA
ctacaacttctcaatcatgcctctgttg

SEQ ID NO: 1672 - DNA, 28 bp, Artificial
  synthetic DNA
cgaggacagaattcgacataaggagaga

SEQ ID NO: 1673 - DNA, 28 bp, Artificial
  synthetic DNA
gccgaacgacacagtgagttgataggta

SEQ ID NO: 1674 - DNA, 28 bp, Artificial
  synthetic DNA
gaacactatatgctgtcgctgtctgagg

SEQ ID NO: 1675 - DNA, 28 bp, Artificial
  synthetic DNA
gttaagttcttcggcggtcatgctcatt

SEQ ID NO: 1676 - DNA, 28 bp, Artificial
  synthetic DNA
ttgcttacagatcgcgtatccatagtat

SEQ ID NO: 1677 - DNA, 28 bp, Artificial
  synthetic DNA
gaggaccacctctgcgaagttcactgtg

SEQ ID NO: 1678 - DNA, 28 bp, Artificial
  synthetic DNA
aatcctagcatatcgagaacgacactga

SEQ ID NO: 1679 - DNA, 28 bp, Artificial
  synthetic DNA
tgaatactatagccatagtcgacttccg

SEQ ID NO: 1680 - DNA, 28 bp, Artificial
  synthetic DNA
gacatccacgaagctggtaatcggaacc

SEQ ID NO: 1681 - DNA, 28 bp, Artificial
  synthetic DNA
ttagccgtcttagaagtgtctgaccggc

SEQ ID NO: 1682 - DNA, 28 bp, Artificial
  synthetic DNA
ctattctgccgtaattgattccttcgtt

SEQ ID NO: 1683 - DNA, 28 bp, Artificial
  synthetic DNA
acgcctctggtcgaaggtagattagctc

SEQ ID NO: 1684 - DNA, 28 bp, Artificial
  synthetic DNA
cagcctattgatcgtaagtagatggtcc

SEQ ID NO: 1685 - DNA, 28 bp, Artificial
  synthetic DNA
ttaagtgaggtggacaaccatcaacttc

SEQ ID NO: 1686 - DNA, 28 bp, Artificial
  synthetic DNA
aaggccttgcggctaagtagtattcatc

SEQ ID NO: 1687 - DNA, 28 bp, Artificial
  synthetic DNA
ttgtgatactaattcttctcaagagtca

SEQ ID NO: 1688 - DNA, 28 bp, Artificial
  synthetic DNA
gcattaggtgacgaccttagtccatcac

SEQ ID NO: 1689 - DNA, 28 bp, Artificial
  synthetic DNA
gcggatggacgtatacagtgagtcgtgc

SEQ ID NO: 1690 - DNA, 28 bp, Artificial
  synthetic DNA
gaacatgccagcctcaactaggctaaga

SEQ ID NO: 1691 - DNA, 28 bp, Artificial
  synthetic DNA
tccgtcattagagtatgagtgactacta

SEQ ID NO: 1692 - DNA, 28 bp, Artificial
  synthetic DNA
aacacttagtaaccagttcggactggac

SEQ ID NO: 1693 - DNA, 28 bp, Artificial
  synthetic DNA
cgctaactattgcgtatattcgcggctt

SEQ ID NO: 1694 - DNA, 28 bp, Artificial
  synthetic DNA
gccatctacgatcttcggcttatcctag

SEQ ID NO: 1695 - DNA, 28 bp, Artificial
  synthetic DNA
cctgagaatgttgactaagatcttgtga

SEQ ID NO: 1696 - DNA, 28 bp, Artificial
  synthetic DNA
tcggttagtctaatcatcacgcaacgga

SEQ ID NO: 1697 - DNA, 28 bp, Artificial
  synthetic DNA
attatctattgaagcagtgacagcgatc

SEQ ID NO: 1698 - DNA, 28 bp, Artificial
  synthetic DNA
gaggagaatcacggaacacggtcacatg

SEQ ID NO: 1699 - DNA, 28 bp, Artificial
  synthetic DNA
gctgcaagcattatgaccatggcatctg

SEQ ID NO: 1700 - DNA, 28 bp, Artificial
  synthetic DNA
gaacaacctataacgacgttgtggacaa

SEQ ID NO: 1701 - DNA, 28 bp, Artificial
  synthetic DNA
ttaatcatcgatagacgacatggaatca

SEQ ID NO: 1702 - DNA, 28 bp, Artificial
  synthetic DNA
tcgagtgtaagcacactacgatctggaa

SEQ ID NO: 1703 - DNA, 28 bp, Artificial
  synthetic DNA
gctacgcacagtctctgcacagctacac

SEQ ID NO: 1704 - DNA, 28 bp, Artificial
  synthetic DNA
cctgtatgtacgttctggctaatacctt

SEQ ID NO: 1705 - DNA, 28 bp, Artificial
  synthetic DNA
tgaagcaccggtacatggtgtatccgga

SEQ ID NO: 1706 - DNA, 28 bp, Artificial
  synthetic DNA
tgctggaacctaactcggtgatgacgat

SEQ ID NO: 1707 - DNA, 28 bp, Artificial
  synthetic DNA
cgctatcttactgccaagttctcatata

SEQ ID NO: 1708 - DNA, 28 bp, Artificial
  synthetic DNA
aacgcgcgcgtatcggcaataatctcaa

SEQ ID NO: 1709 - DNA, 28 bp, Artificial
  synthetic DNA
ccattaggatgaccatcgactattagag

SEQ ID NO: 1710 - DNA, 28 bp, Artificial
  synthetic DNA
tactgctagactgcgtgcattcatggcg

SEQ ID NO: 1711 - DNA, 28 bp, Artificial
  synthetic DNA
cattgcgcgctccacgaactctattgtc

SEQ ID NO: 1712 - DNA, 28 bp, Artificial
  synthetic DNA
gacgcgcctagaactgtatagctctacg

SEQ ID NO: 1713 - DNA, 28 bp, Artificial
  synthetic DNA
cattgcaacttgtcggtgatggcaatcc

SEQ ID NO: 1714 - DNA, 28 bp, Artificial
  synthetic DNA
ttaatgcacatgcagtacggcaccacag

SEQ ID NO: 1715 - DNA, 28 bp, Artificial
  synthetic DNA
agcggtacgtggacgagtggtaattaat

SEQ ID NO: 1716 - DNA, 28 bp, Artificial
  synthetic DNA
gacgtattgctatgcattggaagatgct

SEQ ID NO: 1717 - DNA, 28 bp, Artificial
  synthetic DNA
aacacttcgaccattgcgcctcaatggt

SEQ ID NO: 1718 - DNA, 28 bp, Artificial
  synthetic DNA
cggtacgctctagcggtcataagatgca

SEQ ID NO: 1719 - DNA, 28 bp, Artificial
  synthetic DNA
cctgaataacagccgcgcctaattagat

SEQ ID NO: 1720 - DNA, 28 bp, Artificial
  synthetic DNA
aagcgtctaatgtgccttaagtcacatg

SEQ ID NO: 1721 - DNA, 28 bp, Artificial
  synthetic DNA
gctctccaagaaccagaagtaagcatcg

SEQ ID NO: 1722 - DNA, 28 bp, Artificial
  synthetic DNA
gaggagagttgtccgagtggtgtgatgt

SEQ ID NO: 1723 - DNA, 28 bp, Artificial
  synthetic DNA
taacgagtggtgcgtctaagcaattgag

SEQ ID NO: 1724 - DNA, 28 bp, Artificial
  synthetic DNA
ccaacagtatgctgacataactatgata

SEQ ID NO: 1725 - DNA, 28 bp, Artificial
  synthetic DNA
gatccttgccacgcctatgagatatcgc

SEQ ID NO: 1726 - DNA, 28 bp, Artificial
  synthetic DNA
aacgcgctaccgtccttgtgcatagagg

SEQ ID NO: 1727 - DNA, 28 bp, Artificial
  synthetic DNA
ctacatgtgccttatagtacagaggaac

SEQ ID NO: 1728 - DNA, 28 bp, Artificial
  synthetic DNA
cagcctcgtagttagcgtgattcatgcg

SEQ ID NO: 1729 - DNA, 29 bp, Artificial
  synthetic DNA
ctcctcgccgattgaagtgcgtagaacta

SEQ ID NO: 1730 - DNA, 29 bp, Artificial
  synthetic DNA
cagcaggcctcaataggataagccaacta

SEQ ID NO: 1731 - DNA, 29 bp, Artificial
  synthetic DNA
gaccatcaatctcgaagactacgctctgt

SEQ ID NO: 1732 - DNA, 29 bp, Artificial
  synthetic DNA
ggttgctccgtctgttcagcacactgtta

SEQ ID NO: 1733 - DNA, 29 bp, Artificial
  synthetic DNA
aatgtcgactggccattatcgccaagtgt

SEQ ID NO: 1734 - DNA, 29 bp, Artificial
  synthetic DNA
gatagcttgccatgcgaatggatctccag

SEQ ID NO: 1735 - DNA, 29 bp, Artificial
  synthetic DNA
ccagaccggagccaattggctgccaatat

SEQ ID NO: 1736 - DNA, 29 bp, Artificial
  synthetic DNA
aacgtcgctccatacgttacctaatgcag

SEQ ID NO: 1737 - DNA, 29 bp, Artificial
  synthetic DNA
gaatatgacgcgaacagtctattcggatc

SEQ ID NO: 1738 - DNA, 29 bp, Artificial
  synthetic DNA
gacgagaatgtattaaggataagcaaggt

SEQ ID NO: 1739 - DNA, 29 bp, Artificial
  synthetic DNA
aagtcgtatgaatcgctatcacatgagtc

SEQ ID NO: 1740 - DNA, 29 bp, Artificial
  synthetic DNA
gtcgtggagactacaattctcctcacgtt

SEQ ID NO: 1741 - DNA, 29 bp, Artificial
  synthetic DNA
gttgccaccgttacacgactatcgacagt

SEQ ID NO: 1742 - DNA, 29 bp, Artificial
  synthetic DNA
aggataggctacgccttactctcctaagc

SEQ ID NO: 1743 - DNA, 29 bp, Artificial
  synthetic DNA
taatcatcctgttcgcctcgaggttgtta

SEQ ID NO: 1744 - DNA, 29 bp, Artificial
  synthetic DNA
gacaagcagtaataattactgagtggacg

SEQ ID NO: 1745 - DNA, 29 bp, Artificial
  synthetic DNA
tacagcgttacgcaggtatatcaaggtag

SEQ ID NO: 1746 - DNA, 29 bp, Artificial
  synthetic DNA
ctaacatcacttactattagcggtctcgt

SEQ ID NO: 1747 - DNA, 29 bp, Artificial
  synthetic DNA
ccgcgcttcttgacacgttctccactagg

SEQ ID NO: 1748 - DNA, 29 bp, Artificial
  synthetic DNA
caagtaacatgagatgctatcggtacatt

SEQ ID NO: 1749 - DNA, 29 bp, Artificial
  synthetic DNA
cgaccactaggctgtgaccacgatacgct

SEQ ID NO: 1750 - DNA, 29 bp, Artificial
  synthetic DNA
caggtcatgtgacgcagtcggcagtcaac

SEQ ID NO: 1751 - DNA, 29 bp, Artificial
  synthetic DNA
actccatcgttagttcttccgccgtgctg

SEQ ID NO: 1752 - DNA, 29 bp, Artificial
  synthetic DNA
ctcaccacgtatgcgtcactcggttacgt

SEQ ID NO: 1753 - DNA, 29 bp, Artificial
  synthetic DNA
tgcctatgctatggaccttgcgcgactct

SEQ ID NO: 1754 - DNA, 29 bp, Artificial
  synthetic DNA
aatgaaggtcaacgctctgtagttacgcg

SEQ ID NO: 1755 - DNA, 29 bp, Artificial
  synthetic DNA
caccattgattcatggcttccatcactgc

SEQ ID NO: 1756 - DNA, 29 bp, Artificial
  synthetic DNA
gacacgcaaggtaattcgagattgcagca

SEQ ID NO: 1757 - DNA, 29 bp, Artificial
  synthetic DNA
caccgagaggaaggttcgatcgcttctcg

SEQ ID NO: 1758 - DNA, 29 bp, Artificial
  synthetic DNA
cagttatcggattgtgatattcactcctg

SEQ ID NO: 1759 - DNA, 29 bp, Artificial
  synthetic DNA
atactgtaacgcctcaacctatgctgact

SEQ ID NO: 1760 - DNA, 29 bp, Artificial
  synthetic DNA
atctgtcttattctggcacactcagactt

SEQ ID NO: 1761 - DNA, 29 bp, Artificial
  synthetic DNA
tccaaccggtgacgtgctcttgatccaac

SEQ ID NO: 1762 - DNA, 29 bp, Artificial
  synthetic DNA
cacactcagttcggctatctctgcgatag

SEQ ID NO: 1763 - DNA, 29 bp, Artificial
  synthetic DNA
agctgtaagtcaggtctacgactcgtact

SEQ ID NO: 1764 - DNA, 29 bp, Artificial
  synthetic DNA
gtcggcggcacgcacagctaacattcgta

SEQ ID NO: 1765 - DNA, 29 bp, Artificial
  synthetic DNA
atatggtagccagccacgtatactgaaca

SEQ ID NO: 1766 - DNA, 29 bp, Artificial
  synthetic DNA
tggacaatccgactctaacacagaggtag

SEQ ID NO: 1767 - DNA, 29 bp, Artificial
  synthetic DNA
tccgccgctgacagttcaatctatcaatt

SEQ ID NO: 1768 - DNA, 29 bp, Artificial
  synthetic DNA
ggttccttagaatatgcacctatcagcga

SEQ ID NO: 1769 - DNA, 29 bp, Artificial
  synthetic DNA
cggctgtacgacatggatcataagagtgt

SEQ ID NO: 1770 - DNA, 29 bp, Artificial
  synthetic DNA
tgcagatgtacgctgtggccagtggagag

SEQ ID NO: 1771 - DNA, 29 bp, Artificial
  synthetic DNA
cctactcacttaacaataatcggttcggt

SEQ ID NO: 1772 - DNA, 29 bp, Artificial
  synthetic DNA
cgcttcctactgcctgtgccgcgacataa

SEQ ID NO: 1773 - DNA, 29 bp, Artificial
  synthetic DNA
ctagaccgaccggttatgcgctattgttc

SEQ ID NO: 1774 - DNA, 29 bp, Artificial
  synthetic DNA
ttgtgagcacgtctgcggcaagcctatgg

SEQ ID NO: 1775 - DNA, 29 bp, Artificial
  synthetic DNA
tcatcggccggcgctgttgttgttaccat

SEQ ID NO: 1776 - DNA, 29 bp, Artificial
  synthetic DNA
gcggttaggtgcagttaggaagactatca

SEQ ID NO: 1777 - DNA, 29 bp, Artificial
  synthetic DNA
tatgcggtcgtgaggcgtagcattctaga

SEQ ID NO: 1778 - DNA, 29 bp, Artificial
  synthetic DNA
ccatctattcgtcgaactctcagctcgta

SEQ ID NO: 1779 - DNA, 29 bp, Artificial
  synthetic DNA
atcagatctactgatcgcggtagagtatc

SEQ ID NO: 1780 - DNA, 29 bp, Artificial
  synthetic DNA
tacacataggcggcgcagccttctaatta

SEQ ID NO: 1781 - DNA, 29 bp, Artificial
  synthetic DNA
ttaaccgtagttcttagcttacgccgctc

SEQ ID NO: 1782 - DNA, 29 bp, Artificial
  synthetic DNA
actatagaggacatggcactcctcttcta

SEQ ID NO: 1783 - DNA, 29 bp, Artificial
  synthetic DNA
cagttcgtattaagattgaatgtagcggt

SEQ ID NO: 1784 - DNA, 29 bp, Artificial
  synthetic DNA
agttatcggtatccgcttatccgtacgta

SEQ ID NO: 1785 - DNA, 29 bp, Artificial
  synthetic DNA
agcttattcatacactgcaccacagcaag

SEQ ID NO: 1786 - DNA, 29 bp, Artificial
  synthetic DNA
ccgtcggctagtctatcctctaattagaa

SEQ ID NO: 1787 - DNA, 29 bp, Artificial
  synthetic DNA
gtccgcttccatgcctgctgtacgaacac

SEQ ID NO: 1788 - DNA, 29 bp, Artificial
  synthetic DNA
tctcttcctccttcattgttcgctagctc

SEQ ID NO: 1789 - DNA, 29 bp, Artificial
  synthetic DNA
tctcttgagcggtcctcatacaggtctgc

SEQ ID NO: 1790 - DNA, 29 bp, Artificial
  synthetic DNA
gaccaagtgtaggtgatatcaccggtact

SEQ ID NO: 1791 - DNA, 29 bp, Artificial
  synthetic DNA
aagattgtgataggttggtagttaccaca

SEQ ID NO: 1792 - DNA, 29 bp, Artificial
  synthetic DNA
tcgcctccgaagagtatagcatcggcaga

SEQ ID NO: 1793 - DNA, 29 bp, Artificial
  synthetic DNA
gaggtagttatgagcatcgaggtcctgtt

SEQ ID NO: 1794 - DNA, 29 bp, Artificial
  synthetic DNA
ggacgcaagatcgcaggtacttgtaagct

SEQ ID NO: 1795 - DNA, 29 bp, Artificial
  synthetic DNA
actcgtacacgtcatcgtgcaggtctcag

SEQ ID NO: 1796 - DNA, 29 bp, Artificial
  synthetic DNA
taatccgtcaggagtgagatggctcgaca

SEQ ID NO: 1797 - DNA, 29 bp, Artificial
  synthetic DNA
aagatggttccgcgcattgactagcaagt

SEQ ID NO: 1798 - DNA, 29 bp, Artificial
  synthetic DNA
tccgcgatctgcggatcttgaatgctcac

SEQ ID NO: 1799 - DNA, 29 bp, Artificial
  synthetic DNA
ttcacgagagtcaactgctagtatcctag

SEQ ID NO: 1800 - DNA, 29 bp, Artificial
  synthetic DNA
ttccaactggattcttccaactcctcgaa

SEQ ID NO: 1801 - DNA, 29 bp, Artificial
  synthetic DNA
cactactactcaagttatacggtgttgac

SEQ ID NO: 1802 - DNA, 29 bp, Artificial
  synthetic DNA
caactggattctcaggatgcgtctctagc

SEQ ID NO: 1803 - DNA, 29 bp, Artificial
  synthetic DNA
tggactagagtggagcgattacgtaatat

SEQ ID NO: 1804 - DNA, 29 bp, Artificial
  synthetic DNA
gaggtcattcaactggactcgccacggac

SEQ ID NO: 1805 - DNA, 29 bp, Artificial
  synthetic DNA
caggtgtgtaacgctgcaatcacatgaat

SEQ ID NO: 1806 - DNA, 29 bp, Artificial
  synthetic DNA
tatgctgaggtattagttctaactatgcg

SEQ ID NO: 1807 - DNA, 29 bp, Artificial
  synthetic DNA
cgtctgagtcggataaggaaggttaccgc

SEQ ID NO: 1808 - DNA, 29 bp, Artificial
  synthetic DNA
gtactatcgtcgcaggcactatctctgcc

SEQ ID NO: 1809 - DNA, 29 bp, Artificial
  synthetic DNA
gcttcctccttgcaacttcattgcttcga

SEQ ID NO: 1810 - DNA, 29 bp, Artificial
  synthetic DNA
tgtctacgaagtagaagacacgaataatg

SEQ ID NO: 1811 - DNA, 29 bp, Artificial
  synthetic DNA
ccgtcatctaaggcagagtacatccgcga

SEQ ID NO: 1812 - DNA, 29 bp, Artificial
  synthetic DNA
ccggaggcgtactaactgaccacaacacc

SEQ ID NO: 1813 - DNA, 29 bp, Artificial
  synthetic DNA
aactcgtcgctgcctgaataggtcagagt

SEQ ID NO: 1814 - DNA, 29 bp, Artificial
  synthetic DNA
ttataagattaatgtcggtcagtgtcgga

SEQ ID NO: 1815 - DNA, 29 bp, Artificial
  synthetic DNA
cgtctcgatggatccacacgaacctgttg

SEQ ID NO: 1816 - DNA, 29 bp, Artificial
  synthetic DNA
atgccatcatggtcgtcctatcttaaggc

SEQ ID NO: 1817 - DNA, 29 bp, Artificial
  synthetic DNA
gcgcttcagcgattcgtcatgcaaggcac

SEQ ID NO: 1818 - DNA, 29 bp, Artificial
  synthetic DNA
ccaagcgataccgaggtacggttaacgag

SEQ ID NO: 1819 - DNA, 29 bp, Artificial
  synthetic DNA
atatgacagacaggtggacctaagcaagc

SEQ ID NO: 1820 - DNA, 29 bp, Artificial
  synthetic DNA
cactacatcgtcaggcctggaagcctcag

SEQ ID NO: 1821 - DNA, 29 bp, Artificial
  synthetic DNA
gccgtgtagacgaggacattatgtcgtat

SEQ ID NO: 1822 - DNA, 29 bp, Artificial
  synthetic DNA
caacgtatatacacaccttgtgaagagaa

SEQ ID NO: 1823 - DNA, 29 bp, Artificial
  synthetic DNA
tccaacgtaattccgccgtctgtcgagac

SEQ ID NO: 1824 - DNA, 29 bp, Artificial
  synthetic DNA
aattcgtgcttcgatcaccgtagactcag

SEQ ID NO: 1825 - DNA, 30 bp, Artificial
  synthetic DNA
actatattgtattcacgtccgacgactcgc

SEQ ID NO: 1826 - DNA, 30 bp, Artificial
  synthetic DNA
gacgagcttgtggtacactatacctatgag

SEQ ID NO: 1827 - DNA, 30 bp, Artificial
  synthetic DNA
tgattcaagcaccaggcatgcttaagctag

SEQ ID NO: 1828 - DNA, 30 bp, Artificial
  synthetic DNA
cggtctcctataggaaggctcattctgacg

SEQ ID NO: 1829 - DNA, 30 bp, Artificial
  synthetic DNA
agtcagtgtcgaatcaatcaaggcgtcctt

SEQ ID NO: 1830 - DNA, 30 bp, Artificial
  synthetic DNA
cgaacgtaatggccatcacgcgctggccta

SEQ ID NO: 1831 - DNA, 30 bp, Artificial
  synthetic DNA
cgaacctggaccacctggcattaccattac

SEQ ID NO: 1832 - DNA, 30 bp, Artificial
  synthetic DNA
acattaggttcctgtaatgtcttatcaacg

SEQ ID NO: 1833 - DNA, 30 bp, Artificial
  synthetic DNA
cgtctaatgcaccgtatcgtcttcgcgcat

SEQ ID NO: 1834 - DNA, 30 bp, Artificial
  synthetic DNA
tctatgacttacaacggaatcttacttcgt

SEQ ID NO: 1835 - DNA, 30 bp, Artificial
  synthetic DNA
gtaaccgatcggtaccgtctgctattgttc

SEQ ID NO: 1836 - DNA, 30 bp, Artificial
  synthetic DNA
ggtgattgataagcaacacatattaggagg

SEQ ID NO: 1837 - DNA, 30 bp, Artificial
  synthetic DNA
aattatcgacgctaataggcgagctgttca

SEQ ID NO: 1838 - DNA, 30 bp, Artificial
  synthetic DNA
ggaggtacatgacgagtggacagacagacc

SEQ ID NO: 1839 - DNA, 30 bp, Artificial
  synthetic DNA
ctctaatccgttatgcggtgatgtaatccg

SEQ ID NO: 1840 - DNA, 30 bp, Artificial
  synthetic DNA
gcaagcacgcggcttggcgaacttctatgc

SEQ ID NO: 1841 - DNA, 30 bp, Artificial
  synthetic DNA
tagatgtaggcctggtaggcagaggagtaa

SEQ ID NO: 1842 - DNA, 30 bp, Artificial
  synthetic DNA
ccgagtggcgaccacacaggtacgcattaa

SEQ ID NO: 1843 - DNA, 30 bp, Artificial
  synthetic DNA
gtcctggctcagattagtgcacttagttat

SEQ ID NO: 1844 - DNA, 30 bp, Artificial
  synthetic DNA
gcggtacctacatgttatgactcagacgac

SEQ ID NO: 1845 - DNA, 30 bp, Artificial
  synthetic DNA
tctctgccaatgctggtctcatcgaatcca

SEQ ID NO: 1846 - DNA, 30 bp, Artificial
  synthetic DNA
tctctacacagctacatactatactgtaac

SEQ ID NO: 1847 - DNA, 30 bp, Artificial
  synthetic DNA
tacgacggacgctggtggtgtaagagaagg

SEQ ID NO: 1848 - DNA, 30 bp, Artificial
  synthetic DNA
gcctcgatatatctacgtatagttcaagtt

SEQ ID NO: 1849 - DNA, 30 bp, Artificial
  synthetic DNA
ggctcctgcattcattgaaggtcggccttg

SEQ ID NO: 1850 - DNA, 30 bp, Artificial
  synthetic DNA
cagttcggtgattcaagagaacaatggtgg

SEQ ID NO: 1851 - DNA, 30 bp, Artificial
  synthetic DNA
tataacgaagccggctggaacggtaactca

SEQ ID NO: 1852 - DNA, 30 bp, Artificial
  synthetic DNA
ctgtatcaattcaagtgacagtggcacgtc

SEQ ID NO: 1853 - DNA, 30 bp, Artificial
  synthetic DNA
agcaattgcggttcataggcgtaattatat

SEQ ID NO: 1854 - DNA, 30 bp, Artificial
  synthetic DNA
catatggacctggagatcaccgttcagtcc

SEQ ID NO: 1855 - DNA, 30 bp, Artificial
  synthetic DNA
gaaggccgttggtctatctcttactggagc

SEQ ID NO: 1856 - DNA, 30 bp, Artificial
  synthetic DNA
gtgcgttcatctagcctaagacgctgacct

SEQ ID NO: 1857 - DNA, 30 bp, Artificial
  synthetic DNA
gagtaacttatatcctctctacgacatcga

SEQ ID NO: 1858 - DNA, 30 bp, Artificial
  synthetic DNA
attctacgctgatgtctccgctgaacagga

SEQ ID NO: 1859 - DNA, 30 bp, Artificial
  synthetic DNA
tcatcaacgttactcactagtaccacggct

SEQ ID NO: 1860 - DNA, 30 bp, Artificial
  synthetic DNA
aaccattcttgaacgttgagaacctggtgg

SEQ ID NO: 1861 - DNA, 30 bp, Artificial
  synthetic DNA
acgacacctccgcggaacatacctgattag

SEQ ID NO: 1862 - DNA, 30 bp, Artificial
  synthetic DNA
gcgcacttattgaagtaatctcatggccaa

SEQ ID NO: 1863 - DNA, 30 bp, Artificial
  synthetic DNA
gcgccaattcagccagttagcgtctccgtg

SEQ ID NO: 1864 - DNA, 30 bp, Artificial
  synthetic DNA
agcaacaagtcgctgtatatcgactggccg

SEQ ID NO: 1865 - DNA, 30 bp, Artificial
  synthetic DNA
ccttacaatagacctcgcggcgttcatgcc

SEQ ID NO: 1866 - DNA, 30 bp, Artificial
  synthetic DNA
ggatccaacttcagcgaagcaccaacgtcg

SEQ ID NO: 1867 - DNA, 30 bp, Artificial
  synthetic DNA
gcgccagttctcgtactctcgagaagcgac

SEQ ID NO: 1868 - DNA, 30 bp, Artificial
  synthetic DNA
gagtgcggccaatctggaactcatgacgtt

SEQ ID NO: 1869 - DNA, 30 bp, Artificial
  synthetic DNA
cctgagagtgattcgtgtctgcgaagatgc

SEQ ID NO: 1870 - DNA, 30 bp, Artificial
  synthetic DNA
gtgactggttaaggcaatattggtcgaccg

SEQ ID NO: 1871 - DNA, 30 bp, Artificial
  synthetic DNA
ctatcaagccttacaaggtcacgtccacta

SEQ ID NO: 1872 - DNA, 30 bp, Artificial
  synthetic DNA
actgcgtccttgcgtcggaactccttgtgt

SEQ ID NO: 1873 - DNA, 30 bp, Artificial
  synthetic DNA
tgcaactcagtggcggcgacaccaagagct

SEQ ID NO: 1874 - DNA, 30 bp, Artificial
  synthetic DNA
ttcggttctactaggatctctatctgagct

SEQ ID NO: 1875 - DNA, 30 bp, Artificial
  synthetic DNA
agctaatctattaagacagattagacagga

SEQ ID NO: 1876 - DNA, 30 bp, Artificial
  synthetic DNA
ggaccgctcttaggttatgcacctgcgtat

SEQ ID NO: 1877 - DNA, 30 bp, Artificial
  synthetic DNA
ctctaatactagtccacaggttagtacgaa

SEQ ID NO: 1878 - DNA, 30 bp, Artificial
  synthetic DNA
atccatatatgctcgtcgtcagccagtgtt

SEQ ID NO: 1879 - DNA, 30 bp, Artificial
  synthetic DNA
gctattactgtgttgatgtccacaggagaa

SEQ ID NO: 1880 - DNA, 30 bp, Artificial
  synthetic DNA
gctacggcgcagatctagacaactggaagt

SEQ ID NO: 1881 - DNA, 30 bp, Artificial
  synthetic DNA
gcctcttgtgttagccgaataccaatgacc

SEQ ID NO: 1882 - DNA, 30 bp, Artificial
  synthetic DNA
tgaggacgataacattacctctcgagtcgc

SEQ ID NO: 1883 - DNA, 30 bp, Artificial
  synthetic DNA
cgattaccaatccgacgacttcgcagcagc

SEQ ID NO: 1884 - DNA, 30 bp, Artificial
  synthetic DNA
atgacacgagtccagtacatatgcgaagac

SEQ ID NO: 1885 - DNA, 30 bp, Artificial
  synthetic DNA
gcgctcgcatgcactagtgtagactgacga

SEQ ID NO: 1886 - DNA, 30 bp, Artificial
  synthetic DNA
gcacatctcagaattgatggtctatgtcgc

SEQ ID NO: 1887 - DNA, 30 bp, Artificial
  synthetic DNA
ttcttcgacgccgcgtactaataggtcaat

SEQ ID NO: 1888 - DNA, 30 bp, Artificial
  synthetic DNA
ggaagcgcctctaacaaccgatgcttgtgg

SEQ ID NO: 1889 - DNA, 30 bp, Artificial
  synthetic DNA
ctctagacgcgtcgtgactccaatctgttg

SEQ ID NO: 1890 - DNA, 30 bp, Artificial
  synthetic DNA
gtagttcgtcggagtgacctcgtactcact

SEQ ID NO: 1891 - DNA, 30 bp, Artificial
  synthetic DNA
atgctgtcgagtgtccggcatagagcacac

SEQ ID NO: 1892 - DNA, 30 bp, Artificial
  synthetic DNA
gcgcatcttgcagcgtcctgtagttctgaa

SEQ ID NO: 1893 - DNA, 30 bp, Artificial
  synthetic DNA
gcgattgttgaggaaccacagcggcaccta

SEQ ID NO: 1894 - DNA, 30 bp, Artificial
  synthetic DNA
cacgcgtactctgcttgctgtgtggtcggt

SEQ ID NO: 1895 - DNA, 30 bp, Artificial
  synthetic DNA
catccaacgcaggacctagtagtcatgctt

SEQ ID NO: 1896 - DNA, 30 bp, Artificial
  synthetic DNA
ttctagttgtgatgagaatcgctagcgtgc

SEQ ID NO: 1897 - DNA, 30 bp, Artificial
  synthetic DNA
cattctgaatctggtctctctcgatcatcc

SEQ ID NO: 1898 - DNA, 30 bp, Artificial
  synthetic DNA
attaatgtagaggatagttccgttctctcc

SEQ ID NO: 1899 - DNA, 30 bp, Artificial
  synthetic DNA
gtatcgcgcttacgaatgaggtgtggcttc

SEQ ID NO: 1900 - DNA, 30 bp, Artificial
  synthetic DNA
gctggtgagagagccagattatcggtggag

SEQ ID NO: 1901 - DNA, 30 bp, Artificial
  synthetic DNA
ggcacgagcaggtagaactagaacctagat

SEQ ID NO: 1902 - DNA, 30 bp, Artificial
  synthetic DNA
tgtattatctcgaagcggtgcgttagagtc

SEQ ID NO: 1903 - DNA, 30 bp, Artificial
  synthetic DNA
cacgtgttctagctactaatggcgtcaatt

SEQ ID NO: 1904 - DNA, 30 bp, Artificial
  synthetic DNA
cgcgctacattacttcctacaccatgcgta

SEQ ID NO: 1905 - DNA, 30 bp, Artificial
  synthetic DNA
tgaggcaactagtgttcgcaagatgacgga

SEQ ID NO: 1906 - DNA, 30 bp, Artificial
  synthetic DNA
ttattattgtctgtggaacgcacgccagtc

SEQ ID NO: 1907 - DNA, 30 bp, Artificial
  synthetic DNA
gctatagtattatccatgaattccgtcggc

SEQ ID NO: 1908 - DNA, 30 bp, Artificial
  synthetic DNA
gtatcaatagctcaattcgtcagagttgtg

SEQ ID NO: 1909 - DNA, 30 bp, Artificial
  synthetic DNA
tagtccatgcgtggatatattgagagctga

SEQ ID NO: 1910 - DNA, 30 bp, Artificial
  synthetic DNA
gcacagtacgacttataacaggtctagatc

SEQ ID NO: 1911 - DNA, 30 bp, Artificial
  synthetic DNA
actcaatggtggcacgctcggcgcagcata

SEQ ID NO: 1912 - DNA, 30 bp, Artificial
  synthetic DNA
gtagtaccactccgccttaggcagcttaag

SEQ ID NO: 1913 - DNA, 30 bp, Artificial
  synthetic DNA
cgctcaactgatgcgtgcaaccaatgttat

SEQ ID NO: 1914 - DNA, 30 bp, Artificial
  synthetic DNA
gcagcttgactgcctagacagcagttacag

SEQ ID NO: 1915 - DNA, 30 bp, Artificial
  synthetic DNA
gcaacttcttagtacgaattcatcgtccaa

SEQ ID NO: 1916 - DNA, 30 bp, Artificial
  synthetic DNA
atccgtatgctgcggcagtggaggtggctt

SEQ ID NO: 1917 - DNA, 30 bp, Artificial
  synthetic DNA
tgcggatcaatccagttctgtgtactgtga

SEQ ID NO: 1918 - DNA, 30 bp, Artificial
  synthetic DNA
ttatgattatcaccggcgtaacattccgaa

SEQ ID NO: 1919 - DNA, 30 bp, Artificial
  synthetic DNA
gctacctagattcttcaactcatcgctacc

SEQ ID NO: 1920 - DNA, 30 bp, Artificial
  synthetic DNA
cagtgttagaatggcggtgtgtagccgcta

SEQ ID NO: 1921 - DNA, 35 bp, Artificial
  synthetic DNA
gcttatagactacagctgcgaggtataaggtcact

SEQ ID NO: 1922 - DNA, 35 bp, Artificial
  synthetic DNA
cgctcagcaggatgctatcctaagttaatgtggtg

SEQ ID NO: 1923 - DNA, 35 bp, Artificial
  synthetic DNA
gaactgagcggacatcagctaggcctacaatacat

SEQ ID NO: 1924 - DNA, 35 bp, Artificial
  synthetic DNA
tcgtgaacttctgcgttggtctctaccaaggcggt

SEQ ID NO: 1925 - DNA, 35 bp, Artificial
  synthetic DNA
taagtcaggtatcttatcagtggtacacggtacga

SEQ ID NO: 1926 - DNA, 35 bp, Artificial
  synthetic DNA
taataatgttgcgcgtgaccgaggaggaatccact

SEQ ID NO: 1927 - DNA, 35 bp, Artificial
  synthetic DNA
ctaggagttctcgtaagctggagtaccgtaacgtg

SEQ ID NO: 1928 - DNA, 35 bp, Artificial
  synthetic DNA
ggactctcctcagaggatccttcttgcgcaggcat

SEQ ID NO: 1929 - DNA, 35 bp, Artificial
  synthetic DNA
gctagaggcctgagtacaccttctcgcatcaggat

SEQ ID NO: 1930 - DNA, 35 bp, Artificial
  synthetic DNA
atatcgcgagcactaacgtcgttgtcgttctagga

SEQ ID NO: 1931 - DNA, 35 bp, Artificial
  synthetic DNA
agcggttactatacctggcggctgacgttgttagt

SEQ ID NO: 1932 - DNA, 35 bp, Artificial
  synthetic DNA
gagctaggtagatctccaagtgtagctaagaagag

SEQ ID NO: 1933 - DNA, 35 bp, Artificial
  synthetic DNA
ggagtcgctggtgacgtatgccgaggatgagcttc

SEQ ID NO: 1934 - DNA, 35 bp, Artificial
  synthetic DNA
cgccgacctcctgttcacgaagccgcctgatgtaa

SEQ ID NO: 1935 - DNA, 35 bp, Artificial
  synthetic DNA
agtaggcacttagttatcgattacgttagttagtc

SEQ ID NO: 1936 - DNA, 35 bp, Artificial
  synthetic DNA
ggatgacgtctcagtctacctcgcagtgtcgtcta

SEQ ID NO: 1937 - DNA, 35 bp, Artificial
  synthetic DNA
ctggttcgcgttagcaatactaaggcagtcaggag

SEQ ID NO: 1938 - DNA, 35 bp, Artificial
  synthetic DNA
atatggtcatattggcctcttcgaacacagactgt

SEQ ID NO: 1939 - DNA, 35 bp, Artificial
  synthetic DNA
tatcagaggatagcaggtctgagttgcaaggctaa

SEQ ID NO: 1940 - DNA, 35 bp, Artificial
  synthetic DNA
ggtggtctgaccatagctgttcttctcacagagac

SEQ ID NO: 1941 - DNA, 35 bp, Artificial
  synthetic DNA
gcaataccaacgagatgagtattcgttgaagctct

SEQ ID NO: 1942 - DNA, 35 bp, Artificial
  synthetic DNA
ccaagtcgacgctgcatgaatgagcgctattcact

SEQ ID NO: 1943 - DNA, 35 bp, Artificial
  synthetic DNA
ccattagatcgcttcgagacaattaggagacatga

SEQ ID NO: 1944 - DNA, 35 bp, Artificial
  synthetic DNA
gatgactgtacctcctatcattgagtgtggaccaa

SEQ ID NO: 1945 - DNA, 35 bp, Artificial
  synthetic DNA
atatctggatgaatagtggttaggtaagcaagtaa

SEQ ID NO: 1946 - DNA, 35 bp, Artificial
  synthetic DNA
accgactatgttaattcgtgtctggatggcagaat

SEQ ID NO: 1947 - DNA, 35 bp, Artificial
  synthetic DNA
gtggcagtcttgctagtatcttagaccatcaccaa

SEQ ID NO: 1948 - DNA, 35 bp, Artificial
  synthetic DNA
cgctatcttagtcgagcacaatgtcttcgtatagg

SEQ ID NO: 1949 - DNA, 35 bp, Artificial
  synthetic DNA
attagtacggcacgaaccggccattcatggcagct

SEQ ID NO: 1950 - DNA, 35 bp, Artificial
  synthetic DNA
agtacgactatcaagactccagcgctctccttgga

SEQ ID NO: 1951 - DNA, 35 bp, Artificial
  synthetic DNA
atgagcctcggagcgaacgttatcgatcaggctgt

SEQ ID NO: 1952 - DNA, 35 bp, Artificial
  synthetic DNA
ttgcgtgcagtagcaccgatacacagcgcttgtat

SEQ ID NO: 1953 - DNA, 35 bp, Artificial
  synthetic DNA
aacggctgcatcacctacactatactcaacatcta

SEQ ID NO: 1954 - DNA, 35 bp, Artificial
  synthetic DNA
gtcgctatgcgagaagtggcgtggaatgctatggt

SEQ ID NO: 1955 - DNA, 35 bp, Artificial
  synthetic DNA
catggatacctactgacttgacttctagaggaccg

SEQ ID NO: 1956 - DNA, 35 bp, Artificial
  synthetic DNA
gagtgacgcagacaccgtaacgtcgaatcttctag

SEQ ID NO: 1957 - DNA, 35 bp, Artificial
  synthetic DNA
agtaccgtctgtgtgaatattgttcctacgttaca

SEQ ID NO: 1958 - DNA, 35 bp, Artificial
  synthetic DNA
ggctaatcgatagtgacgagttctgcacgcctgaa

SEQ ID NO: 1959 - DNA, 35 bp, Artificial
  synthetic DNA
ggcgagcgctcgtggttctgagtcgctgttagatg

SEQ ID NO: 1960 - DNA, 35 bp, Artificial
  synthetic DNA
tatctccagcgttataagctactggagccgctcgg

SEQ ID NO: 1961 - DNA, 35 bp, Artificial
  synthetic DNA
ccttctgcgcaagtcaaggattcgcttagatggac

SEQ ID NO: 1962 - DNA, 35 bp, Artificial
  synthetic DNA
gttgctgacagccgttgcgtacttgccttaagaac

SEQ ID NO: 1963 - DNA, 35 bp, Artificial
  synthetic DNA
gtggcctaatcactcgcgcttcataggccgatagg

SEQ ID NO: 1964 - DNA, 35 bp, Artificial
  synthetic DNA
tgcatctagcctacatcggaccttgttatggtaat

SEQ ID NO: 1965 - DNA, 35 bp, Artificial
  synthetic DNA
ggacagctactggacaccaccgaactggtagtgtc

SEQ ID NO: 1966 - DNA, 35 bp, Artificial
  synthetic DNA
aactggcgatggacggccgctcttccgctacatag

SEQ ID NO: 1967 - DNA, 35 bp, Artificial
  synthetic DNA
ggagcagttagctatggagcaggccgataacctga

SEQ ID NO: 1968 - DNA, 35 bp, Artificial
  synthetic DNA
actctacggtgcacctcagccttcatgcaataggc

SEQ ID NO: 1969 - DNA, 35 bp, Artificial
  synthetic DNA
cttgtagcacaatacattactctccacgtgatagc

SEQ ID NO: 1970 - DNA, 35 bp, Artificial
  synthetic DNA
ggacgctatcgataccgttattcctactctgtcgg

SEQ ID NO: 1971 - DNA, 35 bp, Artificial
  synthetic DNA
ggatgatcgtcaacgatcaactgacagttagtcga

SEQ ID NO: 1972 - DNA, 35 bp, Artificial
  synthetic DNA
tgacagtagcaatgtctcacgtctgcacaacggaa

SEQ ID NO: 1973 - DNA, 35 bp, Artificial
  synthetic DNA
gtcgcaggacctcacggatagtagtgcgaggtcta

SEQ ID NO: 1974 - DNA, 35 bp, Artificial
  synthetic DNA
atatcggcggacgcaatgacagttgttggctgatg

SEQ ID NO: 1975 - DNA, 35 bp, Artificial
  synthetic DNA
aagcaccaaggaggtatgttccatcgaggcgctcg

SEQ ID NO: 1976 - DNA, 35 bp, Artificial
  synthetic DNA
gaccgcaccttatagctatatcctggtctagtact

SEQ ID NO: 1977 - DNA, 35 bp, Artificial
  synthetic DNA
tctcagaggaaggttgagcgtctgaccaggttggc

SEQ ID NO: 1978 - DNA, 35 bp, Artificial
  synthetic DNA
tggacctagagacctagctcgtctcttcgcgatcg

SEQ ID NO: 1979 - DNA, 35 bp, Artificial
  synthetic DNA
cggagtggttccacgcgacctcgcaactaatcctt

SEQ ID NO: 1980 - DNA, 35 bp, Artificial
  synthetic DNA
ggagccgcgcgcagactgaccttgcttgatctact

SEQ ID NO: 1981 - DNA, 35 bp, Artificial
  synthetic DNA
actctaagtatatgcgcagttagtatactgaacca

SEQ ID NO: 1982 - DNA, 35 bp, Artificial
  synthetic DNA
gagcattgcttcgcttcgatgtctattctgatcag

SEQ ID NO: 1983 - DNA, 35 bp, Artificial
  synthetic DNA
gcttgtattgccactcgagtaggtcgtggcagtag

SEQ ID NO: 1984 - DNA, 35 bp, Artificial
  synthetic DNA
atctggacattgcattcggtgtgtatacagaaggc

SEQ ID NO: 1985 - DNA, 35 bp, Artificial
  synthetic DNA
ggttgcgatcagcttgatagcaggtcatatcctca

SEQ ID NO: 1986 - DNA, 35 bp, Artificial
  synthetic DNA
gcaggtactaacctgagatgcgtagctaacacagg

SEQ ID NO: 1987 - DNA, 35 bp, Artificial
  synthetic DNA
atctgcaaggacgtaacgtcctcggaaggtgaggt

SEQ ID NO: 1988 - DNA, 35 bp, Artificial
  synthetic DNA
ataatcttacgagcctccagtgaataatgcaagca

SEQ ID NO: 1989 - DNA, 35 bp, Artificial
  synthetic DNA
caatctccgcacagtcttgttcaggtacagactta

SEQ ID NO: 1990 - DNA, 35 bp, Artificial
  synthetic DNA
atgtgcgcaattcagcgtaagtgcctattcataat

SEQ ID NO: 1991 - DNA, 35 bp, Artificial
  synthetic DNA
tcggacgcacacatcctgttgtcgagaagaggaag

SEQ ID NO: 1992 - DNA, 35 bp, Artificial
  synthetic DNA
tcggaagcatcacatgagcatcaggagttcattgc

SEQ ID NO: 1993 - DNA, 35 bp, Artificial
  synthetic DNA
atctggttgtggacttctatacagtaccagagtgg

SEQ ID NO: 1994 - DNA, 35 bp, Artificial
  synthetic DNA
cgtctgaatatagttagctagtagtgtaatccagg

SEQ ID NO: 1995 - DNA, 35 bp, Artificial
  synthetic DNA
taatatctgatccgacctattatctaggactactc

SEQ ID NO: 1996 - DNA, 35 bp, Artificial
  synthetic DNA
tatgcggccgtccgtacctcgtctgcttcagttgg

SEQ ID NO: 1997 - DNA, 35 bp, Artificial
  synthetic DNA
tggctcaagttccatattgccaagacgacctggag

SEQ ID NO: 1998 - DNA, 35 bp, Artificial
  synthetic DNA
gcagttctgctaggcggtccgaggcaattgaagag

SEQ ID NO: 1999 - DNA, 35 bp, Artificial
  synthetic DNA
catggcacagacgaagtatgcaccacgctcattaa

SEQ ID NO: 2000 - DNA, 35 bp, Artificial
  synthetic DNA
ggagcgtactacgaccattcaaccgaatatgttac

SEQ ID NO: 2001 - DNA, 35 bp, Artificial
  synthetic DNA
gcgtagatctcgcgacagagacaaggtgcgaatgg

SEQ ID NO: 2002 - DNA, 35 bp, Artificial
  synthetic DNA
tggactgaggttctccggtctatactcctgtagga

SEQ ID NO: 2003 - DNA, 35 bp, Artificial
  synthetic DNA
tggctatagcaacggcttcttgtgatcgcattgca

SEQ ID NO: 2004 - DNA, 35 bp, Artificial
  synthetic DNA
ggcgaagaatcatgcgagacggagtagacggacgt

SEQ ID NO: 2005 - DNA, 35 bp, Artificial
  synthetic DNA
gagcattgcgagttgcacacgtgatatcagactgt

SEQ ID NO: 2006 - DNA, 35 bp, Artificial
  synthetic DNA
ctgttgacctatgccagaatcaatacctcagatta

SEQ ID NO: 2007 - DNA, 35 bp, Artificial
  synthetic DNA
gttaacaagtagatgccaagatacaacgagagacc

SEQ ID NO: 2008 - DNA, 35 bp, Artificial
  synthetic DNA
gagcaagattatagttaggaagatagttaactcgc

SEQ ID NO: 2009 - DNA, 35 bp, Artificial
  synthetic DNA
tccggagtcgagcatatgtgaccaactctcaacgc

SEQ ID NO: 2010 - DNA, 35 bp, Artificial
  synthetic DNA
ggagctgcgatgccgttaccgacgtcatcttcaag

SEQ ID NO: 2011 - DNA, 35 bp, Artificial
  synthetic DNA
gctctatcttacacattggcgtactggactcgcga

SEQ ID NO: 2012 - DNA, 35 bp, Artificial
  synthetic DNA
ttctacatattcatcgcctaccgagttgcgcgaag

SEQ ID NO: 2013 - DNA, 35 bp, Artificial
  synthetic DNA
tggacgtctgacctgtgtctacatcggtggtgcta

SEQ ID NO: 2014 - DNA, 35 bp, Artificial
  synthetic DNA
ggcaggacagctccgtgttctactcgaaccgcact

SEQ ID NO: 2015 - DNA, 35 bp, Artificial
  synthetic DNA
tgacaacctcatgtctccgaccgcaggcatacaat

SEQ ID NO: 2016 - DNA, 35 bp, Artificial
  synthetic DNA
gcaggcctaacaagtggtcacgaggagtccttatt

SEQ ID NO: 2017 - DNA, 90 bp, Artificial
  synthetic DNA
cccatacacacaccatgaagcttgaactaattaacattctcaaactaattaacaagcatgcaagcatgtttttacacaatgacaatatat

SEQ ID NO: 2018 - DNA, 90 bp, Artificial
  synthetic DNA
atgggtgagggcgcagaggcaaagacatggaggtccggaagggtagaagctcacatcaagtcgagtatgttgaatgcaatcccatatata

SEQ ID NO: 2019 - DNA, 24 bp, Artificial
  synthetic DNA
cccatacacacaccatgaagcttg

SEQ ID NO: 2020 - DNA, 24 bp, Artificial
  synthetic DNA
ggtagaagctcacatcaagtcgag

SEQ ID NO: 2021 - DNA, 90 bp, Artificial
  synthetic DNA
aatcacagaacgaggtctggacgagaacagagctggacatctacacgcaccgcatggtagtagagcatgtactgcaaaagcttgaagcgc

SEQ ID NO: 2022 - DNA, 90 bp, Artificial
  synthetic DNA
gatgctgagggcgaagttgtcagccaagtcctcaatgtcataggcgagatcgcagtagttctgtaaccattccctgctaaactggtccat

SEQ ID NO: 2023 - DNA, 24 bp, Artificial
  synthetic DNA
acgagaacagagctggacatctac

SEQ ID NO: 2024 - DNA, 24 bp, Artificial
  synthetic DNA
tcaatgtcataggcgagatcgcag

SEQ ID NO: 2025 - DNA, 90 bp, Artificial
  synthetic DNA
agaccaacaagcagcaagtagtcagagaagtacaagagaaggagagcaagaaggatagtaagttgcaagcttaccgttacaaagatgata

SEQ ID NO: 2026 - DNA, 90 bp, Artificial
  synthetic DNA
ggaggagcacaactaggcgtttatcaagatgggtcatcgagctcttggtgtcttcaaccttcttgacatcaacttctccaatcttcgtct

SEQ ID NO: 2027 - DNA, 26 bp, Artificial
  synthetic DNA
ggagagcaagaaggatagtaagttgc

SEQ ID NO: 2028 - DNA, 25 bp, Artificial
  synthetic DNA
cgagctcttggtgtcttcaaccttc

SEQ ID NO: 2029 - DNA, 90 bp, Artificial
  synthetic DNA
tggggtagtcctgaagctctaggtatgcctcttcatctccctgcacctctggtgctagcacctcctgctcttcgggcacctctaccgggg

SEQ ID NO: 2030 - DNA, 90 bp, Artificial
  synthetic DNA
ggatactgatgtagctttcacccgggagtattccaaggtatcgattttccacggggaacgcgaagtgcactagttgaggtttagattgcc

SEQ ID NO: 2031 - DNA, 25 bp, Artificial
  synthetic DNA
gaagctctaggtatgcctcttcatc

SEQ ID NO: 2032 - DNA, 25 bp, Artificial
  synthetic DNA
gtgcactagttgaggtttagattgc

SEQ ID NO: 2033 - DNA, 90 bp, Artificial
  synthetic DNA
tcgggaaaacgaacgggcgaactacagatgtcagtacgaagtagtctatggcaggaaatacgtagtccatacgtggtgccagcccaagcc

SEQ ID NO: 2034 - DNA, 90 bp, Artificial
  synthetic DNA
agcaggagggagaaaggaaacgtggcattcatcggctgtctgccattgccatgtgagacaaggaaatctacttcacccccatctatcgag

SEQ ID NO: 2035 - DNA, 24 bp, Artificial
  synthetic DNA
gggcgaactacagatgtcagtacg

SEQ ID NO: 2036 - DNA, 24 bp, Artificial
  synthetic DNA
ctgtctgccattgccatgtgagac

SEQ ID NO: 2037 - DNA, 90 bp, Artificial
  synthetic DNA
agacataagattaactatgaacaaattcacgggtccgattcctttgggatttgcagcttgcaagaaccttcaaatactcattatatcttc

SEQ ID NO: 2038 - DNA, 90 bp, Artificial
  synthetic DNA
ttaagttgcagaatttgatacgaagaacttgaagcatggtgaggttgccgagctcattggggatggttccagaaaggctattgtagctta

SEQ ID NO: 2039 - DNA, 24 bp, Artificial
  synthetic DNA
gaacaaattcacgggtccgattcc

SEQ ID NO: 2040 - DNA, 24 bp, Artificial
  synthetic DNA
cgaagaacttgaagcatggtgagg

SEQ ID NO: 2041 - DNA, 10 bp, Artificial
  synthetic DNA
gttacacacg

SEQ ID NO: 2042 - DNA, 70 bp, Artificial
  synthetic DNA
aatgatacggcgaccaccgagatctacacctctctattcgtcggcagcgtcagatgtgtataagagacag

SEQ ID NO: 2043 - DNA, 66 bp, Artificial
  synthetic DNA
caagcagaagacggcatacgagattaaggcgagtctcgtgggctcggagatgtgtataagagacag

SEQ ID NO: 2044 - DNA, 12 bp, Artificial
  synthetic DNA
taagagacagaa

SEQ ID NO: 2045 - DNA, 12 bp, Artificial
  synthetic DNA
taagagacagat

SEQ ID NO: 2046 - DNA, 12 bp, Artificial
  synthetic DNA
taagagacagac

SEQ ID NO: 2047 - DNA, 12 bp, Artificial
  synthetic DNA
taagagacagag

SEQ ID NO: 2048 - DNA, 12 bp, Artificial
  synthetic DNA
taagagacagta

SEQ ID NO: 2049 - DNA, 12 bp, Artificial
  synthetic DNA
taagagacagtt

SEQ ID NO: 2050 - DNA, 12 bp, Artificial
  synthetic DNA
taagagacagtc

SEQ ID NO: 2051 - DNA, 12 bp, Artificial
  synthetic DNA
taagagacagtg

SEQ ID NO: 2052 - DNA, 12 bp, Artificial
  synthetic DNA
taagagacagca

SEQ ID NO: 2053 - DNA, 12 bp, Artificial
  synthetic DNA
taagagacagct

SEQ ID NO: 2054 - DNA, 12 bp, Artificial
  synthetic DNA
taagagacagcc

SEQ ID NO: 2055 - DNA, 12 bp, Artificial
  synthetic DNA
taagagacagcg

SEQ ID NO: 2056 - DNA, 12 bp, Artificial
  synthetic DNA
taagagacagga

SEQ ID NO: 2057 - DNA, 12 bp, Artificial
  synthetic DNA
taagagacaggt

SEQ ID NO: 2058 - DNA, 12 bp, Artificial
  synthetic DNA
taagagacaggc

SEQ ID NO: 2059 - DNA, 12 bp, Artificial
  synthetic DNA
taagagacaggg

SEQ ID NO: 2060 - DNA, 12 bp, Artificial
  synthetic DNA
  misc_feature (11)..(12): n is a, c, g, or t
taagagacagnn

SEQ ID NO: 2061 - DNA, 13 bp, Artificial
  synthetic DNA
  misc_feature (11)..(13): n is a, c, g, or t
taagagacagnnn

SEQ ID NO: 2062 - DNA, 10 bp, Artificial
  synthetic DNA
taagagacag

SEQ ID NO: 2063 - DNA, 12 bp, Artificial
  synthetic DNA
taagagacagtg

SEQ ID NO: 2064 - DNA, 13 bp, Artificial
  synthetic DNA
taagagacagtgc

SEQ ID NO: 2065 - DNA, 12 bp, Artificial
  synthetic DNA
taagagacagaa

SEQ ID NO: 2066 - DNA, 12 bp, Artificial
  synthetic DNA
taagagacagat

SEQ ID NO: 2067 - DNA, 12 bp, Artificial
  synthetic DNA
taagagacagac

SEQ ID NO: 2068 - DNA, 12 bp, Artificial
  synthetic DNA
taagagacagag

SEQ ID NO: 2069 - DNA, 12 bp, Artificial
  synthetic DNA
taagagacagta

SEQ ID NO: 2070 - DNA, 12 bp, Artificial
  synthetic DNA
taagagacagtt

SEQ ID NO: 2071 - DNA, 12 bp, Artificial
  synthetic DNA
taagagacagtc

SEQ ID NO: 2072 - DNA, 12 bp, Artificial
  synthetic DNA
taagagacagca

SEQ ID NO: 2073 - DNA, 12 bp, Artificial
  synthetic DNA
taagagacagct

SEQ ID NO: 2074 - DNA, 12 bp, Artificial
  synthetic DNA
taagagacagcc

SEQ ID NO: 2075 - DNA, 12 bp, Artificial
  synthetic DNA
taagagacagcg

SEQ ID NO: 2076 - DNA, 12 bp, Artificial
  synthetic DNA
taagagacagga

SEQ ID NO: 2077 - DNA, 12 bp, Artificial
  synthetic DNA
taagagacaggt

SEQ ID NO: 2078 - DNA, 12 bp, Artificial
  synthetic DNA
taagagacaggc

SEQ ID NO: 2079 - DNA, 12 bp, Artificial
  synthetic DNA
taagagacaggg

SEQ ID NO: 2080 - DNA, 13 bp, Artificial
  synthetic DNA
taagagacagaaa

SEQ ID NO: 2081 - DNA, 13 bp, Artificial
  synthetic DNA
taagagacagaac

SEQ ID NO: 2082 - DNA, 13 bp, Artificial
  synthetic DNA
taagagacagaag

SEQ ID NO: 2083 - DNA, 13 bp, Artificial
  synthetic DNA
taagagacagaat

SEQ ID NO: 2084 - DNA, 13 bp, Artificial
  synthetic DNA
taagagacagaca

SEQ ID NO: 2085 - DNA, 13 bp, Artificial
  synthetic DNA
taagagacagacc

SEQ ID NO: 2086 - DNA, 13 bp, Artificial
  synthetic DNA
taagagacagacg

SEQ ID NO: 2087 - DNA, 13 bp, Artificial
  synthetic DNA
taagagacagact

SEQ ID NO: 2088 - DNA, 13 bp, Artificial
  synthetic DNA
taagagacagaga

SEQ ID NO: 2089 - DNA, 13 bp, Artificial
  synthetic DNA
taagagacagagc

SEQ ID NO: 2090 - DNA, 13 bp, Artificial
  synthetic DNA
taagagacagagg

SEQ ID NO: 2091 - DNA, 13 bp, Artificial
  synthetic DNA
taagagacagagt

SEQ ID NO: 2092 - DNA, 13 bp, Artificial
  synthetic DNA
taagagacagata

SEQ ID NO: 2093 - DNA, 13 bp, Artificial
  synthetic DNA
taagagacagatc

SEQ ID NO: 2094 - DNA, 13 bp, Artificial
  synthetic DNA
taagagacagatg

SEQ ID NO: 2095 - DNA, 13 bp, Artificial
  synthetic DNA
taagagacagatt

SEQ ID NO: 2096 - DNA, 13 bp, Artificial
  synthetic DNA
taagagacagcaa

SEQ ID NO: 2097 - DNA, 13 bp, Artificial
  synthetic DNA
taagagacagcac

SEQ ID NO: 2098 - DNA, 13 bp, Artificial
  synthetic DNA
taagagacagcag

SEQ ID NO: 2099 - DNA, 13 bp, Artificial
  synthetic DNA
taagagacagcat

SEQ ID NO: 2100 - DNA, 13 bp, Artificial
  synthetic DNA
taagagacagcca

SEQ ID NO: 2101 - DNA, 13 bp, Artificial
  synthetic DNA
taagagacagccc

SEQ ID NO: 2102 - DNA, 13 bp, Artificial
  synthetic DNA
taagagacagccg

SEQ ID NO: 2103 - DNA, 13 bp, Artificial
  synthetic DNA
taagagacagcct

SEQ ID NO: 2104 - DNA, 13 bp, Artificial
  synthetic DNA
taagagacagcga

SEQ ID NO: 2105 - DNA, 13 bp, Artificial
  synthetic DNA
taagagacagcgc

SEQ ID NO: 2106 - DNA, 13 bp, Artificial
  synthetic DNA
taagagacagcgg

SEQ ID NO: 2107 - DNA, 13 bp, Artificial
  synthetic DNA
taagagacagcgt

SEQ ID NO: 2108 - DNA, 13 bp, Artificial
  synthetic DNA
taagagacagcta

SEQ ID NO: 2109 - DNA, 13 bp, Artificial
  synthetic DNA
taagagacagctc

SEQ ID NO: 2110 - DNA, 13 bp, Artificial
  synthetic DNA
taagagacagctg

SEQ ID NO: 2111 - DNA, 13 bp, Artificial
  synthetic DNA
taagagacagctt

SEQ ID NO: 2112 - DNA, 13 bp, Artificial
  synthetic DNA
taagagacaggaa

SEQ ID NO: 2113 - DNA, 13 bp, Artificial
  synthetic DNA
taagagacaggac

SEQ ID NO: 2114 - DNA, 13 bp, Artificial
  synthetic DNA
taagagacaggag

SEQ ID NO: 2115 - DNA, 13 bp, Artificial
  synthetic DNA
taagagacaggat

SEQ ID NO: 2116 - DNA, 13 bp, Artificial
  synthetic DNA
taagagacaggca

SEQ ID NO: 2117 - DNA, 13 bp, Artificial
  synthetic DNA
taagagacaggcc

SEQ ID NO: 2118 - DNA, 13 bp, Artificial
  synthetic DNA
taagagacaggcg

SEQ ID NO: 2119 - DNA, 13 bp, Artificial
  synthetic DNA
taagagacaggct

SEQ ID NO: 2120 - DNA, 13 bp, Artificial
  synthetic DNA
taagagacaggga

SEQ ID NO: 2121 - DNA, 13 bp, Artificial
  synthetic DNA
taagagacagggc

SEQ ID NO: 2122 - DNA, 13 bp, Artificial
  synthetic DNA
taagagacagggg

SEQ ID NO: 2123 - DNA, 13 bp, Artificial
  synthetic DNA
taagagacagggt

SEQ ID NO: 2124 - DNA, 13 bp, Artificial
  synthetic DNA
taagagacaggta

SEQ ID NO: 2125 - DNA, 13 bp, Artificial
  synthetic DNA
taagagacaggtc

SEQ ID NO: 2126 - DNA, 13 bp, Artificial
  synthetic DNA
taagagacaggtg

SEQ ID NO: 2127 - DNA, 13 bp, Artificial
  synthetic DNA
taagagacaggtt

SEQ ID NO: 2128 - DNA, 13 bp, Artificial
  synthetic DNA
taagagacagtaa

SEQ ID NO: 2129 - DNA, 13 bp, Artificial
  synthetic DNA
taagagacagtac

SEQ ID NO: 2130 - DNA, 13 bp, Artificial
  synthetic DNA
taagagacagtag

SEQ ID NO: 2131 - DNA, 13 bp, Artificial
  synthetic DNA
taagagacagtat

SEQ ID NO: 2132 - DNA, 13 bp, Artificial
  synthetic DNA
taagagacagtca

SEQ ID NO: 2133 - DNA, 13 bp, Artificial
  synthetic DNA
taagagacagtcc

SEQ ID NO: 2134 - DNA, 13 bp, Artificial
  synthetic DNA
taagagacagtcg

SEQ ID NO: 2135 - DNA, 13 bp, Artificial
  synthetic DNA
taagagacagtct

SEQ ID NO: 2136 - DNA, 13 bp, Artificial
  synthetic DNA
taagagacagtga

SEQ ID NO: 2137 - DNA, 13 bp, Artificial
  synthetic DNA
taagagacagtgg

SEQ ID NO: 2138 - DNA, 13 bp, Artificial
  synthetic DNA
taagagacagtgt

SEQ ID NO: 2139 - DNA, 13 bp, Artificial
  synthetic DNA
taagagacagtta

SEQ ID NO: 2140 - DNA, 13 bp, Artificial
  synthetic DNA
taagagacagttc

SEQ ID NO: 2141 - DNA, 13 bp, Artificial
  synthetic DNA
taagagacagttg

SEQ ID NO: 2142 - DNA, 13 bp, Artificial
  synthetic DNA
taagagacagttt

SEQ ID NO: 2143 - DNA, 70 bp, Artificial
  synthetic DNA
aatgatacggcgaccaccgagatctacacgtcgtgcatcgtcggcagcgtcagatgtgtataagagacag

SEQ ID NO: 2144 - DNA, 70 bp, Artificial
  synthetic DNA
aatgatacggcgaccaccgagatctacactcgctgcatcgtcggcagcgtcagatgtgtataagagacag

SEQ ID NO: 2145 - DNA, 70 bp, Artificial
  synthetic DNA
aatgatacggcgaccaccgagatctacaccacagtagtcgtcggcagcgtcagatgtgtataagagacag

SEQ ID NO: 2146 - DNA, 70 bp, Artificial
  synthetic DNA
aatgatacggcgaccaccgagatctacactgctcgattcgtcggcagcgtcagatgtgtataagagacag

SEQ ID NO: 2147 - DNA, 70 bp, Artificial
  synthetic DNA
aatgatacggcgaccaccgagatctacactgacgagttcgtcggcagcgtcagatgtgtataagagacag

SEQ ID NO: 2148 - DNA, 70 bp, Artificial
  synthetic DNA
aatgatacggcgaccaccgagatctacacgcatatgttcgtcggcagcgtcagatgtgtataagagacag

SEQ ID NO: 2149 - DNA, 66 bp, Artificial
  synthetic DNA
caagcagaagacggcatacgagataagaggcagtctcgtgggctcggagatgtgtataagagacag

SEQ ID NO: 2150 - DNA, 66 bp, Artificial
  synthetic DNA
caagcagaagacggcatacgagataggagtccgtctcgtgggctcggagatgtgtataagagacag

SEQ ID NO: 2151 - DNA, 66 bp, Artificial
  synthetic DNA
caagcagaagacggcatacgagatgtagagaggtctcgtgggctcggagatgtgtataagagacag

SEQ ID NO: 2152 - DNA, 66 bp, Artificial
  synthetic DNA
caagcagaagacggcatacgagatcctctctggtctcgtgggctcggagatgtgtataagagacag

SEQ ID NO: 2153 - DNA, 349 bp, Zea mays
gtgggtaggtagagaatacctaggggcgcgagacaactctctctaaggaactcggcaaaatagccccgtaacttcgggagaaggggtgccccctcgcaaaagggggtcgcagtgaccaggcccgggcgactgtataccaaaaacacaggtctccgcaaagtcgtaagaccatgtatgggggctgacgcctgcccagtgccggaaggtcaaggaagttggtgaactgatgacagggaagccggcgaccgaagccccggtgaacggcggccgtaactataacggtcctaaggtagcgaaattccttgtcgggtaagttccgacccgcacgaaaggcgtaacgatctgggca

SEQ ID NO: 2154 - DNA, 348 bp, Oryza sativa
gtgggtaggtagagaatacctaggggcgcgagacaactctctctaaggaactcggcaaaatagccccgtaacttcgggagaaggggtgccccctcgcaaaagggggtcgcagtgaccaggcccgggcgactgtttaccaaaaacacaggtctccgcaaagtcgtaagaccatgtatgggggctgacgcctgcccagtgccggaagtcaaggaagttggtgaactgatgacagggaagccggcgaccgaagccccggtgaacggcggccgtaactataacggtcctaaggtagcgaaattccttgtcgggtaagttccgacccgcacgaaaggcgtaacgatctgggca

SEQ ID NO: 2155 - DNA, 348 bp, Solanum tuberosum
gtgggtaggtagagaatacctaggggcgcgagacaactctctctaaggaactcggcaaaatagccccgtaacttcgggagaaggggtgcctcctcacaaagggggtcgcagtgaccaggcccgggcgactgtttaccaaaaacacaggtctccgcaaagtcgtaagaccatgtatgggggctgacgcctgcccagtgccggaaggtcaaggaagttggtgacctgatgacaggggagccggcgaccgaagccccggtgaacggcggccgtaactataacggtcctaaggtagcgaaattccttgtcgggtaagttccgacccgcacgaaaggcgtaacgatctgggca

SEQ ID NO: 2156 - DNA, 348 bp, Glycine max
gtgggtaggtagagaatacctagaggcgcgagacaactctctctaaggaactcggcaaaatagccccgtaacttcgggagaaggggtgcctcctcacaaagggggtcgcagtgaccaggcccgggcgactgtttaccaaaaacacaggtctccgcaaagtcgtaagaccatgtatgggggctgacgcctgcccagtgccggaaggtcaaggaagttggtgacctgatgacaggggagccgacgaccgaagccccggtgaacggcggccgtaactataacggtcctaaggtagcgaaattccttgtcgggtaagttccgacccgcacgaaaggcgtaacgatctgggca

SEQ ID NO: 2157 - DNA, 349 bp, Zea mays; identical to SEQ ID NO: 2153

SEQ ID NO: 2158 - DNA, 348 bp, Oryza sativa; identical to SEQ ID NO: 2154

SEQ ID NO: 2159 - DNA, 348 bp, Solanum tuberosum; identical to SEQ ID NO: 2155

SEQ ID NO: 2160 - DNA, 348 bp, Glycine max; identical to SEQ ID NO: 2156

SEQ ID NO: 2161 - DNA, 114 bp, Oryza sativa
gtattgcgagacagccagaagcagaaggtaaaatacgcggtactttattgcttagtctagcttttatggaagctttaacaatttatggactagttgtggcactggcgcttttat

SEQ ID NO: 2162 - DNA, 87 bp, Oryza sativa
ccagaagcagaaggtaaaatacgcggtactttattgcttagtctagcttttatggaagctttaacaatttatggactagttgtggca